European Patent Specification EP 3 174 993 B1, published December 6, 2023. Title: PROBE LIBRARY CONSTRUCTION. Applicant: President and Fellows of Harvard College. Application Not Yet Assigned. The sequence listing filed with the application follows.

SEQUENCE LISTING (937 sequences)

SEQ ID NO: 1 - DNA, 20 bp, Artificial Sequence
  Synthetic Polynucleotide
taatacgactcactataggg

SEQ ID NO: 2 - DNA, 20 bp, Artificial Sequence
  Synthetic Polynucleotide
caggcatccgagaggtctgg

SEQ ID NO: 3 - DNA, 102 bp, Artificial Sequence
  Synthetic Polynucleotide
acaaccgcgtgttacaaggccaggcatccgagaggtctgggaatgccagcagctctacaagtgcggccatttggttcattgcgcttctccggaaacattagc

SEQ ID NO: 4 - DNA, 20 bp, Artificial Sequence
  Synthetic Polynucleotide
cggtaggaccctacacatcc

SEQ ID NO: 5 - DNA, 20 bp, Artificial Sequence
  Synthetic Polynucleotide
tgtggcgcctaaccatacac

SEQ ID NO: 6 - DNA, 20 bp, Artificial Sequence
  Synthetic Polynucleotide
gacaccgagctagaattcgg

SEQ ID NO: 7 - DNA, 20 bp, Artificial Sequence
  Synthetic Polynucleotide
tgtcttgggtcctcttacgg

SEQ ID NO: 8 - DNA, 20 bp, Artificial Sequence
  Synthetic Polynucleotide
tatcacgtgaggctccgtgt

SEQ ID NO: 9 - DNA, 20 bp, Artificial Sequence
  Synthetic Polynucleotide
gtctacggatccttgcgtgt

SEQ ID NO: 10 - DNA, 20 bp, Artificial Sequence
  Synthetic Polynucleotide
acgggtacattggatccact

SEQ ID NO: 11 - DNA, 20 bp, Artificial Sequence
  Synthetic Polynucleotide
aagacgtggtccaccctgat

SEQ ID NO: 12 - DNA, 20 bp, Artificial Sequence
  Synthetic Polynucleotide
tgccaggtccactacttggg

SEQ ID NO: 13 - DNA, 20 bp, Artificial Sequence
  Synthetic Polynucleotide
gacccgaaggagaatgcaaa

SEQ ID NO: 14 - DNA, 20 bp, Artificial Sequence
  Synthetic Polynucleotide
atgtcgtctctcagggcttt

SEQ ID NO: 15 - DNA, 20 bp, Artificial Sequence
  Synthetic Polynucleotide
aagggcggaagcactctctt

SEQ ID NO: 16 - DNA, 20 bp, Artificial Sequence
  Synthetic Polynucleotide
tggtcccgcatttgtacctt

SEQ ID NO: 17 - DNA, 20 bp, Artificial Sequence
  Synthetic Polynucleotide
aagtccgtctgctaagccat

SEQ ID NO: 18 - DNA, 20 bp, Artificial Sequence
  Synthetic Polynucleotide
cttccagagtcctggcatga

SEQ ID NO: 19 - DNA, 20 bp, Artificial Sequence
  Synthetic Polynucleotide
tctaacgagctccgtggttg

SEQ ID NO: 20 - DNA, 20 bp, Artificial Sequence
  Synthetic Polynucleotide
cctgggcaggaaacaacact

SEQ ID NO: 21 - DNA, 20 bp, Artificial Sequence
  Synthetic Polynucleotide
gcgcacaccttagtcatagc

SEQ ID NO: 22 - DNA, 20 bp, Artificial Sequence
  Synthetic Polynucleotide
gtgcgattgtcacatgtgct

SEQ ID NO: 23 - DNA, 20 bp, Artificial Sequence
  Synthetic Polynucleotide
ggcttgtcctcaattatccg

SEQ ID NO: 24 - DNA, 20 bp, Artificial Sequence
  Synthetic Polynucleotide
cccacgtgacttgacttctc

SEQ ID NO: 25 - DNA, 20 bp, Artificial Sequence
  Synthetic Polynucleotide
cctctacatgctccggatcc

SEQ ID NO: 26 - DNA, 20 bp, Artificial Sequence
  Synthetic Polynucleotide
gaatagtaacccggtcgcaa

SEQ ID NO: 27 - DNA, 20 bp, Artificial Sequence
  Synthetic Polynucleotide
tgggccactagtcttcgcta

SEQ ID NO: 28 - DNA, 20 bp, Artificial Sequence
  Synthetic Polynucleotide
cggcacgtaccctttacagg

SEQ ID NO: 29 - DNA, 20 bp, Artificial Sequence
  Synthetic Polynucleotide
gatcagtgagcctcaccaag

SEQ ID NO: 30 - DNA, 20 bp, Artificial Sequence
  Synthetic Polynucleotide
tggtatgtgagctctttggg

SEQ ID NO: 31 - DNA, 20 bp, Artificial Sequence
  Synthetic Polynucleotide
agagtcacgcatacttggga

SEQ ID NO: 32 - DNA, 20 bp, Artificial Sequence
  Synthetic Polynucleotide
gggtcaggcgtcatagattg

SEQ ID NO: 33 - DNA, 20 bp, Artificial Sequence
  Synthetic Polynucleotide
agaatgtggaggacatgtgg

SEQ ID NO: 34 - DNA, 20 bp, Artificial Sequence
  Synthetic Polynucleotide
tcggactgtgagacatttcc

SEQ ID NO: 35 - DNA, 20 bp, Artificial Sequence
  Synthetic Polynucleotide
atcaaatgcctcggtcgttg

SEQ ID NO: 36 - DNA, 20 bp, Artificial Sequence
  Synthetic Polynucleotide
gcaatgctatgctgggacaa

SEQ ID NO: 37 - DNA, 20 bp, Artificial Sequence
  Synthetic Polynucleotide
atggaggccgttctctgaca

SEQ ID NO: 38 - DNA, 20 bp, Artificial Sequence
  Synthetic Polynucleotide
gcagatgggtgcattcattc

SEQ ID NO: 39 - DNA, 20 bp, Artificial Sequence
  Synthetic Polynucleotide
tatgcactctgcggatgacc

SEQ ID NO: 40 - DNA, 20 bp, Artificial Sequence
  Synthetic Polynucleotide
gacccgggagttatgatacg

SEQ ID NO: 41 - DNA, 20 bp, Artificial Sequence
  Synthetic Polynucleotide
ctcgggtaggctatctccaa

SEQ ID NO: 42 - DNA, 20 bp, Artificial Sequence
  Synthetic Polynucleotide
ctgcaggtgctctagatgga

SEQ ID NO: 43 - DNA, 20 bp, Artificial Sequence
  Synthetic Polynucleotide
gtccaggctcgtcttctcga

SEQ ID NO: 44 - DNA, 20 bp, Artificial Sequence
  Synthetic Polynucleotide
cttacctgagcgcagttcga

SEQ ID NO: 45 - DNA, 20 bp, Artificial Sequence
  Synthetic Polynucleotide
gttgttcgatccctccacca

SEQ ID NO: 46 - DNA, 20 bp, Artificial Sequence
  Synthetic Polynucleotide
cggcagaggataatcctagc

SEQ ID NO: 47 - DNA, 20 bp, Artificial Sequence
  Synthetic Polynucleotide
gggagtccggatgttagtgc

SEQ ID NO: 48 - DNA, 20 bp, Artificial Sequence
  Synthetic Polynucleotide
cgcatctatgctccgcttac

SEQ ID NO: 49 - DNA, 20 bp, Artificial Sequence
  Synthetic Polynucleotide
aacgcgctacccaattctag

SEQ ID NO: 50 - DNA, 20 bp, Artificial Sequence
  Synthetic Polynucleotide
tactggacgattcccgactg

SEQ ID NO: 51 - DNA, 20 bp, Artificial Sequence
  Synthetic Polynucleotide
agcgtcgtacccagttaagc

SEQ ID NO: 52 - DNA, 20 bp, Artificial Sequence
  Synthetic Polynucleotide
gagattcacgccctcatgag

SEQ ID NO: 53 - DNA, 20 bp, Artificial Sequence
  Synthetic Polynucleotide
ccgctagcgttacctctacc

SEQ ID NO: 54 - DNA, 20 bp, Artificial Sequence
  Synthetic Polynucleotide
ccacaccgtatgcatttctg

SEQ ID NO: 55 - DNA, 20 bp, Artificial Sequence
  Synthetic Polynucleotide
ccttagcgcacaaagagacg

SEQ ID NO: 56 - DNA, 20 bp, Artificial Sequence
  Synthetic Polynucleotide
gtcctgatggctttctcacg

SEQ ID NO: 57 - DNA, 20 bp, Artificial Sequence
  Synthetic Polynucleotide
ggtcgtcggtagatcattgc

SEQ ID NO: 58 - DNA, 20 bp, Artificial Sequence
  Synthetic Polynucleotide
agagccggtatgatccatcg

SEQ ID NO: 59 - DNA, 20 bp, Artificial Sequence
  Synthetic Polynucleotide
ccggacgaaggttgatatcc

SEQ ID NO: 60 - DNA, 20 bp, Artificial Sequence
  Synthetic Polynucleotide
acccggtacctgttatcacg

SEQ ID NO: 61 - DNA, 20 bp, Artificial Sequence
  Synthetic Polynucleotide
atcccgtctcgttctatggg

SEQ ID NO: 62 - DNA, 20 bp, Artificial Sequence
  Synthetic Polynucleotide
caggtgagggtctctccttc

SEQ ID NO: 63 - DNA, 20 bp, Artificial Sequence
  Synthetic Polynucleotide
ccttatggaaacgtgatgcc

SEQ ID NO: 64 - DNA, 20 bp, Artificial Sequence
  Synthetic Polynucleotide
ggctgggcatacatagacct

SEQ ID NO: 65 - DNA, 20 bp, Artificial Sequence
  Synthetic Polynucleotide
agtggcggctattaccggat

SEQ ID NO: 66 - DNA, 20 bp, Artificial Sequence
  Synthetic Polynucleotide
tgataacgtccgctcgttga

SEQ ID NO: 67 - DNA, 20 bp, Artificial Sequence
  Synthetic Polynucleotide
tacatcgttgaggcccgttt

SEQ ID NO: 68 - DNA, 20 bp, Artificial Sequence
  Synthetic Polynucleotide
cgttgtggcatcagctagag

SEQ ID NO: 69 - DNA, 20 bp, Artificial Sequence
  Synthetic Polynucleotide
actggcccacacacttacct

SEQ ID NO: 70 - DNA, 20 bp, Artificial Sequence
  Synthetic Polynucleotide
atcgggtcacggaatatgac

SEQ ID NO: 71 - DNA, 20 bp, Artificial Sequence
  Synthetic Polynucleotide
cgtaggttcacagatttgcg

SEQ ID NO: 72 - DNA, 20 bp, Artificial Sequence
  Synthetic Polynucleotide
tagggcacgagaaggtatcc

SEQ ID NO: 73 - DNA, 20 bp, Artificial Sequence
  Synthetic Polynucleotide
actagcttgtatcgccggat

SEQ ID NO: 74 - DNA, 20 bp, Artificial Sequence
  Synthetic Polynucleotide
cggcggtttgatattcgaag

SEQ ID NO: 75 - DNA, 20 bp, Artificial Sequence
  Synthetic Polynucleotide
gccgagtgtttatgagcaag

SEQ ID NO: 76 - DNA, 20 bp, Artificial Sequence
  Synthetic Polynucleotide
tctccgaagatccgatatcg

SEQ ID NO: 77 - DNA, 20 bp, Artificial Sequence
  Synthetic Polynucleotide
gatgcagggcctaattaacg

SEQ ID NO: 78 - DNA, 20 bp, Artificial Sequence
  Synthetic Polynucleotide
tgacgcggctaaatactgac

SEQ ID NO: 79 - DNA, 20 bp, Artificial Sequence
  Synthetic Polynucleotide
gcaatgcacgctctcctagt

SEQ ID NO: 80 - DNA, 20 bp, Artificial Sequence
  Synthetic Polynucleotide
tggcgtcagatggattagga

SEQ ID NO: 81 - DNA, 20 bp, Artificial Sequence
  Synthetic Polynucleotide
gttggcgggagactaagaag

SEQ ID NO: 82 - DNA, 20 bp, Artificial Sequence
  Synthetic Polynucleotide
tcgcgtctcgtccttctacc

SEQ ID NO: 83 - DNA, 20 bp, Artificial Sequence
  Synthetic Polynucleotide
cggtcacgtcggaaataacc

SEQ ID NO: 84 - DNA, 20 bp, Artificial Sequence
  Synthetic Polynucleotide
attaacgggccaggttactg

SEQ ID NO: 85 - DNA, 20 bp, Artificial Sequence
  Synthetic Polynucleotide
attgtatggaggcgccctat

SEQ ID NO: 86 - DNA, 20 bp, Artificial Sequence
  Synthetic Polynucleotide
gccagctttccaagattcag

SEQ ID NO: 87 - DNA, 20 bp, Artificial Sequence
  Synthetic Polynucleotide
acaaccgcgtgttacaaggc

SEQ ID NO: 88 - DNA, 20 bp, Artificial Sequence
  Synthetic Polynucleotide
gctaatgtttccggagaagc

SEQ ID NO: 89 - DNA, 20 bp, Artificial Sequence
  Synthetic Polynucleotide
gaagtatccggcatcacagc

SEQ ID NO: 90 - DNA, 20 bp, Artificial Sequence
  Synthetic Polynucleotide
tcgttacggactttcacgac

SEQ ID NO: 91 - DNA, 20 bp, Artificial Sequence
  Synthetic Polynucleotide
gccattctgacatacccaga

SEQ ID NO: 92 - DNA, 20 bp, Artificial Sequence
  Synthetic Polynucleotide
gtatttgaaccggccagctg

SEQ ID NO: 93 - DNA, 20 bp, Artificial Sequence
  Synthetic Polynucleotide
ggttgtgggccatatccaat

SEQ ID NO: 94 - DNA, 20 bp, Artificial Sequence
  Synthetic Polynucleotide
ggcgttccatcgaaactcta

SEQ ID NO: 95 - DNA, 20 bp, Artificial Sequence
  Synthetic Polynucleotide
ggccatcgacttagattcca

SEQ ID NO: 96 - DNA, 20 bp, Artificial Sequence
  Synthetic Polynucleotide
ggtgctcctgccattatagg

SEQ ID NO: 97 - DNA, 20 bp, Artificial Sequence
  Synthetic Polynucleotide
tgtcgacgtgcggaaagtag

SEQ ID NO: 98 - DNA, 20 bp, Artificial Sequence
  Synthetic Polynucleotide
gccgcacgagtatgctactg

SEQ ID NO: 99 - DNA, 20 bp, Artificial Sequence
  Synthetic Polynucleotide
tgctgccgcttactactgct

SEQ ID NO: 100 - DNA, 20 bp, Artificial Sequence
  Synthetic Polynucleotide
tagcactcttctggccatcg

SEQ ID NO: 101 - DNA, 20 bp, Artificial Sequence
  Synthetic Polynucleotide
cggtaatcggttcaccagtg

SEQ ID NO: 102 - DNA, 20 bp, Artificial Sequence
  Synthetic Polynucleotide
tttagtgcctggctccgttg

SEQ ID NO: 103 - DNA, 20 bp, Artificial Sequence
  Synthetic Polynucleotide
ggagttacagccactttcgg

SEQ ID NO: 104 - DNA, 20 bp, Artificial Sequence
  Synthetic Polynucleotide
gtgtggacggaacctgacaa

SEQ ID NO: 105 - DNA, 20 bp, Artificial Sequence
  Synthetic Polynucleotide
cacacgtggaattgttctgc

SEQ ID NO: 106 - DNA, 20 bp, Artificial Sequence
  Synthetic Polynucleotide
cttgtacatggagggcgact

SEQ ID NO: 107 - DNA, 20 bp, Artificial Sequence
  Synthetic Polynucleotide
aatccggtgtacaggttccc

SEQ ID NO: 108 - DNA, 20 bp, Artificial Sequence
  Synthetic Polynucleotide
aggtgcgacgatatacacca

SEQ ID NO: 109 - DNA, 20 bp, Artificial Sequence
  Synthetic Polynucleotide
actgcatatgaccgctgcaa

SEQ ID NO: 110 - DNA, 20 bp, Artificial Sequence
  Synthetic Polynucleotide
ccttccattagccgagatca

SEQ ID NO: 111 - DNA, 20 bp, Artificial Sequence
  Synthetic Polynucleotide
gacgcgaggagtgatcgact

SEQ ID NO: 112 - DNA, 20 bp, Artificial Sequence
  Synthetic Polynucleotide
cgaccctcacacatttgggt

SEQ ID NO: 113 - DNA, 20 bp, Artificial Sequence
  Synthetic Polynucleotide
cgctcccgtattcttctgtg

SEQ ID NO: 114 - DNA, 20 bp, Artificial Sequence
  Synthetic Polynucleotide
cagggatagtcaggccagtg

SEQ ID NO: 115 - DNA, 20 bp, Artificial Sequence
  Synthetic Polynucleotide
cgtaatgagtgcttcgccat

SEQ ID NO: 116 - DNA, 20 bp, Artificial Sequence
  Synthetic Polynucleotide
ctcgtctcgtggaacacatg

SEQ ID NO: 117 - DNA, 20 bp, Artificial Sequence
  Synthetic Polynucleotide
tatgctgggcagtaatcagg

SEQ ID NO: 118 - DNA, 20 bp, Artificial Sequence
  Synthetic Polynucleotide
gcatctcgtagcatcctgct

SEQ ID NO: 119 - DNA, 20 bp, Artificial Sequence
  Synthetic Polynucleotide
agtatggtaccgggaacagc

SEQ ID NO: 120 - DNA, 20 bp, Artificial Sequence
  Synthetic Polynucleotide
accattctcgcaactcgcta

SEQ ID NO: 121 - DNA, 20 bp, Artificial Sequence
  Synthetic Polynucleotide
cgtgggcgaagtacttggtc

SEQ ID NO: 122 - DNA, 20 bp, Artificial Sequence
  Synthetic Polynucleotide
ccggacgtcttcgataatgc

SEQ ID NO: 123 - DNA, 20 bp, Artificial Sequence
  Synthetic Polynucleotide
tgatgctctttgcagttcgg

SEQ ID NO: 124 - DNA, 20 bp, Artificial Sequence
  Synthetic Polynucleotide
atgccggtcataacagtgtc

SEQ ID NO: 125 - DNA, 20 bp, Artificial Sequence
  Synthetic Polynucleotide
tggtggctcgttatcacaag

SEQ ID NO: 126 - DNA, 20 bp, Artificial Sequence
  Synthetic Polynucleotide
tctgaagcgtggccattacc

SEQ ID NO: 127 - DNA, 20 bp, Artificial Sequence
  Synthetic Polynucleotide
catatgccggacattcagct

SEQ ID NO: 128 - DNA, 20 bp, Artificial Sequence
  Synthetic Polynucleotide
actaatggtcctgcggcata

SEQ ID NO: 129 - DNA, 20 bp, Artificial Sequence
  Synthetic Polynucleotide
ggtgccgtgttgcatgtaag

SEQ ID NO: 130 - DNA, 20 bp, Artificial Sequence
  Synthetic Polynucleotide
aagcggtcgtggtttatacc

SEQ ID NO: 131 - DNA, 20 bp, Artificial Sequence
  Synthetic Polynucleotide
gccaccttgtatggtatcga

SEQ ID NO: 132 - DNA, 20 bp, Artificial Sequence
  Synthetic Polynucleotide
taatgcttaggcccgtcggt

SEQ ID NO: 133 - DNA, 20 bp, Artificial Sequence
  Synthetic Polynucleotide
gacgcgacggattatttagg

SEQ ID NO: 134 - DNA, 20 bp, Artificial Sequence
  Synthetic Polynucleotide
ggtcgcgcccatatataagg

SEQ ID NO: 135 - DNA, 20 bp, Artificial Sequence
  Synthetic Polynucleotide
tgactacggttgggtgcatc

SEQ ID NO: 136 - DNA, 20 bp, Artificial Sequence
  Synthetic Polynucleotide
tcaggcgctcattgtatgtc

SEQ ID NO: 137 - DNA, 20 bp, Artificial Sequence
  Synthetic Polynucleotide
gtagatactcccggcccgaa

SEQ ID NO: 138 - DNA, 20 bp, Artificial Sequence
  Synthetic Polynucleotide
gcagcacttagggcagcatc

SEQ ID NO: 139 - DNA, 20 bp, Artificial Sequence
  Synthetic Polynucleotide
cgcgggaaccatattaggaa

SEQ ID NO: 140 - DNA, 20 bp, Artificial Sequence
  Synthetic Polynucleotide
gatccatggccagttcgtat

SEQ ID NO: 141 - DNA, 20 bp, Artificial Sequence
  Synthetic Polynucleotide
gtgcgccaaaggacttagtg

SEQ ID NO: 142 - DNA, 20 bp, Artificial Sequence
  Synthetic Polynucleotide
gatcccgctattcaccgatt

SEQ ID NO: 143 - DNA, 20 bp, Artificial Sequence
  Synthetic Polynucleotide
gcatagatggttcacccgta

SEQ ID NO: 144 - DNA, 20 bp, Artificial Sequence
  Synthetic Polynucleotide
gtctataagccgcgctgcaa

SEQ ID NO: 145 - DNA, 20 bp, Artificial Sequence
  Synthetic Polynucleotide
gcggagtatgccatcatgag

SEQ ID NO: 146 - DNA, 20 bp, Artificial Sequence
  Synthetic Polynucleotide
tgccgcgatcatctactatg

SEQ ID NO: 147 - DNA, 20 bp, Artificial Sequence
  Synthetic Polynucleotide
gaccgggtattcgacgtcat

SEQ ID NO: 148 - DNA, 20 bp, Artificial Sequence
  Synthetic Polynucleotide
gcagtgcgggtagatacgct

SEQ ID NO: 149 - DNA, 20 bp, Artificial Sequence
  Synthetic Polynucleotide
aggcgtgggtagcaacgtat

SEQ ID NO: 150 - DNA, 20 bp, Artificial Sequence
  Synthetic Polynucleotide
gctcattggactttctccca

SEQ ID NO: 151 - DNA, 20 bp, Artificial Sequence
  Synthetic Polynucleotide
aaggaccacgtatctgcatg

SEQ ID NO: 152 - DNA, 20 bp, Artificial Sequence
  Synthetic Polynucleotide
atctgatagtgccgcgacgt

SEQ ID NO: 153 - DNA, 20 bp, Artificial Sequence
  Synthetic Polynucleotide
tgacctgcacggatagtagg

SEQ ID NO: 154 - DNA, 20 bp, Artificial Sequence
  Synthetic Polynucleotide
gttattcgcagtccttgggt

SEQ ID NO: 155 - DNA, 20 bp, Artificial Sequence
  Synthetic Polynucleotide
gtgcagtgtgcttaaatccg

SEQ ID NO: 156 - DNA, 20 bp, Artificial Sequence
  Synthetic Polynucleotide
cgcgggtgttaaataaggac

SEQ ID NO: 157 - DNA, 20 bp, Artificial Sequence
  Synthetic Polynucleotide
gcgaggcgtggtaatagtca

SEQ ID NO: 158 - DNA, 20 bp, Artificial Sequence
  Synthetic Polynucleotide
caaggcgcaaacatagacag

SEQ ID NO: 159 - DNA, 20 bp, Artificial Sequence
  Synthetic Polynucleotide
ggaacaagggcgtctatgtc

SEQ ID NO: 160 - DNA, 20 bp, Artificial Sequence
  Synthetic Polynucleotide
gcagtgcggataagctacac

SEQ ID NO: 161 - DNA, 20 bp, Artificial Sequence
  Synthetic Polynucleotide
agagatgcgtgtaggcgatt

SEQ ID NO: 162 - DNA, 20 bp, Artificial Sequence
  Synthetic Polynucleotide
ccctttcgagctaagtttgg

SEQ ID NO: 163 - DNA, 20 bp, Artificial Sequence
  Synthetic Polynucleotide
ccttaagcaacccgtcgatg

SEQ ID NO: 164 - DNA, 20 bp, Artificial Sequence
  Synthetic Polynucleotide
ttgctcgtgactgaacaacg

SEQ ID NO: 165 - DNA, 20 bp, Artificial Sequence
  Synthetic Polynucleotide
ggtcgtgcgtataagcctca

SEQ ID NO: 166 - DNA, 20 bp, Artificial Sequence
  Synthetic Polynucleotide
cggatggtcttcgtttaacc

SEQ ID NO: 167 - DNA, 20 bp, Artificial Sequence
  Synthetic Polynucleotide
ggcacggtggctagtaacga

SEQ ID NO: 168 - DNA, 20 bp, Artificial Sequence
  Synthetic Polynucleotide
gccggcccaactgatagtag

SEQ ID NO: 169 - DNA, 20 bp, Artificial Sequence
  Synthetic Polynucleotide
tcgacttcggtcacctttcc

SEQ ID NO: 170 - DNA, 20 bp, Artificial Sequence
  Synthetic Polynucleotide
cgggtcgatactttcctcgt

SEQ ID NO: 171 - DNA, 20 bp, Artificial Sequence
  Synthetic Polynucleotide
gtgccgtgtgtaatatccga

SEQ ID NO: 172 - DNA, 20 bp, Artificial Sequence
  Synthetic Polynucleotide
cgcgcctggaataactccta

SEQ ID NO: 173 - DNA, 20 bp, Artificial Sequence
  Synthetic Polynucleotide
gtcagggaaccgtttcttca

SEQ ID NO: 174 - DNA, 20 bp, Artificial Sequence
  Synthetic Polynucleotide
cttgtcatgtacccgaatgg

SEQ ID NO: 175 - DNA, 20 bp, Artificial Sequence
  Synthetic Polynucleotide
cgacctggctacgtagaacc

SEQ ID NO: 176 - DNA, 20 bp, Artificial Sequence
  Synthetic Polynucleotide
ctagctaaagggccgtgcgt

SEQ ID NO: 177 - DNA, 20 bp, Artificial Sequence
  Synthetic Polynucleotide
aagtattagcgcggcaacgt

SEQ ID NO: 178 - DNA, 20 bp, Artificial Sequence
  Synthetic Polynucleotide
ggttgcgtgccacttaaagc

SEQ ID NO: 179 - DNA, 20 bp, Artificial Sequence
  Synthetic Polynucleotide
ggaggttcggttgtactgca

SEQ ID NO: 180 - DNA, 20 bp, Artificial Sequence
  Synthetic Polynucleotide
gttgtcgtcctccatcggtt

SEQ ID NO: 181 - DNA, 20 bp, Artificial Sequence
  Synthetic Polynucleotide
gggacggaactacacatgtg

SEQ ID NO: 182 - DNA, 20 bp, Artificial Sequence
  Synthetic Polynucleotide
gatccatcctgattgagggt

SEQ ID NO: 183 - DNA, 20 bp, Artificial Sequence
  Synthetic Polynucleotide
cttcatggtaccggttgaga

SEQ ID NO: 184 - DNA, 20 bp, Artificial Sequence
  Synthetic Polynucleotide
tcggtcggctgtaaggatac

SEQ ID NO: 185 - DNA, 20 bp, Artificial Sequence
  Synthetic Polynucleotide
attgcacgaggtcagagtcg

SEQ ID NO: 186 - DNA, 20 bp, Artificial Sequence
  Synthetic Polynucleotide
gcttagatccgctcgctacg

SEQ ID NO: 187 - DNA, 20 bp, Artificial Sequence
  Synthetic Polynucleotide
cggctggcctactgtagaga

SEQ ID NO: 188 - DNA, 20 bp, Artificial Sequence
  Synthetic Polynucleotide
gcaacatgacctgtcatcgc

SEQ ID NO: 189 - DNA, 20 bp, Artificial Sequence
  Synthetic Polynucleotide
ggccgcacgatatatttgac

SEQ ID NO: 190 - DNA, 20 bp, Artificial Sequence
  Synthetic Polynucleotide
cagccgggccataatagttg

SEQ ID NO: 191 - DNA, 20 bp, Artificial Sequence
  Synthetic Polynucleotide
tgcggtggacctattatcct

SEQ ID NO: 192 - DNA, 20 bp, Artificial Sequence
  Synthetic Polynucleotide
cctgcgttaggcaatccatc

SEQ ID NO: 193 - DNA, 20 bp, Artificial Sequence
  Synthetic Polynucleotide
gtgggctcttcgaagtaacc

SEQ ID NO: 194 - DNA, 20 bp, Artificial Sequence
  Synthetic Polynucleotide
gccgtggaccactaaagttc

SEQ ID NO: 195 - DNA, 20 bp, Artificial Sequence
  Synthetic Polynucleotide
gcttaagtcatgggcgcatc

SEQ ID NO: 196 - DNA, 20 bp, Artificial Sequence
  Synthetic Polynucleotide
acaggttagttccgcgcact

SEQ ID NO: 197 - DNA, 20 bp, Artificial Sequence
  Synthetic Polynucleotide
ggcgtggcatttagactacc

SEQ ID NO: 198 - DNA, 20 bp, Artificial Sequence
  Synthetic Polynucleotide
actacggccaacaaccaaca

SEQ ID NO: 199 - DNA, 20 bp, Artificial Sequence
  Synthetic Polynucleotide
gttgacaaggctctgtacgg

SEQ ID NO: 200 - DNA, 20 bp, Artificial Sequence
  Synthetic Polynucleotide
ttgttctcttgccggtcgat

SEQ ID NO: 201 - DNA, 20 bp, Artificial Sequence
  Synthetic Polynucleotide
gttgatcgtagccaattcgg

SEQ ID NO: 202 - DNA, 102 bp, Artificial Sequence; identical to SEQ ID NO: 3
  Synthetic Polynucleotide

SEQ ID NO: 203 - DNA, 102 bp, Artificial Sequence
  Synthetic Polynucleotide
acaaccgcgtgttacaaggccaggcatccgagaggtctgggaatgcctttcgcgatagcagccaggaagcctgcttcattgcgcttctccggaaacattagc

SEQ ID NO: 204 - DNA, 102 bp, Artificial Sequence
  Synthetic Polynucleotide
acaaccgcgtgttacaaggccaggcatccgagaggtctgggaatgcccagcgggaaacctttctgttgcagagcttcattgcgcttctccggaaacattagc

SEQ ID NO: 205 - DNA, 102 bp, Artificial Sequence
  Synthetic Polynucleotide
acaaccgcgtgttacaaggccaggcatccgagaggtctgggaatgccgccagttccgcagaagccaggaagacattcattgcgcttctccggaaacattagc

SEQ ID NO: 206 - DNA, 102 bp, Artificial Sequence
  Synthetic Polynucleotide
acaaccgcgtgttacaaggccaggcatccgagaggtctgggaatgccggtgtggcagaaagactgcatcaccaggtcattgcgcttctccggaaacattagc

SEQ ID NO: 207 - DNA, 102 bp, Artificial Sequence
  Synthetic Polynucleotide
acaaccgcgtgttacaaggccaggcatccgagaggtctgggaatgccgccgcgtttgttcggcacatgtggaatatcattgcgcttctccggaaacattagc

SEQ ID NO: 208 - DNA, 102 bp, Artificial Sequence
  Synthetic Polynucleotide
acaaccgcgtgttacaaggccaggcatccgagaggtctgggaatgcggtgcgtgttcacgtcaactggcttcggatcattgcgcttctccggaaacattagc

SEQ ID NO: 209 - DNA, 102 bp, Artificial Sequence
  Synthetic Polynucleotide
acaaccgcgtgttacaaggccaggcatccgagaggtctgggaatgccatctgcatcggcttccagcagctcaggatcattgcgcttctccggaaacattagc

SEQ ID NO: 210 - DNA, 102 bp, Artificial Sequence
  Synthetic Polynucleotide
acaaccgcgtgttacaaggccaggcatccgagaggtctgggaatgccgcagcacggaagtgaccgatgttggtcatcattgcgcttctccggaaacattagc

SEQ ID NO: 211 - DNA, 102 bp, Artificial Sequence
  Synthetic Polynucleotide
acaaccgcgtgttacaaggccaggcatccgagaggtctgggaatgccatccgggtcgttcggagcacacaggattgcattgcgcttctccggaaacattagc

SEQ ID NO: 212 - DNA, 102 bp, Artificial Sequence
  Synthetic Polynucleotide
acaaccgcgtgttacaaggccaggcatccgagaggtctgggaatgcatacgcgcaccactcttaccgaagacgctgcattgcgcttctccggaaacattagc

SEQ ID NO: 213 - DNA, 102 bp, Artificial Sequence
  Synthetic Polynucleotide
acaaccgcgtgttacaaggccaggcatccgagaggtctgggaatgcatcggctttctcggtgtactgagaaagctgcattgcgcttctccggaaacattagc

SEQ ID NO: 214 - DNA, 102 bp, Artificial Sequence
  Synthetic Polynucleotide
acaaccgcgtgttacaaggccaggcatccgagaggtctgggaatgccagtacccagacggttcgggaagttacgggcattgcgcttctccggaaacattagc

SEQ ID NO: 215 - DNA, 102 bp, Artificial Sequence
  Synthetic Polynucleotide
acaaccgcgtgttacaaggccaggcatccgagaggtctgggaatgcctttgttcagcttgatggtacaaccagcggcattgcgcttctccggaaacattagc

SEQ ID NO: 216 - DNA, 102 bp, Artificial Sequence
  Synthetic Polynucleotide
acaaccgcgtgttacaaggccaggcatccgagaggtctgggaatgccatccgcccaggactgcataacctgcttcgcattgcgcttctccggaaacattagc

SEQ ID NO: 217 - DNA, 102 bp, Artificial Sequence
  Synthetic Polynucleotide
acaaccgcgtgttacaaggccaggcatccgagaggtctgggaatgccccataaaccacagaacggagttagtggcgcattgcgcttctccggaaacattagc

SEQ ID NO: 218 - DNA, 102 bp, Artificial Sequence
  Synthetic Polynucleotide
acaaccgcgtgttacaaggccaggcatccgagaggtctgggaatgctcgttgcctgctttcgctttctcttctacgcattgcgcttctccggaaacattagc

SEQ ID NO: 219 - DNA, 102 bp, Artificial Sequence
  Synthetic Polynucleotide
acaaccgcgtgttacaaggccaggcatccgagaggtctgggaatgcccggtgccggagaaaggtcatcggtgttagcattgcgcttctccggaaacattagc

SEQ ID NO: 220 - DNA, 102 bp, Artificial Sequence
  Synthetic Polynucleotide
acaaccgcgtgttacaaggccaggcatccgagaggtctgggaatgcaccgccacggttcataatgaagtccggcagcattgcgcttctccggaaacattagc

SEQ ID NO: 221 - DNA, 102 bp, Artificial Sequence
  Synthetic Polynucleotide
acaaccgcgtgttacaaggccaggcatccgagaggtctgggaatgcggtcggcaactgacctttatgcgcatccagcattgcgcttctccggaaacattagc

SEQ ID NO: 222 - DNA, 102 bp, Artificial Sequence
  Synthetic Polynucleotide
acaaccgcgtgttacaaggccaggcatccgagaggtctgggaatgccagttcgccggtttcgtggttacgcacttccattgcgcttctccggaaacattagc

SEQ ID NO: 223 - DNA, 102 bp, Artificial Sequence
  Synthetic Polynucleotide
acaaccgcgtgttacaaggccaggcatccgagaggtctgggaatgctcgccgtaaccttccgcgatcatccacttccattgcgcttctccggaaacattagc

SEQ ID NO: 224 - DNA, 102 bp, Artificial Sequence
  Synthetic Polynucleotide
acaaccgcgtgttacaaggccaggcatccgagaggtctgggaatgccttgatcggaccaacaacaccaggctggtccattgcgcttctccggaaacattagc

SEQ ID NO: 225 - DNA, 102 bp, Artificial Sequence
  Synthetic Polynucleotide
acaaccgcgtgttacaaggccaggcatccgagaggtctgggaatgcccggtggtgtcctgggaacctacagaagtccattgcgcttctccggaaacattagc

SEQ ID NO: 226 - DNA, 102 bp, Artificial Sequence
  Synthetic Polynucleotide
acaaccgcgtgttacaaggccaggcatccgagaggtctgggaatgcggacgcatcggttagctcaaaggcctgctccattgcgcttctccggaaacattagc

SEQ ID NO: 227 - DNA, 102 bp, Artificial Sequence
  Synthetic Polynucleotide
acaaccgcgtgttacaaggccaggcatccgagaggtctgggaatgcatctacctgcgccacgtaggtctggtactccattgcgcttctccggaaacattagc

SEQ ID NO: 228 - DNA, 102 bp, Artificial Sequence
  Synthetic Polynucleotide
acaaccgcgtgttacaaggccaggcatccgagaggtctgggaatgcatacggccaccagcacgcacttcatcaatccattgcgcttctccggaaacattagc

SEQ ID NO: 229 - DNA, 102 bp, Artificial Sequence
  Synthetic Polynucleotide
acaaccgcgtgttacaaggccaggcatccgagaggtctgggaatgcatcgaacatcagcagcgtgtgagaaagtgccattgcgcttctccggaaacattagc

SEQ ID NO: 230 - DNA, 102 bp, Artificial Sequence
  Synthetic Polynucleotide
acaaccgcgtgttacaaggccaggcatccgagaggtctgggaatgcaatatccgccagatcgatgtcgatcactgccattgcgcttctccggaaacattagc

SEQ ID NO: 231 - DNA, 102 bp, Artificial Sequence
  Synthetic Polynucleotide
acaaccgcgtgttacaaggccaggcatccgagaggtctgggaatgcaacacttcgtcgatcttctcaccctgtacccattgcgcttctccggaaacattagc

SEQ ID NO: 232 - DNA, 102 bp, Artificial Sequence
  Synthetic Polynucleotide
acaaccgcgtgttacaaggccaggcatccgagaggtctgggaatgccttgcctttcttctcaacggtcagcagacccattgcgcttctccggaaacattagc

SEQ ID NO: 233 - DNA, 102 bp, Artificial Sequence
  Synthetic Polynucleotide
acaaccgcgtgttacaaggccaggcatccgagaggtctgggaatgcccatgccctgaatacgacgttccagggtaccattgcgcttctccggaaacattagc

SEQ ID NO: 234 - DNA, 102 bp, Artificial Sequence
  Synthetic Polynucleotide
acaaccgcgtgttacaaggccaggcatccgagaggtctgggaatgcggaaacgggtatgggagtcaccaccggtaccattgcgcttctccggaaacattagc

SEQ ID NO: 235 - DNA, 102 bp, Artificial Sequence
  Synthetic Polynucleotide
acaaccgcgtgttacaaggccaggcatccgagaggtctgggaatgccgaagaacccgtacccacaacgtcaccgaccattgcgcttctccggaaacattagc

SEQ ID NO: 236 - DNA, 102 bp, Artificial Sequence
  Synthetic Polynucleotide
acaaccgcgtgttacaaggccaggcatccgagaggtctgggaatgcacgtcaatcacgtcgcccatgttcaggttacattgcgcttctccggaaacattagc

SEQ ID NO: 237 - DNA, 102 bp, Artificial Sequence
  Synthetic Polynucleotide
acaaccgcgtgttacaaggccaggcatccgagaggtctgggaatgcaccagaccagaacccgccgggaaagagatacattgcgcttctccggaaacattagc

SEQ ID NO: 238 - DNA, 102 bp, Artificial Sequence
  Synthetic Polynucleotide
acaaccgcgtgttacaaggccaggcatccgagaggtctgggaatgcttgaagcgcaccagaacggattccggcatacattgcgcttctccggaaacattagc

SEQ ID NO: 239 - DNA, 102 bp, Artificial Sequence
  Synthetic Polynucleotide
acaaccgcgtgttacaaggccaggcatccgagaggtctgggaatgcccttcttcggtcaactgtgcggcgtccatacattgcgcttctccggaaacattagc

SEQ ID NO: 240 - DNA, 102 bp, Artificial Sequence
  Synthetic Polynucleotide
acaaccgcgtgttacaaggccaggcatccgagaggtctgggaatgcggttacccatacacagggaacagccagggacattgcgcttctccggaaacattagc

SEQ ID NO: 241 - DNA, 102 bp, Artificial Sequence
  Synthetic Polynucleotide
acaaccgcgtgttacaaggccaggcatccgagaggtctgggaatgctcagatccggcagaccttcaatttccaggacattgcgcttctccggaaacattagc

SEQ ID NO: 242 - DNA, 102 bp, Artificial Sequence
  Synthetic Polynucleotide
acaaccgcgtgttacaaggccaggcatccgagaggtctgggaatgcccagtttggcatcatccagcgcgtcgatcacattgcgcttctccggaaacattagc

SEQ ID NO: 243 - DNA, 102 bp, Artificial Sequence
  Synthetic Polynucleotide
acaaccgcgtgttacaaggccaggcatccgagaggtctgggaatgccccaggcacgccaggtctttcagttcatcacattgcgcttctccggaaacattagc

SEQ ID NO: 244 - DNA, 102 bp, Artificial Sequence
  Synthetic Polynucleotide
acaaccgcgtgttacaaggccaggcatccgagaggtctgggaatgcctttggtggtcaggccacgcccgataatcacattgcgcttctccggaaacattagc

SEQ ID NO: 245 - DNA, 102 bp, Artificial Sequence
  Synthetic Polynucleotide
acaaccgcgtgttacaaggccaggcatccgagaggtctgggaatgctgatcgcatacagcggaatagcgtgtaccacattgcgcttctccggaaacattagc

SEQ ID NO: 246 - DNA, 102 bp, Artificial Sequence
  Synthetic Polynucleotide
acaaccgcgtgttacaaggccaggcatccgagaggtctgggaatgcgcagtgcacccgcgtcttccatcgtgttaacattgcgcttctccggaaacattagc

SEQ ID NO: 247 - DNA, 102 bp, Artificial Sequence
  Synthetic Polynucleotide
acaaccgcgtgttacaaggccaggcatccgagaggtctgggaatgcgcagcagcatacggttcagccaggagtgaacattgcgcttctccggaaacattagc

SEQ ID NO: 248 - DNA, 102 bp, Artificial Sequence
  Synthetic Polynucleotide
acaaccgcgtgttacaaggccaggcatccgagaggtctgggaatgcgctctcagcgacatctttcgcctgacggaacattgcgcttctccggaaacattagc

SEQ ID NO: 249 - DNA, 102 bp, Artificial Sequence
  Synthetic Polynucleotide
acaaccgcgtgttacaaggccaggcatccgagaggtctgggaatgcggtttcaaggtcgcccgccagtttctgtttcattgcgcttctccggaaacattagc

SEQ ID NO: 250 - DNA, 102 bp, Artificial Sequence
  Synthetic Polynucleotide
acaaccgcgtgttacaaggccaggcatccgagaggtctgggaatgccacggtgctggaaccaccggcatagaagttcattgcgcttctccggaaacattagc

SEQ ID NO: 251 - DNA, 102 bp, Artificial Sequence
  Synthetic Polynucleotide
acaaccgcgtgttacaaggccaggcatccgagaggtctgggaatgcggtcccgttgataccaacagcataacctgtcattgcgcttctccggaaacattagc

SEQ ID NO: 252 - DNA, 102 bp, Artificial Sequence
  Synthetic Polynucleotide
acaaccgcgtgttacaaggccaggcatccgagaggtctgggaatgctgaaacgggcataaccgcgatccagatagtcattgcgcttctccggaaacattagc

SEQ ID NO: 253 - DNA, 102 bp, Artificial Sequence
  Synthetic Polynucleotide
acaaccgcgtgttacaaggccaggcatccgagaggtctgggaatgccggaacacgttgggtatcggtatcgacagtcattgcgcttctccggaaacattagc

SEQ ID NO: 254 - DNA, 102 bp, Artificial Sequence
  Synthetic Polynucleotide
acaaccgcgtgttacaaggccaggcatccgagaggtctgggaatgcacggtgaagtacgggttggttaccgacagtcattgcgcttctccggaaacattagc

SEQ ID NO: 255 - DNA, 102 bp, Artificial Sequence
  Synthetic Polynucleotide
acaaccgcgtgttacaaggccaggcatccgagaggtctgggaatgcacagctcacccggctcgatcttagtcagctcattgcgcttctccggaaacattagc

SEQ ID NO: 256 - DNA, 102 bp, Artificial Sequence
  Synthetic Polynucleotide
acaaccgcgtgttacaaggccaggcatccgagaggtctgggaatgctgttggtatagtcggacaggtcggcgtcatcattgcgcttctccggaaacattagc

SEQ ID NO: 257 - DNA, 102 bp, Artificial Sequence
  Synthetic Polynucleotide
acaaccgcgtgttacaaggccaggcatccgagaggtctgggaatgcggcgacacgctgaaggccttcgaaatgaatcattgcgcttctccggaaacattagc

SEQ ID NO: 258 - DNA, 102 bp, Artificial Sequence
  Synthetic Polynucleotide
acaaccgcgtgttacaaggccaggcatccgagaggtctgggaatgctggaaatgagagatcagttcgtcggtggtgcattgcgcttctccggaaacattagc

SEQ ID NO: 259 - DNA, 102 bp, Artificial Sequence
  Synthetic Polynucleotide
acaaccgcgtgttacaaggccaggcatccgagaggtctgggaatgcttgctggatttcagctgacacaccttcctgcattgcgcttctccggaaacattagc

SEQ ID NO: 260 - DNA, 102 bp, Artificial Sequence
  Synthetic Polynucleotide
acaaccgcgtgttacaaggccaggcatccgagaggtctgggaatgcgtcggcatcgttaatttcgggcatcgactgcattgcgcttctccggaaacattagc

SEQ ID NO: 261 - DNA, 102 bp, Artificial Sequence
  Synthetic Polynucleotide
acaaccgcgtgttacaaggccaggcatccgagaggtctgggaatgcactgctttcggaccaatggtattggactggcattgcgcttctccggaaacattagc

SEQ ID NO: 262 - DNA, 102 bp, Artificial Sequence
  Synthetic Polynucleotide
acaaccgcgtgttacaaggccaggcatccgagaggtctgggaatgcaccttgtagacgacatcaacctggtccgggcattgcgcttctccggaaacattagc

SEQ ID NO: 263 - DNA, 102 bp, Artificial Sequence
  Synthetic Polynucleotide
acaaccgcgtgttacaaggccaggcatccgagaggtctgggaatgctatccgatccaggaatggtcactttaccggcattgcgcttctccggaaacattagc

SEQ ID NO: 264 - DNA, 102 bp, Artificial Sequence
  Synthetic Polynucleotide
acaaccgcgtgttacaaggccaggcatccgagaggtctgggaatgctcactacgaacccttcagcaccgtatacggcattgcgcttctccggaaacattagc

SEQ ID NO: 265 - DNA, 102 bp, Artificial Sequence
  Synthetic Polynucleotide
acaaccgcgtgttacaaggccaggcatccgagaggtctgggaatgcagccatgcaccttccatctgacgcatttcgcattgcgcttctccggaaacattagc

SEQ ID NO: 266 - DNA, 102 bp, Artificial Sequence
  Synthetic Polynucleotide
acaaccgcgtgttacaaggccaggcatccgagaggtctgggaatgccccagacctgcacgcagcgagttatattcgcattgcgcttctccggaaacattagc

SEQ ID NO: 267 - DNA, 102 bp, Artificial Sequence
  Synthetic Polynucleotide
acaaccgcgtgttacaaggccaggcatccgagaggtctgggaatgcaactggaactgttctgccttgtctccatcgcattgcgcttctccggaaacattagc

SEQ ID NO: 268 - DNA, 102 bp, Artificial Sequence
  Synthetic Polynucleotide
acaaccgcgtgttacaaggccaggcatccgagaggtctgggaatgcatcttcatcattaaccgtgtcgcctgtgcgcattgcgcttctccggaaacattagc

SEQ ID NO: 269 - DNA, 102 bp, Artificial Sequence
  Synthetic Polynucleotide
acaaccgcgtgttacaaggccaggcatccgagaggtctgggaatgctccaaccatagttgaacgtgaagtcgtccgcattgcgcttctccggaaacattagc

SEQ ID NO: 270 - DNA, 102 bp, Artificial Sequence
  Synthetic Polynucleotide
acaaccgcgtgttacaaggccaggcatccgagaggtctgggaatgcccattgtaatgcgatacccgcagacatacgcattgcgcttctccggaaacattagc

SEQ ID NO: 271 - DNA, 102 bp, Artificial Sequence
  Synthetic Polynucleotide
acaaccgcgtgttacaaggccaggcatccgagaggtctgggaatgcatttacgatcgcctaccacgttccaccacgcattgcgcttctccggaaacattagc

SEQ ID NO: 272 - DNA, 102 bp, Artificial Sequence
  Synthetic Polynucleotide
acaaccgcgtgttacaaggccaggcatccgagaggtctgggaatgctggctggaatcccagtttgtatcccaaacgcattgcgcttctccggaaacattagc

SEQ ID NO: 273 - DNA, 102 bp, Artificial Sequence
  Synthetic Polynucleotide
acaaccgcgtgttacaaggccaggcatccgagaggtctgggaatgcacgctggcgctatatttaccgacgctgtagcattgcgcttctccggaaacattagc

SEQ ID NO: 274 - DNA, 102 bp, Artificial Sequence
  Synthetic Polynucleotide
acaaccgcgtgttacaaggccaggcatccgagaggtctgggaatgcaccgcctacagcatcatccgatttacacagcattgcgcttctccggaaacattagc

SEQ ID NO: 275 - DNA, 102 bp, Artificial Sequence
  Synthetic Polynucleotide
acaaccgcgtgttacaaggccaggcatccgagaggtctgggaatgcatctggcgtcagactgacctgggtagagtccattgcgcttctccggaaacattagc

SEQ ID NO: 276 - DNA, 102 bp, Artificial Sequence
  Synthetic Polynucleotide
acaaccgcgtgttacaaggccaggcatccgagaggtctgggaatgccgcgccgtcctgagtcgcacattcgtaatccattgcgcttctccggaaacattagc

SEQ ID NO: 277 - DNA, 102 bp, Artificial Sequence
  Synthetic Polynucleotide
acaaccgcgtgttacaaggccaggcatccgagaggtctgggaatgcacaacccatttgtgatcgtcatcgatcggccattgcgcttctccggaaacattagc

SEQ ID NO: 278 - DNA, 102 bp, Artificial Sequence
  Synthetic Polynucleotide
acaaccgcgtgttacaaggccaggcatccgagaggtctgggaatgcacccatagagtacagataacgccacatcgccattgcgcttctccggaaacattagc

SEQ ID NO: 279 - DNA, 102 bp, Artificial Sequence
  Synthetic Polynucleotide
acaaccgcgtgttacaaggccaggcatccgagaggtctgggaatgcataccaaagttgaagctaccggtgttgcgccattgcgcttctccggaaacattagc

SEQ ID NO: 280 - DNA, 102 bp, Artificial Sequence
  Synthetic Polynucleotide
acaaccgcgtgttacaaggccaggcatccgagaggtctgggaatgctatagaagagacgaccaccgaggcttacgccattgcgcttctccggaaacattagc

SEQ ID NO: 281 - DNA, 102 bp, Artificial Sequence
  Synthetic Polynucleotide
acaaccgcgtgttacaaggccaggcatccgagaggtctgggaatgcgtcatcttccatcttggtcactttggtgcccattgcgcttctccggaaacattagc

SEQ ID NO: 282 - DNA, 102 bp, Artificial Sequence
  Synthetic Polynucleotide
acaaccgcgtgttacaaggccaggcatccgagaggtctgggaatgccggatcttacgcacgtagaaacggttaccccattgcgcttctccggaaacattagc

SEQ ID NO: 283 - DNA, 102 bp, Artificial Sequence
  Synthetic Polynucleotide
acaaccgcgtgttacaaggccaggcatccgagaggtctgggaatgccaggacggcatctttcgaggtatcgttacccattgcgcttctccggaaacattagc

SEQ ID NO: 284 - DNA, 102 bp, Artificial Sequence
  Synthetic Polynucleotide
acaaccgcgtgttacaaggccaggcatccgagaggtctgggaatgcagaagcccagacgattcagacgctccttaccattgcgcttctccggaaacattagc

SEQ ID NO: 285 - DNA, 102 bp, Artificial Sequence
  Synthetic Polynucleotide
acaaccgcgtgttacaaggccaggcatccgagaggtctgggaatgctgacacgtgaaccatctgtcgggaagtaaccattgcgcttctccggaaacattagc

SEQ ID NO: 286 - DNA, 102 bp, Artificial Sequence
  Synthetic Polynucleotide
acaaccgcgtgttacaaggccaggcatccgagaggtctgggaatgcctgctaaacagcagcgacgctatgagcaaccattgcgcttctccggaaacattagc

SEQ ID NO: 287 - DNA, 102 bp, Artificial Sequence
  Synthetic Polynucleotide
acaaccgcgtgttacaaggccaggcatccgagaggtctgggaatgcgaggctgcatgttggacagggagttatgtacattgcgcttctccggaaacattagc

SEQ ID NO: 288 - DNA, 102 bp, Artificial Sequence
  Synthetic Polynucleotide
acaaccgcgtgttacaaggccaggcatccgagaggtctgggaatgccgggaagcccaacgtcacgtctgtaccatacattgcgcttctccggaaacattagc

SEQ ID NO: 289 - DNA, 102 bp, Artificial Sequence
  Synthetic Polynucleotide
acaaccgcgtgttacaaggccaggcatccgagaggtctgggaatgcccggatcataattactggcctgatgcgggacattgcgcttctccggaaacattagc

SEQ ID NO: 290 - DNA, 102 bp, Artificial Sequence
  Synthetic Polynucleotide
acaaccgcgtgttacaaggccaggcatccgagaggtctgggaatgcaagctgttatcctgatcagaggtgctcggacattgcgcttctccggaaacattagc

SEQ ID NO: 291 - DNA, 102 bp, Artificial Sequence
  Synthetic Polynucleotide
acaaccgcgtgttacaaggccaggcatccgagaggtctgggaatgcacctgaaccagaagggtatcaccatcacgacattgcgcttctccggaaacattagc

SEQ ID NO: 292 - DNA, 102 bp, Artificial Sequence
  Synthetic Polynucleotide
acaaccgcgtgttacaaggccaggcatccgagaggtctgggaatgcggcatctctttgccgcctaaaccatcaccacattgcgcttctccggaaacattagc

SEQ ID NO: 293 - DNA, 102 bp, Artificial Sequence
  Synthetic Polynucleotide
acaaccgcgtgttacaaggccaggcatccgagaggtctgggaatgcccagttatcctgctgcacaccagcctggaacattgcgcttctccggaaacattagc

SEQ ID NO: 294 - DNA, 102 bp, Artificial Sequence
  Synthetic Polynucleotide
acaaccgcgtgttacaaggccaggcatccgagaggtctgggaatgcgcggataggcataaccatagcgaccgagaacattgcgcttctccggaaacattagc

SEQ ID NO: 295 - DNA, 102 bp, Artificial Sequence
  Synthetic Polynucleotide
acaaccgcgtgttacaaggccaggcatccgagaggtctgggaatgccaaggttgccgctcacttcaacgccagaaacattgcgcttctccggaaacattagc

SEQ ID NO: 296 - DNA, 102 bp, Artificial Sequence
  Synthetic Polynucleotide
acaaccgcgtgttacaaggccaggcatccgagaggtctgggaatgcgcgaacatcctcaaagttgccggtagcaaacattgcgcttctccggaaacattagc

SEQ ID NO: 297 - DNA, 102 bp, Artificial Sequence
  Synthetic Polynucleotide
acaaccgcgtgttacaaggccaggcatccgagaggtctgggaatgcacgtgggcttgcacgttcaaaccagtcactcattgcgcttctccggaaacattagc

SEQ ID NO: 298 - DNA, 102 bp, Artificial Sequence
  Synthetic Polynucleotide
acaaccgcgtgttacaaggccaggcatccgagaggtctgggaatgccctgtgaaagcgcattacagagctgttgtgcattgcgcttctccggaaacattagc

SEQ ID NO: 299 - DNA, 102 bp, Artificial Sequence
  Synthetic Polynucleotide
acaaccgcgtgttacaaggccaggcatccgagaggtctgggaatgcttgcgctttcaattgcgcgtactgatccagcattgcgcttctccggaaacattagc

SEQ ID NO: 300 - DNA, 102 bp, Artificial Sequence
  Synthetic Polynucleotide
acaaccgcgtgttacaaggccaggcatccgagaggtctgggaatgcgcgcttgtggaggatagtcggaatagctgccattgcgcttctccggaaacattagc

SEQ ID NO: 301 - DNA, 102 bp, Artificial Sequence
  Synthetic Polynucleotide
acaaccgcgtgttacaaggccaggcatccgagaggtctgggaatgcaggaatttggtccggtccgcctgtaatgaccattgcgcttctccggaaacattagc

SEQ ID NO: 302 - DNA, 102 bp, Artificial Sequence
  Synthetic Polynucleotide
acaaccgcgtgttacaaggccaggcatccgagaggtctgggaatgccgagcgtgctaacacctgttcgcggctaaccattgcgcttctccggaaacattagc

SEQ ID NO: 303 - DNA, 102 bp, Artificial Sequence
  Synthetic Polynucleotide
acaaccgcgtgttacaaggccaggcatccgagaggtctgggaatgcgcattacctccacgccaggcaatcaccagacattgcgcttctccggaaacattagc

SEQ ID NO: 304 - DNA, 102 bp, Artificial Sequence
  Synthetic Polynucleotide
acaaccgcgtgttacaaggccaggcatccgagaggtctgggaatgcgcaaaggcaagttcagtgttggcgggagaacattgcgcttctccggaaacattagc

SEQ ID NO: 305 - DNA, 102 bp, Artificial Sequence
  Synthetic Polynucleotide
acaaccgcgtgttacaaggccaggcatccgagaggtctgggaatgcgatatcgcggatatgcagcagccagttgttcattgcgcttctccggaaacattagc

SEQ ID NO: 306 - DNA, 102 bp, Artificial Sequence
  Synthetic Polynucleotide
acaaccgcgtgttacaaggccaggcatccgagaggtctgggaatgcgcagttcaggtcagtgtgaatgaccaggttcattgcgcttctccggaaacattagc

SEQ ID NO: 307 - DNA, 102 bp, Artificial Sequence
  Synthetic Polynucleotide
acaaccgcgtgttacaaggccaggcatccgagaggtctgggaatgccattacggtgaacaaagagttcgcccggctcattgcgcttctccggaaacattagc

SEQ ID NO: 308 - DNA, 102 bp, Artificial Sequence
  Synthetic Polynucleotide
acaaccgcgtgttacaaggccaggcatccgagaggtctgggaatgcttgtggttggcgtgtttcagcttgaggttgcattgcgcttctccggaaacattagc

SEQ ID NO: 309 - DNA, 102 bp, Artificial Sequence
  Synthetic Polynucleotide
acaaccgcgtgttacaaggccaggcatccgagaggtctgggaatgcccggttaaacgttctgcaggaacgcgactgcattgcgcttctccggaaacattagc

SEQ ID NO: 310 - DNA, 102 bp, Artificial Sequence
  Synthetic Polynucleotide
acaaccgcgtgttacaaggccaggcatccgagaggtctgggaatgccctgttccatgacgttcagttcacacaaggcattgcgcttctccggaaacattagc

SEQ ID NO: 311 - DNA, 102 bp, Artificial Sequence
  Synthetic Polynucleotide
acaaccgcgtgttacaaggccaggcatccgagaggtctgggaatgctcgagtacatccactgcatactgaaccacgcattgcgcttctccggaaacattagc

SEQ ID NO: 312 - DNA, 102 bp, Artificial Sequence
  Synthetic Polynucleotide
acaaccgcgtgttacaaggccaggcatccgagaggtctgggaatgccgtttccacgctgattgcataatggtggagcattgcgcttctccggaaacattagc

SEQ ID NO: 313 - DNA, 102 bp, Artificial Sequence
  Synthetic Polynucleotide
acaaccgcgtgttacaaggccaggcatccgagaggtctgggaatgccccgtgacggtaacgttgctcaagggtttccattgcgcttctccggaaacattagc

SEQ ID NO: 314 - DNA, 102 bp, Artificial Sequence
  Synthetic Polynucleotide
acaaccgcgtgttacaaggccaggcatccgagaggtctgggaatgcccgccgcaaccgtagtggccacagataatacattgcgcttctccggaaacattagc

SEQ ID NO: 315 - DNA, 102 bp, Artificial Sequence
  Synthetic Polynucleotide
acaaccgcgtgttacaaggccaggcatccgagaggtctgggaatgcggtggcggtaacatccagatcacgcagcaacattgcgcttctccggaaacattagc

SEQ ID NO: 316 - DNA, 102 bp, Artificial Sequence
  Synthetic Polynucleotide
acaaccgcgtgttacaaggccaggcatccgagaggtctgggaatgctaatgattctcgtcatagtgccaggcccgtcattgcgcttctccggaaacattagc

SEQ ID NO: 317 - DNA, 102 bp, Artificial Sequence
  Synthetic Polynucleotide
acaaccgcgtgttacaaggccaggcatccgagaggtctgggaatgccagaaacaacgccgcgatgacgacgggtatcattgcgcttctccggaaacattagc

SEQ ID NO: 318 - DNA, 102 bp, Artificial Sequence
  Synthetic Polynucleotide
acaaccgcgtgttacaaggccaggcatccgagaggtctgggaatgcgccagcatgcagaccaccagcgttacaatgcattgcgcttctccggaaacattagc

SEQ ID NO: 319 - DNA, 102 bp, Artificial Sequence
  Synthetic Polynucleotide
acaaccgcgtgttacaaggccaggcatccgagaggtctgggaatgcagagttacgccagattgctgcggaacctggcattgcgcttctccggaaacattagc

SEQ ID NO: 320 - DNA, 102 bp, Artificial Sequence
  Synthetic Polynucleotide
acaaccgcgtgttacaaggccaggcatccgagaggtctgggaatgccgaagcccaaagtgagatttcaaccagcggcattgcgcttctccggaaacattagc

SEQ ID NO: 321 - DNA, 102 bp, Artificial Sequence
  Synthetic Polynucleotide
acaaccgcgtgttacaaggccaggcatccgagaggtctgggaatgcgtaacaacaagcaagcaaagaccggtaccgcattgcgcttctccggaaacattagc

SEQ ID NO: 322 - DNA, 102 bp, Artificial Sequence
  Synthetic Polynucleotide
acaaccgcgtgttacaaggccaggcatccgagaggtctgggaatgcggatcatgacatagagcagccatattgcgccattgcgcttctccggaaacattagc

SEQ ID NO: 323 - DNA, 102 bp, Artificial Sequence
  Synthetic Polynucleotide
acaaccgcgtgttacaaggccaggcatccgagaggtctgggaatgctaccaccgtgtcctggaattaaatgaccgccattgcgcttctccggaaacattagc

SEQ ID NO: 324 - DNA, 102 bp, Artificial Sequence
  Synthetic Polynucleotide
acaaccgcgtgttacaaggccaggcatccgagaggtctgggaatgctttgccaaacatatatgcgccggagtcagccattgcgcttctccggaaacattagc

SEQ ID NO: 325 - DNA, 102 bp, Artificial Sequence
  Synthetic Polynucleotide
acaaccgcgtgttacaaggccaggcatccgagaggtctgggaatgcccgctgcagtagcgagtccaccgataaagccattgcgcttctccggaaacattagc

SEQ ID NO: 326 - DNA, 102 bp, Artificial Sequence
  Synthetic Polynucleotide
acaaccgcgtgttacaaggccaggcatccgagaggtctgggaatgcacgcttaaacatactctcggtcagatcgcccattgcgcttctccggaaacattagc

SEQ ID NO: 327 - DNA, 102 bp, Artificial Sequence
  Synthetic Polynucleotide
acaaccgcgtgttacaaggccaggcatccgagaggtctgggaatgcgcatcagcgccaacaataacccgcataacacattgcgcttctccggaaacattagc

SEQ ID NO: 328 - DNA, 102 bp, Artificial Sequence
  Synthetic Polynucleotide
acaaccgcgtgttacaaggccaggcatccgagaggtctgggaatgcgcgacgtcgagattcgcccacatgccataacattgcgcttctccggaaacattagc

SEQ ID NO: 329 - DNA, 102 bp, Artificial Sequence
  Synthetic Polynucleotide
acaaccgcgtgttacaaggccaggcatccgagaggtctgggaatgcagcaccagcaatagcgcgacaatccaccaacattgcgcttctccggaaacattagc

SEQ ID NO: 330 - DNA, 102 bp, Artificial Sequence
  Synthetic Polynucleotide
acaaccgcgtgttacaaggccaggcatccgagaggtctgggaatgcctgaggctaacgctgcgacaatagagcaaacattgcgcttctccggaaacattagc

SEQ ID NO: 331 - DNA, 102 bp, Artificial Sequence
  Synthetic Polynucleotide
acaaccgcgtgttacaaggccaggcatccgagaggtctgggaatgcgaacgcgaccgtagtggatttcgccggtttcattgcgcttctccggaaacattagc

SEQ ID NO: 332 - DNA, 102 bp, Artificial Sequence
  Synthetic Polynucleotide
acaaccgcgtgttacaaggccaggcatccgagaggtctgggaatgcccggaatccagcagggcgatcacctgatttcattgcgcttctccggaaacattagc

SEQ ID NO: 333 - DNA, 102 bp, Artificial Sequence
  Synthetic Polynucleotide
acaaccgcgtgttacaaggccaggcatccgagaggtctgggaatgcgtgccttcatcaacatatgcgccgatgttgcattgcgcttctccggaaacattagc

SEQ ID NO: 334 - DNA, 102 bp, Artificial Sequence
  Synthetic Polynucleotide
acaaccgcgtgttacaaggccaggcatccgagaggtctgggaatgccaaccactgatgcgtcacccactgaccgtccattgcgcttctccggaaacattagc

SEQ ID NO: 335 - DNA, 102 bp, Artificial Sequence
  Synthetic Polynucleotide
acaaccgcgtgttacaaggccaggcatccgagaggtctgggaatgcgtaacggtgtctgcattggctggcgtgatccattgcgcttctccggaaacattagc

SEQ ID NO: 336 - DNA, 102 bp, Artificial Sequence
  Synthetic Polynucleotide
acaaccgcgtgttacaaggccaggcatccgagaggtctgggaatgcaaccgcacagtagaggctgtatttgccatccattgcgcttctccggaaacattagc

SEQ ID NO: 337 - DNA, 102 bp, Artificial Sequence
  Synthetic Polynucleotide
acaaccgcgtgttacaaggccaggcatccgagaggtctgggaatgcagtcgatggtacgcagcagttcgttaatgccattgcgcttctccggaaacattagc

SEQ ID NO: 338 - DNA, 102 bp, Artificial Sequence
  Synthetic Polynucleotide
acaaccgcgtgttacaaggccaggcatccgagaggtctgggaatgcaatacgggtgctctgaccaatgtatacgcccattgcgcttctccggaaacattagc

SEQ ID NO: 339 - DNA, 102 bp, Artificial Sequence
  Synthetic Polynucleotide
acaaccgcgtgttacaaggccaggcatccgagaggtctgggaatgcacttcagagcgcgcgccgatgaagcaattacattgcgcttctccggaaacattagc

SEQ ID NO: 340 - DNA, 102 bp, Artificial Sequence
  Synthetic Polynucleotide
acaaccgcgtgttacaaggccaggcatccgagaggtctgggaatgcgacggcatcagcacggtgttacgggcaatacattgcgcttctccggaaacattagc

SEQ ID NO: 341 - DNA, 102 bp, Artificial Sequence
  Synthetic Polynucleotide
acaaccgcgtgttacaaggccaggcatccgagaggtctgggaatgccttcgtcgtagtcggcgaatttcatcggcacattgcgcttctccggaaacattagc

SEQ ID NO: 342 - DNA, 102 bp, Artificial Sequence
  Synthetic Polynucleotide
acaaccgcgtgttacaaggccaggcatccgagaggtctgggaatgctggcacaacgcggaagccttctttctggaacattgcgcttctccggaaacattagc

SEQ ID NO: 343 - DNA, 102 bp, Artificial Sequence
  Synthetic Polynucleotide
acaaccgcgtgttacaaggccaggcatccgagaggtctgggaatgccacaagaaccgacggtcgcccaggtatcaacattgcgcttctccggaaacattagc

SEQ ID NO: 344 - DNA, 102 bp, Artificial Sequence
  Synthetic Polynucleotide
acaaccgcgtgttacaaggccaggcatccgagaggtctgggaatgcccggtaaaccggcaccttgccatagaagttcattgcgcttctccggaaacattagc

SEQ ID NO: 345 - DNA, 102 bp, Artificial Sequence
  Synthetic Polynucleotide
acaaccgcgtgttacaaggccaggcatccgagaggtctgggaatgcggtcgacaggatacgcgtcaataccgccttcattgcgcttctccggaaacattagc

SEQ ID NO: 346 - DNA, 102 bp, Artificial Sequence
  Synthetic Polynucleotide
acaaccgcgtgttacaaggccaggcatccgagaggtctgggaatgcgctgtggctggtcatacccggtgaggtattcattgcgcttctccggaaacattagc

SEQ ID NO: 347 - DNA, 102 bp, Artificial Sequence
  Synthetic Polynucleotide
acaaccgcgtgttacaaggccaggcatccgagaggtctgggaatgcctgtccatcgctgtccagcataacgtcaatcattgcgcttctccggaaacattagc

SEQ ID NO: 348 - DNA, 102 bp, Artificial Sequence
  Synthetic Polynucleotide
acaaccgcgtgttacaaggccaggcatccgagaggtctgggaatgctcgcctcataatcatagaaggttccggacgcattgcgcttctccggaaacattagc

SEQ ID NO: 349 - DNA, 102 bp, Artificial Sequence
  Synthetic Polynucleotide
acaaccgcgtgttacaaggccaggcatccgagaggtctgggaatgccctttgcaacctaacgtcgtccatgctttccattgcgcttctccggaaacattagc

SEQ ID NO: 350 - DNA, 102 bp, Artificial Sequence
  Synthetic Polynucleotide
acaaccgcgtgttacaaggccaggcatccgagaggtctgggaatgcccgcgaccgtgtagcgcgataaacactttccattgcgcttctccggaaacattagc

SEQ ID NO: 351 - DNA, 102 bp, Artificial Sequence
  Synthetic Polynucleotide
acaaccgcgtgttacaaggccaggcatccgagaggtctgggaatgcgacattcccacactggaaccttcgcggctccattgcgcttctccggaaacattagc

SEQ ID NO: 352 - DNA, 102 bp, Artificial Sequence
  Synthetic Polynucleotide
acaaccgcgtgttacaaggccaggcatccgagaggtctgggaatgcttcttcaccgagtatcgcaaccgtgaactccattgcgcttctccggaaacattagc

SEQ ID NO: 353 - DNA, 102 bp, Artificial Sequence
  Synthetic Polynucleotide
acaaccgcgtgttacaaggccaggcatccgagaggtctgggaatgcaaccggcaaacccagagcagaaatttctgccattgcgcttctccggaaacattagc

SEQ ID NO: 354 - DNA, 102 bp, Artificial Sequence
  Synthetic Polynucleotide
acaaccgcgtgttacaaggccaggcatccgagaggtctgggaatgctaatgcctgcaaattggcctcttgtgacgccattgcgcttctccggaaacattagc

SEQ ID NO: 355 - DNA, 102 bp, Artificial Sequence
  Synthetic Polynucleotide
acaaccgcgtgttacaaggccaggcatccgagaggtctgggaatgcatccattgaaagcgcagatgccatcactcccattgcgcttctccggaaacattagc

SEQ ID NO: 356 - DNA, 102 bp, Artificial Sequence
  Synthetic Polynucleotide
acaaccgcgtgttacaaggccaggcatccgagaggtctgggaatgctagtccgccagttccagaattcgtactacccattgcgcttctccggaaacattagc

SEQ ID NO: 357 - DNA, 102 bp, Artificial Sequence
  Synthetic Polynucleotide
acaaccgcgtgttacaaggccaggcatccgagaggtctgggaatgcgcccatcgacttcagttgcgtcacgtcgaccattgcgcttctccggaaacattagc

SEQ ID NO: 358 - DNA, 102 bp, Artificial Sequence
  Synthetic Polynucleotide
acaaccgcgtgttacaaggccaggcatccgagaggtctgggaatgcggctaacaccgctgcgccagaattcagagacattgcgcttctccggaaacattagc

SEQ ID NO: 359 - DNA, 102 bp, Artificial Sequence
  Synthetic Polynucleotide
acaaccgcgtgttacaaggccaggcatccgagaggtctgggaatgccggtataaggcaagcccatcagctcgagcacattgcgcttctccggaaacattagc

SEQ ID NO: 360 - DNA, 102 bp, Artificial Sequence
  Synthetic Polynucleotide
acaaccgcgtgttacaaggccaggcatccgagaggtctgggaatgccacgttgttcactaccacgccctgatctttcattgcgcttctccggaaacattagc

SEQ ID NO: 361 - DNA, 102 bp, Artificial Sequence
  Synthetic Polynucleotide
acaaccgcgtgttacaaggccaggcatccgagaggtctgggaatgcgttcaggttaaccagcgcaccaccggagttcattgcgcttctccggaaacattagc

SEQ ID NO: 362 - DNA, 102 bp, Artificial Sequence
  Synthetic Polynucleotide
acaaccgcgtgttacaaggccaggcatccgagaggtctgggaatgcctgcagttccaggttcacgttaacctgcttcattgcgcttctccggaaacattagc

SEQ ID NO: 363 - DNA, 102 bp, Artificial Sequence
  Synthetic Polynucleotide
acaaccgcgtgttacaaggccaggcatccgagaggtctgggaatgcgcagcggaggaattaggcagaacctggcttcattgcgcttctccggaaacattagc

SEQ ID NO: 364 - DNA, 102 bp, Artificial Sequence
  Synthetic Polynucleotide
acaaccgcgtgttacaaggccaggcatccgagaggtctgggaatgcactcagagccagtgcactcagtgctaatgtcattgcgcttctccggaaacattagc

SEQ ID NO: 365 - DNA, 102 bp, Artificial Sequence
  Synthetic Polynucleotide
acaaccgcgtgttacaaggccaggcatccgagaggtctgggaatgctgttgctcatctcagcgccttcaatgccgtcattgcgcttctccggaaacattagc

SEQ ID NO: 366 - DNA, 102 bp, Artificial Sequence
  Synthetic Polynucleotide
acaaccgcgtgttacaaggccaggcatccgagaggtctgggaatgctgaatgttgagtgccagcacagacggtttgcattgcgcttctccggaaacattagc

SEQ ID NO: 367 - DNA, 102 bp, Artificial Sequence
  Synthetic Polynucleotide
acaaccgcgtgttacaaggccaggcatccgagaggtctgggaatgcgccggaacccagcgccatgaatttctgttgcattgcgcttctccggaaacattagc

SEQ ID NO: 368 - DNA, 102 bp, Artificial Sequence
  Synthetic Polynucleotide
acaaccgcgtgttacaaggccaggcatccgagaggtctgggaatgcatggagctggaatcaacctgattctggctgcattgcgcttctccggaaacattagc

SEQ ID NO: 369 - DNA, 102 bp, Artificial Sequence
  Synthetic Polynucleotide
acaaccgcgtgttacaaggccaggcatccgagaggtctgggaatgcataatacccagctcaccgcgtttcacctggcattgcgcttctccggaaacattagc

SEQ ID NO: 370 - DNA, 102 bp, Artificial Sequence
  Synthetic Polynucleotide
acaaccgcgtgttacaaggccaggcatccgagaggtctgggaatgcggcaaagctgctgatcggcttaccgttcagcattgcgcttctccggaaacattagc

SEQ ID NO: 371 - DNA, 102 bp, Artificial Sequence
  Synthetic Polynucleotide
acaaccgcgtgttacaaggccaggcatccgagaggtctgggaatgcctgggcgtcaactttcatcgctttcgccagcattgcgcttctccggaaacattagc

SEQ ID NO: 372 - DNA, 102 bp, Artificial Sequence
  Synthetic Polynucleotide
acaaccgcgtgttacaaggccaggcatccgagaggtctgggaatgcgcatctgctgggctgtcgttgctgaagaagcattgcgcttctccggaaacattagc

SEQ ID NO: 373 - DNA, 102 bp, Artificial Sequence
  Synthetic Polynucleotide
acaaccgcgtgttacaaggccaggcatccgagaggtctgggaatgcagcgcagagacaatcccggaagttaccgtccattgcgcttctccggaaacattagc

SEQ ID NO: 374 - DNA, 102 bp, Artificial Sequence
  Synthetic Polynucleotide
acaaccgcgtgttacaaggccaggcatccgagaggtctgggaatgccgggttctggatttggatcagcgcgatatccattgcgcttctccggaaacattagc

SEQ ID NO: 375 - DNA, 102 bp, Artificial Sequence
  Synthetic Polynucleotide
acaaccgcgtgttacaaggccaggcatccgagaggtctgggaatgcggtgcgaggatcgcggtgttgataccgatccattgcgcttctccggaaacattagc

SEQ ID NO: 376 - DNA, 102 bp, Artificial Sequence
  Synthetic Polynucleotide
acaaccgcgtgttacaaggccaggcatccgagaggtctgggaatgcactgcattaacaggtagatggtgctgtcgccattgcgcttctccggaaacattagc

SEQ ID NO: 377 - DNA, 102 bp, Artificial Sequence
  Synthetic Polynucleotide
acaaccgcgtgttacaaggccaggcatccgagaggtctgggaatgccaacaacgtggttgttggtgacgacatagccattgcgcttctccggaaacattagc

SEQ ID NO: 378 - DNA, 102 bp, Artificial Sequence
  Synthetic Polynucleotide
acaaccgcgtgttacaaggccaggcatccgagaggtctgggaatgccggccatcgctcagttgaactttaatgacccattgcgcttctccggaaacattagc

SEQ ID NO: 379 - DNA, 102 bp, Artificial Sequence
  Synthetic Polynucleotide
acaaccgcgtgttacaaggccaggcatccgagaggtctgggaatgcacgttaatgctgaccactgaaggcatcacccattgcgcttctccggaaacattagc

SEQ ID NO: 380 - DNA, 102 bp, Artificial Sequence
  Synthetic Polynucleotide
acaaccgcgtgttacaaggccaggcatccgagaggtctgggaatgccactgcctgctggttcgcgccaataatcaccattgcgcttctccggaaacattagc

SEQ ID NO: 381 - DNA, 102 bp, Artificial Sequence
  Synthetic Polynucleotide
acaaccgcgtgttacaaggccaggcatccgagaggtctgggaatgcacgcgcagtgcatcagaatccgccatcttacattgcgcttctccggaaacattagc

SEQ ID NO: 382 - DNA, 102 bp, Artificial Sequence
  Synthetic Polynucleotide
acaaccgcgtgttacaaggccaggcatccgagaggtctgggaatgcaccaaacgggttaccaatcgctacggtgtacattgcgcttctccggaaacattagc

SEQ ID NO: 383 - DNA, 102 bp, Artificial Sequence
  Synthetic Polynucleotide
acaaccgcgtgttacaaggccaggcatccgagaggtctgggaatgcggcatacgcggcgtattaacggttgtgctacattgcgcttctccggaaacattagc

SEQ ID NO: 384 - DNA, 102 bp, Artificial Sequence
  Synthetic Polynucleotide
acaaccgcgtgttacaaggccaggcatccgagaggtctgggaatgcgcagtaagcccagggtcagtttgctgcctacattgcgcttctccggaaacattagc

SEQ ID NO: 385 - DNA, 102 bp, Artificial Sequence
  Synthetic Polynucleotide
acaaccgcgtgttacaaggccaggcatccgagaggtctgggaatgcgcggatctttgccaaccatcttcgcgtcgacattgcgcttctccggaaacattagc

SEQ ID NO: 386 - DNA, 102 bp, Artificial Sequence
  Synthetic Polynucleotide
acaaccgcgtgttacaaggccaggcatccgagaggtctgggaatgctggcagaacggagagctctggaacggagaacattgcgcttctccggaaacattagc

SEQ ID NO: 387 - DNA, 102 bp, Artificial Sequence
  Synthetic Polynucleotide
acaaccgcgtgttacaaggccaggcatccgagaggtctgggaatgcctggcagaacggagaatcatcaccgaagaacattgcgcttctccggaaacattagc

SEQ ID NO: 388 - DNA, 102 bp, Artificial Sequence
  Synthetic Polynucleotide
acaaccgcgtgttacaaggccaggcatccgagaggtctgggaatgcgccgttgcagagagcggagataacgccaaacattgcgcttctccggaaacattagc

SEQ ID NO: 389 - DNA, 102 bp, Artificial Sequence
  Synthetic Polynucleotide
acaaccgcgtgttacaaggccaggcatccgagaggtctgggaatgccgatggtcatatcgccttcgttcacctgatcattgcgcttctccggaaacattagc

SEQ ID NO: 390 - DNA, 102 bp, Artificial Sequence
  Synthetic Polynucleotide
acaaccgcgtgttacaaggccaggcatccgagaggtctgggaatgcagattcgggttatcttcgtcagcgatcaggcattgcgcttctccggaaacattagc

SEQ ID NO: 391 - DNA, 102 bp, Artificial Sequence
  Synthetic Polynucleotide
acaaccgcgtgttacaaggccaggcatccgagaggtctgggaatgcagatactaaaggaagaaccgcaaccgcaggcattgcgcttctccggaaacattagc

SEQ ID NO: 392 - DNA, 102 bp, Artificial Sequence
  Synthetic Polynucleotide
acaaccgcgtgttacaaggccaggcatccgagaggtctgggaatgcaactttgttggctgctgcgtcggtaaactccattgcgcttctccggaaacattagc

SEQ ID NO: 393 - DNA, 102 bp, Artificial Sequence
  Synthetic Polynucleotide
acaaccgcgtgttacaaggccaggcatccgagaggtctgggaatgcaccttcggtataatcaacggaaccgccgaccattgcgcttctccggaaacattagc

SEQ ID NO: 394 - DNA, 102 bp, Artificial Sequence
  Synthetic Polynucleotide
acaaccgcgtgttacaaggccaggcatccgagaggtctgggaatgccgcgttcgggttggtcacgatgaaacgagacattgcgcttctccggaaacattagc

SEQ ID NO: 395 - DNA, 102 bp, Artificial Sequence
  Synthetic Polynucleotide
acaaccgcgtgttacaaggccaggcatccgagaggtctgggaatgcaaggtgaaaccatactggaagccgctgcaacattgcgcttctccggaaacattagc

SEQ ID NO: 396 - DNA, 102 bp, Artificial Sequence
  Synthetic Polynucleotide
acaaccgcgtgttacaaggccaggcatccgagaggtctgggaatgcgccctgcaacttcaggccattcagatagttcattgcgcttctccggaaacattagc

SEQ ID NO: 397 - DNA, 102 bp, Artificial Sequence
  Synthetic Polynucleotide
acaaccgcgtgttacaaggccaggcatccgagaggtctgggaatgccagtctggaacaggctgtcagtaccggcttcattgcgcttctccggaaacattagc

SEQ ID NO: 398 - DNA, 102 bp, Artificial Sequence
  Synthetic Polynucleotide
acaaccgcgtgttacaaggccaggcatccgagaggtctgggaatgcgctgaccatattcaacaggccgccaggactcattgcgcttctccggaaacattagc

SEQ ID NO: 399 - DNA, 102 bp, Artificial Sequence
  Synthetic Polynucleotide
acaaccgcgtgttacaaggccaggcatccgagaggtctgggaatgccaccaccacgccaggtaaactgtttgtcatcattgcgcttctccggaaacattagc

SEQ ID NO: 400 - DNA, 102 bp, Artificial Sequence
  Synthetic Polynucleotide
acaaccgcgtgttacaaggccaggcatccgagaggtctgggaatgccgtcgtaaccaaaccaggcgttgatgtcatcattgcgcttctccggaaacattagc

SEQ ID NO: 401 - DNA, 102 bp, Artificial Sequence
  Synthetic Polynucleotide
acaaccgcgtgttacaaggccaggcatccgagaggtctgggaatgcgtaaagcacggaaaccgggccacgcataatcattgcgcttctccggaaacattagc

SEQ ID NO: 402 - DNA, 102 bp, Artificial Sequence
  Synthetic Polynucleotide
acaaccgcgtgttacaaggccaggcatccgagaggtctgggaatgccggtagcagactgtcgcgccgcaatagttgcattgcgcttctccggaaacattagc

SEQ ID NO: 403 - DNA, 102 bp, Artificial Sequence
  Synthetic Polynucleotide
acaaccgcgtgttacaaggccaggcatccgagaggtctgggaatgccgtcccggcaacgcggttaagagattcttgcattgcgcttctccggaaacattagc

SEQ ID NO: 404 - DNA, 102 bp, Artificial Sequence
  Synthetic Polynucleotide
acaaccgcgtgttacaaggccaggcatccgagaggtctgggaatgcccgctttcgcttcgatttctacgccacgtgcattgcgcttctccggaaacattagc

SEQ ID NO: 405 - DNA, 102 bp, Artificial Sequence
  Synthetic Polynucleotide
acaaccgcgtgttacaaggccaggcatccgagaggtctgggaatgcgtcgatatcgccagtggcaaacttgctctgcattgcgcttctccggaaacattagc

SEQ ID NO: 406 - DNA, 102 bp, Artificial Sequence
  Synthetic Polynucleotide
acaaccgcgtgttacaaggccaggcatccgagaggtctgggaatgctacgtgccagataatggcctttatccgctgcattgcgcttctccggaaacattagc

SEQ ID NO: 407 - DNA, 102 bp, Artificial Sequence
  Synthetic Polynucleotide
acaaccgcgtgttacaaggccaggcatccgagaggtctgggaatgctcggagcagacgccgtaaccataaacgctgcattgcgcttctccggaaacattagc

SEQ ID NO: 408 - DNA, 102 bp, Artificial Sequence
  Synthetic Polynucleotide
acaaccgcgtgttacaaggccaggcatccgagaggtctgggaatgcaggtagtatcggtggtgtattccgcatcggcattgcgcttctccggaaacattagc

SEQ ID NO: 409 - DNA, 102 bp, Artificial Sequence
  Synthetic Polynucleotide
acaaccgcgtgttacaaggccaggcatccgagaggtctgggaatgcatacgcataaagtcgacaccggtcagcaggcattgcgcttctccggaaacattagc

SEQ ID NO: 410 - DNA, 102 bp, Artificial Sequence
  Synthetic Polynucleotide
acaaccgcgtgttacaaggccaggcatccgagaggtctgggaatgcgacttcggctgatgcagcgccatctcttcgcattgcgcttctccggaaacattagc

SEQ ID NO: 411 - DNA, 102 bp, Artificial Sequence
  Synthetic Polynucleotide
acaaccgcgtgttacaaggccaggcatccgagaggtctgggaatgcgccggatctttggcattgaagtcgaaatcgcattgcgcttctccggaaacattagc

SEQ ID NO: 412 - DNA, 102 bp, Artificial Sequence
  Synthetic Polynucleotide
acaaccgcgtgttacaaggccaggcatccgagaggtctgggaatgccacgatcgaacaggttgttaacatgcagcgcattgcgcttctccggaaacattagc

SEQ ID NO: 413 - DNA, 102 bp, Artificial Sequence
  Synthetic Polynucleotide
acaaccgcgtgttacaaggccaggcatccgagaggtctgggaatgctcattaaagtctgtcggcagacgcttaccgcattgcgcttctccggaaacattagc

SEQ ID NO: 414 - DNA, 102 bp, Artificial Sequence
  Synthetic Polynucleotide
acaaccgcgtgttacaaggccaggcatccgagaggtctgggaatgccgcgttccagcatatacgggtcaatgaccgcattgcgcttctccggaaacattagc

SEQ ID NO: 415 - DNA, 102 bp, Artificial Sequence
  Synthetic Polynucleotide
acaaccgcgtgttacaaggccaggcatccgagaggtctgggaatgcatacacggcaccagtaactacaatcggacgcattgcgcttctccggaaacattagc

SEQ ID NO: 416 - DNA, 102 bp, Artificial Sequence
  Synthetic Polynucleotide
acaaccgcgtgttacaaggccaggcatccgagaggtctgggaatgcccagtcataacgaccgcctagggtgaccagcattgcgcttctccggaaacattagc

SEQ ID NO: 417 - DNA, 102 bp, Artificial Sequence
  Synthetic Polynucleotide
acaaccgcgtgttacaaggccaggcatccgagaggtctgggaatgcaccatccttcccaacttgcgaagaaggttccattgcgcttctccggaaacattagc

SEQ ID NO: 418 - DNA, 102 bp, Artificial Sequence
  Synthetic Polynucleotide
acaaccgcgtgttacaaggccaggcatccgagaggtctgggaatgccgcaggtgcagcggtaacggtgatagtgtccattgcgcttctccggaaacattagc

SEQ ID NO: 419 - DNA, 102 bp, Artificial Sequence
  Synthetic Polynucleotide
acaaccgcgtgttacaaggccaggcatccgagaggtctgggaatgcaattcgtgatcgaagctgtagccgaccatccattgcgcttctccggaaacattagc

SEQ ID NO: 420 - DNA, 102 bp, Artificial Sequence
  Synthetic Polynucleotide
acaaccgcgtgttacaaggccaggcatccgagaggtctgggaatgcgaagcagccataagtgttaaagcagctggccattgcgcttctccggaaacattagc

SEQ ID NO: 421 - DNA, 102 bp, Artificial Sequence
  Synthetic Polynucleotide
acaaccgcgtgttacaaggccaggcatccgagaggtctgggaatgctcccactttaaaggagttagccggatcacccattgcgcttctccggaaacattagc

SEQ ID NO: 422 - DNA, 102 bp, Artificial Sequence
  Synthetic Polynucleotide
acaaccgcgtgttacaaggccaggcatccgagaggtctgggaatgcttagaaacggaaggttgcggttgcaacgaccattgcgcttctccggaaacattagc

SEQ ID NO: 423 - DNA, 102 bp, Artificial Sequence
  Synthetic Polynucleotide
acaaccgcgtgttacaaggccaggcatccgagaggtctgggaatgccaccggattgtacagattgagcagtggcaccattgcgcttctccggaaacattagc

SEQ ID NO: 424 - DNA, 102 bp, Artificial Sequence
  Synthetic Polynucleotide
acaaccgcgtgttacaaggccaggcatccgagaggtctgggaatgcgccaggtgaacgccggtgcaatagcataaccattgcgcttctccggaaacattagc

SEQ ID NO: 425 - DNA, 102 bp, Artificial Sequence
  Synthetic Polynucleotide
acaaccgcgtgttacaaggccaggcatccgagaggtctgggaatgccgcaagaccggtcaggcgataagagtaaaccattgcgcttctccggaaacattagc

SEQ ID NO: 426 - DNA, 102 bp, Artificial Sequence
  Synthetic Polynucleotide
acaaccgcgtgttacaaggccaggcatccgagaggtctgggaatgcatcccactgcgcctgatcctgaacataaaccattgcgcttctccggaaacattagc

SEQ ID NO: 427 - DNA, 102 bp, Artificial Sequence
  Synthetic Polynucleotide
acaaccgcgtgttacaaggccaggcatccgagaggtctgggaatgcccatgccgactcgcgccagatcataacgtacattgcgcttctccggaaacattagc

SEQ ID NO: 428 - DNA, 102 bp, Artificial Sequence
  Synthetic Polynucleotide
acaaccgcgtgttacaaggccaggcatccgagaggtctgggaatgcgtaccaacagagacacccggcgtgtagctacattgcgcttctccggaaacattagc

SEQ ID NO: 429 - DNA, 102 bp, Artificial Sequence
  Synthetic Polynucleotide
acaaccgcgtgttacaaggccaggcatccgagaggtctgggaatgccgcaaagccgcgaatgatcaggtggtcatacattgcgcttctccggaaacattagc

SEQ ID NO: 430 - DNA, 102 bp, Artificial Sequence
  Synthetic Polynucleotide
acaaccgcgtgttacaaggccaggcatccgagaggtctgggaatgctgaacttctttcagcggttcggtggtcggacattgcgcttctccggaaacattagc

SEQ ID NO: 431 - DNA, 102 bp, Artificial Sequence
  Synthetic Polynucleotide
acaaccgcgtgttacaaggccaggcatccgagaggtctgggaatgccgctaaccgctgtggctactacaactgcgacattgcgcttctccggaaacattagc

SEQ ID NO: 432 - DNA, 102 bp, Artificial Sequence
  Synthetic Polynucleotide
acaaccgcgtgttacaaggccaggcatccgagaggtctgggaatgccggttcaaccgctgcctgtgcataaacagacattgcgcttctccggaaacattagc

SEQ ID NO: 433 - DNA, 102 bp, Artificial Sequence
  Synthetic Polynucleotide
acaaccgcgtgttacaaggccaggcatccgagaggtctgggaatgcaccggtttccggctcgttctggaagtaagacattgcgcttctccggaaacattagc

SEQ ID NO: 434 - DNA, 102 bp, Artificial Sequence
  Synthetic Polynucleotide
acaaccgcgtgttacaaggccaggcatccgagaggtctgggaatgctcttctgaccctttctgctgggcattggcacattgcgcttctccggaaacattagc

SEQ ID NO: 435 - DNA, 102 bp, Artificial Sequence
  Synthetic Polynucleotide
acaaccgcgtgttacaaggccaggcatccgagaggtctgggaatgccagcaaagcgcaggttctgacgcacagtaacattgcgcttctccggaaacattagc

SEQ ID NO: 436 - DNA, 102 bp, Artificial Sequence
  Synthetic Polynucleotide
acaaccgcgtgttacaaggccaggcatccgagaggtctgggaatgcatctcgccaccttcaaccgagaagaaggaacattgcgcttctccggaaacattagc

SEQ ID NO: 437 - DNA, 102 bp, Artificial Sequence
  Synthetic Polynucleotide
acaaccgcgtgttacaaggccaggcatccgagaggtctgggaatgccagcgtcagacctgaaagcggaccgtcaaacattgcgcttctccggaaacattagc

SEQ ID NO: 438 - DNA, 102 bp, Artificial Sequence
  Synthetic Polynucleotide
acaaccgcgtgttacaaggccaggcatccgagaggtctgggaatgcgaggaagctgctgcggcaaataagccacttcattgcgcttctccggaaacattagc

SEQ ID NO: 439 - DNA, 102 bp, Artificial Sequence
  Synthetic Polynucleotide
acaaccgcgtgttacaaggccaggcatccgagaggtctgggaatgcgcgacagcacatcaacctggtgggcgatatcattgcgcttctccggaaacattagc

SEQ ID NO: 440 - DNA, 102 bp, Artificial Sequence
  Synthetic Polynucleotide
acaaccgcgtgttacaaggccaggcatccgagaggtctgggaatgcgagcagagtggatttaccagaaccgttgtgcattgcgcttctccggaaacattagc

SEQ ID NO: 441 - DNA, 102 bp, Artificial Sequence
  Synthetic Polynucleotide
acaaccgcgtgttacaaggccaggcatccgagaggtctgggaatgccccatcgggatgccataaatcatttcgaggcattgcgcttctccggaaacattagc

SEQ ID NO: 442 - DNA, 102 bp, Artificial Sequence
  Synthetic Polynucleotide
acaaccgcgtgttacaaggccaggcatccgagaggtctgggaatgccaaacgctttgctgctccagctttccagcgcattgcgcttctccggaaacattagc

SEQ ID NO: 443 - DNA, 102 bp, Artificial Sequence
  Synthetic Polynucleotide
acaaccgcgtgttacaaggccaggcatccgagaggtctgggaatgcccgcgcagggcgaccagataatcacagtagcattgcgcttctccggaaacattagc

SEQ ID NO: 444 - DNA, 102 bp, Artificial Sequence
  Synthetic Polynucleotide
acaaccgcgtgttacaaggccaggcatccgagaggtctgggaatgcccacgggtaacgaccaatcgccaccagttccattgcgcttctccggaaacattagc

SEQ ID NO: 445 - DNA, 102 bp, Artificial Sequence
  Synthetic Polynucleotide
acaaccgcgtgttacaaggccaggcatccgagaggtctgggaatgcccgaggtcggttcgtcgagcaacagacaaccattgcgcttctccggaaacattagc

SEQ ID NO: 446 - DNA, 102 bp, Artificial Sequence
  Synthetic Polynucleotide
acaaccgcgtgttacaaggccaggcatccgagaggtctgggaatgcgaccggtcactttcccggcaggaaaggttacattgcgcttctccggaaacattagc

SEQ ID NO: 447 - DNA, 102 bp, Artificial Sequence
  Synthetic Polynucleotide
acaaccgcgtgttacaaggccaggcatccgagaggtctgggaatgccaatgaccgtcaggccacgctcctgacttacattgcgcttctccggaaacattagc

SEQ ID NO: 448 - DNA, 102 bp, Artificial Sequence
  Synthetic Polynucleotide
acaaccgcgtgttacaaggccaggcatccgagaggtctgggaatgcgtgcgcccgggcacacgaaaggagatattacattgcgcttctccggaaacattagc

SEQ ID NO: 449 - DNA, 102 bp, Artificial Sequence
  Synthetic Polynucleotide
acaaccgcgtgttacaaggccaggcatccgagaggtctgggaatgcgacgttcgccgccagagagactatcgaccacattgcgcttctccggaaacattagc

SEQ ID NO: 450 - DNA, 102 bp, Artificial Sequence
  Synthetic Polynucleotide
acaaccgcgtgttacaaggccaggcatccgagaggtctgggaatgcgcataatttccgcaggcgttccctgagcaacattgcgcttctccggaaacattagc

SEQ ID NO: 451 - DNA, 102 bp, Artificial Sequence
  Synthetic Polynucleotide
acaaccgcgtgttacaaggccaggcatccgagaggtctgggaatgctagtgcggaacggtcaggcgttcagtatttcattgcgcttctccggaaacattagc

SEQ ID NO: 452 - DNA, 102 bp, Artificial Sequence
  Synthetic Polynucleotide
acaaccgcgtgttacaaggccaggcatccgagaggtctgggaatgccggagaggccagattgctgcctatggcaatcattgcgcttctccggaaacattagc

SEQ ID NO: 453 - DNA, 102 bp, Artificial Sequence
  Synthetic Polynucleotide
acaaccgcgtgttacaaggccaggcatccgagaggtctgggaatgctaccaaacagcatgatgtcgagatccagcgcattgcgcttctccggaaacattagc

SEQ ID NO: 454 - DNA, 102 bp, Artificial Sequence
  Synthetic Polynucleotide
acaaccgcgtgttacaaggccaggcatccgagaggtctgggaatgcatcaggaaacaccaactccggcgcgatttccattgcgcttctccggaaacattagc

SEQ ID NO: 455 - DNA, 102 bp, Artificial Sequence
  Synthetic Polynucleotide
acaaccgcgtgttacaaggccaggcatccgagaggtctgggaatgccacggctgcgtttaagtaatcgggttgatccattgcgcttctccggaaacattagc

SEQ ID NO: 456 - DNA, 102 bp, Artificial Sequence
  Synthetic Polynucleotide
acaaccgcgtgttacaaggccaggcatccgagaggtctgggaatgccggtaagaatgtggctttcagggatatcgccattgcgcttctccggaaacattagc

SEQ ID NO: 457 - DNA, 102 bp, Artificial Sequence
  Synthetic Polynucleotide
acaaccgcgtgttacaaggccaggcatccgagaggtctgggaatgcagtagctcttcaggtgcaagagaggtttcccattgcgcttctccggaaacattagc

SEQ ID NO: 458 - DNA, 102 bp, Artificial Sequence
  Synthetic Polynucleotide
acaaccgcgtgttacaaggccaggcatccgagaggtctgggaatgcgcggccacagcataaatccacgattcttcacattgcgcttctccggaaacattagc

SEQ ID NO: 459 - DNA, 102 bp, Artificial Sequence
  Synthetic Polynucleotide
acaaccgcgtgttacaaggccaggcatccgagaggtctgggaatgcctttgcggacgcgaccttgctgcaattcaacattgcgcttctccggaaacattagc

SEQ ID NO: 460 - DNA, 102 bp, Artificial Sequence
  Synthetic Polynucleotide
acaaccgcgtgttacaaggccaggcatccgagaggtctgggaatgcgctcgatcacctctgccagtgtctgacgttcattgcgcttctccggaaacattagc

SEQ ID NO: 461 - DNA, 102 bp, Artificial Sequence
  Synthetic Polynucleotide
acaaccgcgtgttacaaggccaggcatccgagaggtctgggaatgccaccgatatcgacgacgcagacacccagttcattgcgcttctccggaaacattagc

SEQ ID NO: 462 - DNA, 102 bp, Artificial Sequence
  Synthetic Polynucleotide
acaaccgcgtgttacaaggccaggcatccgagaggtctgggaatgccggcgtgccaaaggcgtaagcgatatcactcattgcgcttctccggaaacattagc

SEQ ID NO: 463 - DNA, 102 bp, Artificial Sequence
  Synthetic Polynucleotide
acaaccgcgtgttacaaggccaggcatccgagaggtctgggaatgctactaaagcggcaaccttcgcggtaccaatcattgcgcttctccggaaacattagc

SEQ ID NO: 464 - DNA, 102 bp, Artificial Sequence
  Synthetic Polynucleotide
acaaccgcgtgttacaaggccaggcatccgagaggtctgggaatgccgcacgcccgaaagtcctaccggattcttgcattgcgcttctccggaaacattagc

SEQ ID NO: 465 - DNA, 102 bp, Artificial Sequence
  Synthetic Polynucleotide
acaaccgcgtgttacaaggccaggcatccgagaggtctgggaatgccgccatatcgttgtgacatgtgatcaggtgcattgcgcttctccggaaacattagc

SEQ ID NO: 466 - DNA, 102 bp, Artificial Sequence
  Synthetic Polynucleotide
acaaccgcgtgttacaaggccaggcatccgagaggtctgggaatgcggcaccataccaatttcattctggcagctgcattgcgcttctccggaaacattagc

SEQ ID NO: 467 - DNA, 102 bp, Artificial Sequence
  Synthetic Polynucleotide
acaaccgcgtgttacaaggccaggcatccgagaggtctgggaatgccctttatccataccacgcgacgggcagctgcattgcgcttctccggaaacattagc

SEQ ID NO: 468 - DNA, 102 bp, Artificial Sequence
  Synthetic Polynucleotide
acaaccgcgtgttacaaggccaggcatccgagaggtctgggaatgctcctgatagtcaatcgcatactcttgcgggcattgcgcttctccggaaacattagc

SEQ ID NO: 469 - DNA, 102 bp, Artificial Sequence
  Synthetic Polynucleotide
acaaccgcgtgttacaaggccaggcatccgagaggtctgggaatgcgccagcataaggaattaccttagtgtggcgcattgcgcttctccggaaacattagc

SEQ ID NO: 470 - DNA, 102 bp, Artificial Sequence
  Synthetic Polynucleotide
acaaccgcgtgttacaaggccaggcatccgagaggtctgggaatgcactctttcccatagtgaagcaatcccaccgcattgcgcttctccggaaacattagc

SEQ ID NO: 471 - DNA, 102 bp, Artificial Sequence
  Synthetic Polynucleotide
acaaccgcgtgttacaaggccaggcatccgagaggtctgggaatgctacggctcctgagcataatccgttaaaccgcattgcgcttctccggaaacattagc

SEQ ID NO: 472 - DNA, 102 bp, Artificial Sequence
  Synthetic Polynucleotide
acaaccgcgtgttacaaggccaggcatccgagaggtctgggaatgcgccaatgatattgaccataccgtcgggcagcattgcgcttctccggaaacattagc

SEQ ID NO: 473 - DNA, 102 bp, Artificial Sequence
  Synthetic Polynucleotide
acaaccgcgtgttacaaggccaggcatccgagaggtctgggaatgccagttggtcaactttcagcccacaacgttccattgcgcttctccggaaacattagc

SEQ ID NO: 474 - DNA, 102 bp, Artificial Sequence
  Synthetic Polynucleotide
acaaccgcgtgttacaaggccaggcatccgagaggtctgggaatgcctgacaatctgccatcaattctgcctggtccattgcgcttctccggaaacattagc

SEQ ID NO: 475 - DNA, 102 bp, Artificial Sequence
  Synthetic Polynucleotide
acaaccgcgtgttacaaggccaggcatccgagaggtctgggaatgctatctcttcgttgaccaggttgagcagctccattgcgcttctccggaaacattagc

SEQ ID NO: 476 - DNA, 102 bp, Artificial Sequence
  Synthetic Polynucleotide
acaaccgcgtgttacaaggccaggcatccgagaggtctgggaatgccccagcgcacaaccgtggcgaactttaatccattgcgcttctccggaaacattagc

SEQ ID NO: 477 - DNA, 102 bp, Artificial Sequence
  Synthetic Polynucleotide
acaaccgcgtgttacaaggccaggcatccgagaggtctgggaatgccaataccgaataacttgatgccagtccggccattgcgcttctccggaaacattagc

SEQ ID NO: 478 - DNA, 102 bp, Artificial Sequence
  Synthetic Polynucleotide
acaaccgcgtgttacaaggccaggcatccgagaggtctgggaatgcgcacttgcgtatgaaacacgcgctgagcaccattgcgcttctccggaaacattagc

SEQ ID NO: 479 - DNA, 102 bp, Artificial Sequence
  Synthetic Polynucleotide
acaaccgcgtgttacaaggccaggcatccgagaggtctgggaatgccgcagccaactattgagtcgcttgatccaccattgcgcttctccggaaacattagc

SEQ ID NO: 480 - DNA, 102 bp, Artificial Sequence
  Synthetic Polynucleotide
acaaccgcgtgttacaaggccaggcatccgagaggtctgggaatgccttcgatctgcgctgcgccaccggttaatacattgcgcttctccggaaacattagc

SEQ ID NO: 481 - DNA, 102 bp, Artificial Sequence
  Synthetic Polynucleotide
acaaccgcgtgttacaaggccaggcatccgagaggtctgggaatgccgcgttgtacgcacttgaccacggattcgacattgcgcttctccggaaacattagc

SEQ ID NO: 482 - DNA, 102 bp, Artificial Sequence
  Synthetic Polynucleotide
acaaccgcgtgttacaaggccaggcatccgagaggtctgggaatgccgttctggcggcacgctgaaggtatttcctcattgcgcttctccggaaacattagc

SEQ ID NO: 483 - DNA, 102 bp, Artificial Sequence
  Synthetic Polynucleotide
acaaccgcgtgttacaaggccaggcatccgagaggtctgggaatgccttccgggccatacagcattggaagcacctcattgcgcttctccggaaacattagc

SEQ ID NO: 484 - DNA, 102 bp, Artificial Sequence
  Synthetic Polynucleotide
acaaccgcgtgttacaaggccaggcatccgagaggtctgggaatgctttcgcgatagccctgcaacacttcattggcattgcgcttctccggaaacattagc

SEQ ID NO: 485 - DNA, 102 bp, Artificial Sequence
  Synthetic Polynucleotide
acaaccgcgtgttacaaggccaggcatccgagaggtctgggaatgcgttgctgagtagattcctctggcggcaaggcattgcgcttctccggaaacattagc

SEQ ID NO: 486 - DNA, 102 bp, Artificial Sequence
  Synthetic Polynucleotide
acaaccgcgtgttacaaggccaggcatccgagaggtctgggaatgccccaatgccaggatcgactgccggatatcgcattgcgcttctccggaaacattagc

SEQ ID NO: 487 - DNA, 102 bp, Artificial Sequence
  Synthetic Polynucleotide
acaaccgcgtgttacaaggccaggcatccgagaggtctgggaatgctaatccacggcaggcgttgttctatttgcgcattgcgcttctccggaaacattagc

SEQ ID NO: 488 - DNA, 102 bp, Artificial Sequence
  Synthetic Polynucleotide
acaaccgcgtgttacaaggccaggcatccgagaggtctgggaatgctgttgacatcctgggtcataaaggtacccgcattgcgcttctccggaaacattagc

SEQ ID NO: 489 - DNA, 102 bp, Artificial Sequence
  Synthetic Polynucleotide
acaaccgcgtgttacaaggccaggcatccgagaggtctgggaatgcatcgttattcagcgtcaactgccaggaacgcattgcgcttctccggaaacattagc

SEQ ID NO: 490 - DNA, 102 bp, Artificial Sequence
  Synthetic Polynucleotide
acaaccgcgtgttacaaggccaggcatccgagaggtctgggaatgcccagacgcgttccattattgcggcgagaagcattgcgcttctccggaaacattagc

SEQ ID NO: 491 - DNA, 102 bp, Artificial Sequence
  Synthetic Polynucleotide
acaaccgcgtgttacaaggccaggcatccgagaggtctgggaatgccggtcatcgccgcttccttcagagtaaatccattgcgcttctccggaaacattagc

SEQ ID NO: 492 - DNA, 102 bp, Artificial Sequence
  Synthetic Polynucleotide
acaaccgcgtgttacaaggccaggcatccgagaggtctgggaatgcacgtagctaatccgtttgccatcggtttgccattgcgcttctccggaaacattagc

SEQ ID NO: 493 - DNA, 102 bp, Artificial Sequence
  Synthetic Polynucleotide
acaaccgcgtgttacaaggccaggcatccgagaggtctgggaatgcgtctaccatatgttgatcattccaccgcgccattgcgcttctccggaaacattagc

SEQ ID NO: 494 - DNA, 102 bp, Artificial Sequence
  Synthetic Polynucleotide
acaaccgcgtgttacaaggccaggcatccgagaggtctgggaatgctcaattcatcaggccactgctttctgacgccattgcgcttctccggaaacattagc

SEQ ID NO: 495 - DNA, 102 bp, Artificial Sequence
  Synthetic Polynucleotide
acaaccgcgtgttacaaggccaggcatccgagaggtctgggaatgccagcctactgccgctccagagtcataacgccattgcgcttctccggaaacattagc

SEQ ID NO: 496 - DNA, 102 bp, Artificial Sequence
  Synthetic Polynucleotide
acaaccgcgtgttacaaggccaggcatccgagaggtctgggaatgcacgtgtgtaatggcgttcaccggtcaacaccattgcgcttctccggaaacattagc

SEQ ID NO: 497 - DNA, 102 bp, Artificial Sequence
  Synthetic Polynucleotide
acaaccgcgtgttacaaggccaggcatccgagaggtctgggaatgctcttcttcgctgtttcgcgtgttcagagcacattgcgcttctccggaaacattagc

SEQ ID NO: 498 - DNA, 102 bp, Artificial Sequence
  Synthetic Polynucleotide
acaaccgcgtgttacaaggccaggcatccgagaggtctgggaatgcagcaaatgcacggatggtgttacctaccgtcattgcgcttctccggaaacattagc

SEQ ID NO: 499 - DNA, 102 bp, Artificial Sequence
  Synthetic Polynucleotide
acaaccgcgtgttacaaggccaggcatccgagaggtctgggaatgctgcacagcgcctttcagtacatcgttcgctcattgcgcttctccggaaacattagc

SEQ ID NO: 500 - DNA, 102 bp, Artificial Sequence
  Synthetic Polynucleotide
acaaccgcgtgttacaaggccaggcatccgagaggtctgggaatgcagagaagtaccgataaccacagtcgcgttgcattgcgcttctccggaaacattagc

SEQ ID NO: 501 - DNA, 102 bp, Artificial Sequence
  Synthetic Polynucleotide
acaaccgcgtgttacaaggccaggcatccgagaggtctgggaatgctgctgaacctgcttattggtcaccagagtgcattgcgcttctccggaaacattagc

SEQ ID NO: 502 - DNA, 102 bp, Artificial Sequence
  Synthetic Polynucleotide
acaaccgcgtgttacaaggccaggcatccgagaggtctgggaatgccggttacgcgcagctcgtcattcatatccgcattgcgcttctccggaaacattagc

SEQ ID NO: 503 - DNA, 102 bp, Artificial Sequence
  Synthetic Polynucleotide
acaaccgcgtgttacaaggccaggcatccgagaggtctgggaatgccagggagataccgcggcccagaactttcagcattgcgcttctccggaaacattagc

SEQ ID NO: 504 - DNA, 102 bp, Artificial Sequence
  Synthetic Polynucleotide
acaaccgcgtgttacaaggccaggcatccgagaggtctgggaatgccgcgccagacaggtcgatatcttccagcagcattgcgcttctccggaaacattagc

SEQ ID NO: 505 - DNA, 102 bp, Artificial Sequence
  Synthetic Polynucleotide
acaaccgcgtgttacaaggccaggcatccgagaggtctgggaatgccaggtcgaagcccgccgtgatgttaaccagcattgcgcttctccggaaacattagc

SEQ ID NO: 506 - DNA, 102 bp, Artificial Sequence
  Synthetic Polynucleotide
acaaccgcgtgttacaaggccaggcatccgagaggtctgggaatgcaggacgtttgtccatgccgatacctgtcgccattgcgcttctccggaaacattagc

SEQ ID NO: 507 - DNA, 102 bp, Artificial Sequence
  Synthetic Polynucleotide
acaaccgcgtgttacaaggccaggcatccgagaggtctgggaatgcagagatagccatttcagcagcttcttccgccattgcgcttctccggaaacattagc

SEQ ID NO: 508 - DNA, 102 bp, Artificial Sequence
  Synthetic Polynucleotide
acaaccgcgtgttacaaggccaggcatccgagaggtctgggaatgcccaccacccatacccgcagcaataaagacccattgcgcttctccggaaacattagc

SEQ ID NO: 509 - DNA, 102 bp, Artificial Sequence
  Synthetic Polynucleotide
acaaccgcgtgttacaaggccaggcatccgagaggtctgggaatgccttcagcgacgactggtgctgcacctgtaccattgcgcttctccggaaacattagc

SEQ ID NO: 510 - DNA, 102 bp, Artificial Sequence
  Synthetic Polynucleotide
acaaccgcgtgttacaaggccaggcatccgagaggtctgggaatgccagcgcccagtcctttggtgataccgctaccattgcgcttctccggaaacattagc

SEQ ID NO: 511 - DNA, 102 bp, Artificial Sequence
  Synthetic Polynucleotide
acaaccgcgtgttacaaggccaggcatccgagaggtctgggaatgccgcagtttgcggcgcattgtcattcacgaccattgcgcttctccggaaacattagc

SEQ ID NO: 512 - DNA, 102 bp, Artificial Sequence
  Synthetic Polynucleotide
acaaccgcgtgttacaaggccaggcatccgagaggtctgggaatgccattacggtgcgtacgtctgcaaagtccaccattgcgcttctccggaaacattagc

SEQ ID NO: 513 - DNA, 102 bp, Artificial Sequence
  Synthetic Polynucleotide
acaaccgcgtgttacaaggccaggcatccgagaggtctgggaatgctcaaacccggacgagtaatcagttcagcgacattgcgcttctccggaaacattagc

SEQ ID NO: 514 - DNA, 102 bp, Artificial Sequence
  Synthetic Polynucleotide
acaaccgcgtgttacaaggccaggcatccgagaggtctgggaatgctgaaaggcttagtgacgacagcaacggtcacattgcgcttctccggaaacattagc

SEQ ID NO: 515 - DNA, 102 bp, Artificial Sequence
  Synthetic Polynucleotide
acaaccgcgtgttacaaggccaggcatccgagaggtctgggaatgcccgacgccgatgactttaatcaccgcgtcacattgcgcttctccggaaacattagc

SEQ ID NO: 516 - DNA, 102 bp, Artificial Sequence
  Synthetic Polynucleotide
acaaccgcgtgttacaaggccaggcatccgagaggtctgggaatgcccatcccatgctgctggtagcgatccatcacattgcgcttctccggaaacattagc

SEQ ID NO: 517 - DNA, 102 bp, Artificial Sequence
  Synthetic Polynucleotide
acaaccgcgtgttacaaggccaggcatccgagaggtctgggaatgctgtcgttcgggatagtgatcagagagtccacattgcgcttctccggaaacattagc

SEQ ID NO: 518 - DNA, 102 bp, Artificial Sequence
  Synthetic Polynucleotide
acaaccgcgtgttacaaggccaggcatccgagaggtctgggaatgccagcgcttgtgcatcggtatttaccgcgaacattgcgcttctccggaaacattagc

SEQ ID NO: 519 - DNA, 102 bp, Artificial Sequence
  Synthetic Polynucleotide
acaaccgcgtgttacaaggccaggcatccgagaggtctgggaatgccttcaatgcgctcgcgcaccatgtgttcaacattgcgcttctccggaaacattagc

SEQ ID NO: 520 - DNA, 102 bp, Artificial Sequence
  Synthetic Polynucleotide
acaaccgcgtgttacaaggccaggcatccgagaggtctgggaatgcgacccggtttggtgtctggcatattgctttcattgcgcttctccggaaacattagc

SEQ ID NO: 521 - DNA, 102 bp, Artificial Sequence
  Synthetic Polynucleotide
acaaccgcgtgttacaaggccaggcatccgagaggtctgggaatgccatcacttccggcgaagcggtttctgctttcattgcgcttctccggaaacattagc

SEQ ID NO: 522 - DNA, 102 bp, Artificial Sequence
  Synthetic Polynucleotide
acaaccgcgtgttacaaggccaggcatccgagaggtctgggaatgctggtgcccaggagtttggcgagttaaaggtcattgcgcttctccggaaacattagc

SEQ ID NO: 523 - DNA, 102 bp, Artificial Sequence
  Synthetic Polynucleotide
acaaccgcgtgttacaaggccaggcatccgagaggtctgggaatgccatgataagagacaccacggcaggttacgtcattgcgcttctccggaaacattagc

SEQ ID NO: 524 - DNA, 102 bp, Artificial Sequence
  Synthetic Polynucleotide
acaaccgcgtgttacaaggccaggcatccgagaggtctgggaatgctgtgttcgtcagacgggattgcgttcggatcattgcgcttctccggaaacattagc

SEQ ID NO: 525 - DNA, 102 bp, Artificial Sequence
  Synthetic Polynucleotide
acaaccgcgtgttacaaggccaggcatccgagaggtctgggaatgcccggaaccaccagttcgccattacgacgatcattgcgcttctccggaaacattagc

SEQ ID NO: 526 - DNA, 102 bp, Artificial Sequence
  Synthetic Polynucleotide
acaaccgcgtgttacaaggccaggcatccgagaggtctgggaatgccaccgctaatcagcagtgcgaccaccagtgcattgcgcttctccggaaacattagc

SEQ ID NO: 527 - DNA, 102 bp, Artificial Sequence
  Synthetic Polynucleotide
acaaccgcgtgttacaaggccaggcatccgagaggtctgggaatgccgccggagcgtaaataactggcactttctgcattgcgcttctccggaaacattagc

SEQ ID NO: 528 - DNA, 102 bp, Artificial Sequence
  Synthetic Polynucleotide
acaaccgcgtgttacaaggccaggcatccgagaggtctgggaatgccgcccactttaatcggcgtcacttcattggcattgcgcttctccggaaacattagc

SEQ ID NO: 529 - DNA, 102 bp, Artificial Sequence
  Synthetic Polynucleotide
acaaccgcgtgttacaaggccaggcatccgagaggtctgggaatgctgctggctgtttacatggcagaccaaatggcattgcgcttctccggaaacattagc

SEQ ID NO: 530 - DNA, 102 bp, Artificial Sequence
  Synthetic Polynucleotide
acaaccgcgtgttacaaggccaggcatccgagaggtctgggaatgcaatcgcaatcagtcgaccatcattgaccggcattgcgcttctccggaaacattagc

SEQ ID NO: 531 - DNA, 102 bp, Artificial Sequence
  Synthetic Polynucleotide
acaaccgcgtgttacaaggccaggcatccgagaggtctgggaatgcttgagcacgcctttattggcgaaggtttcgcattgcgcttctccggaaacattagc

SEQ ID NO: 532 - DNA, 102 bp, Artificial Sequence
  Synthetic Polynucleotide
acaaccgcgtgttacaaggccaggcatccgagaggtctgggaatgcacatatccgcaccgctcaaatctttcgtcgcattgcgcttctccggaaacattagc

SEQ ID NO: 533 - DNA, 102 bp, Artificial Sequence
  Synthetic Polynucleotide
acaaccgcgtgttacaaggccaggcatccgagaggtctgggaatgccgttatcggcgttaatttgtttcagcggcgcattgcgcttctccggaaacattagc

SEQ ID NO: 534 - DNA, 102 bp, Artificial Sequence
  Synthetic Polynucleotide
acaaccgcgtgttacaaggccaggcatccgagaggtctgggaatgcgggctgttagcgtgacgagtaatcgtcgcgcattgcgcttctccggaaacattagc

SEQ ID NO: 535 - DNA, 102 bp, Artificial Sequence
  Synthetic Polynucleotide
acaaccgcgtgttacaaggccaggcatccgagaggtctgggaatgctagtcgcccatcttcgtaccaaatgaaccgcattgcgcttctccggaaacattagc

SEQ ID NO: 536 - DNA, 102 bp, Artificial Sequence
  Synthetic Polynucleotide
acaaccgcgtgttacaaggccaggcatccgagaggtctgggaatgcccgagcatcacaaggccagcgatagggtagcattgcgcttctccggaaacattagc

SEQ ID NO: 537 - DNA, 102 bp, Artificial Sequence
  Synthetic Polynucleotide
acaaccgcgtgttacaaggccaggcatccgagaggtctgggaatgcctgcggatcgttaaatccggcccaggtcagcattgcgcttctccggaaacattagc

SEQ ID NO: 538 - DNA, 102 bp, Artificial Sequence
  Synthetic Polynucleotide
acaaccgcgtgttacaaggccaggcatccgagaggtctgggaatgccaggcgctggtgagcggtacacaggtaaagcattgcgcttctccggaaacattagc

SEQ ID NO: 539 - DNA, 102 bp, Artificial Sequence
  Synthetic Polynucleotide
acaaccgcgtgttacaaggccaggcatccgagaggtctgggaatgcgttacccgggaagaccagcgtaccctgttccattgcgcttctccggaaacattagc

SEQ ID NO: 540 - DNA, 102 bp, Artificial Sequence
  Synthetic Polynucleotide
acaaccgcgtgttacaaggccaggcatccgagaggtctgggaatgcatcggtgataatcggtggcgaagtcggttccattgcgcttctccggaaacattagc

SEQ ID NO: 541 - DNA, 102 bp, Artificial Sequence
  Synthetic Polynucleotide
acaaccgcgtgttacaaggccaggcatccgagaggtctgggaatgcctgtgccggaagatccatgtcccacaggtccattgcgcttctccggaaacattagc

SEQ ID NO: 542 - DNA, 102 bp, Artificial Sequence
  Synthetic Polynucleotide
acaaccgcgtgttacaaggccaggcatccgagaggtctgggaatgcggtcacgcccatcggcagatagaccagatccattgcgcttctccggaaacattagc

SEQ ID NO: 543 - DNA, 102 bp, Artificial Sequence
  Synthetic Polynucleotide
acaaccgcgtgttacaaggccaggcatccgagaggtctgggaatgccaggatcgtaatgccatttctctttgccgccattgcgcttctccggaaacattagc

SEQ ID NO: 544 - DNA, 102 bp, Artificial Sequence
  Synthetic Polynucleotide
acaaccgcgtgttacaaggccaggcatccgagaggtctgggaatgcttacttcacatcatccggcagcgcataagccattgcgcttctccggaaacattagc

SEQ ID NO: 545 - DNA, 102 bp, Artificial Sequence
  Synthetic Polynucleotide
acaaccgcgtgttacaaggccaggcatccgagaggtctgggaatgcgaacggtctggtagctccacgccagtttcccattgcgcttctccggaaacattagc

SEQ ID NO: 546 - DNA, 102 bp, Artificial Sequence
  Synthetic Polynucleotide
acaaccgcgtgttacaaggccaggcatccgagaggtctgggaatgcgcctgcggagatcaccacatactgcttacccattgcgcttctccggaaacattagc

SEQ ID NO: 547 - DNA, 102 bp, Artificial Sequence
  Synthetic Polynucleotide
acaaccgcgtgttacaaggccaggcatccgagaggtctgggaatgcctgccgtagcggcgataaacagcacgttaccattgcgcttctccggaaacattagc

SEQ ID NO: 548 - DNA, 102 bp, Artificial Sequence
  Synthetic Polynucleotide
acaaccgcgtgttacaaggccaggcatccgagaggtctgggaatgccttcataggtcattggcgtagcctgaccaccattgcgcttctccggaaacattagc

SEQ ID NO: 549 - DNA, 102 bp, Artificial Sequence
  Synthetic Polynucleotide
acaaccgcgtgttacaaggccaggcatccgagaggtctgggaatgcggcaatcgccacttcacgatttggatcaaccattgcgcttctccggaaacattagc

SEQ ID NO: 550 - DNA, 102 bp, Artificial Sequence
  Synthetic Polynucleotide
acaaccgcgtgttacaaggccaggcatccgagaggtctgggaatgccggagtcagcgcccagaagtcgaaaccaaccattgcgcttctccggaaacattagc

SEQ ID NO: 551 - DNA, 102 bp, Artificial Sequence
  Synthetic Polynucleotide
acaaccgcgtgttacaaggccaggcatccgagaggtctgggaatgcggaacgggttgagcgtgacaccatacggtacattgcgcttctccggaaacattagc

SEQ ID NO: 552 - DNA, 102 bp, Artificial Sequence
  Synthetic Polynucleotide
acaaccgcgtgttacaaggccaggcatccgagaggtctgggaatgcaccgttgctcatgttgtaagcgcgcaggtacattgcgcttctccggaaacattagc

SEQ ID NO: 553 - DNA, 102 bp, Artificial Sequence
  Synthetic Polynucleotide
acaaccgcgtgttacaaggccaggcatccgagaggtctgggaatgcggatcgttcggctgcttcacatcgccagtacattgcgcttctccggaaacattagc

SEQ ID NO: 554 - DNA, 102 bp, Artificial Sequence
  Synthetic Polynucleotide
acaaccgcgtgttacaaggccaggcatccgagaggtctgggaatgcgaccagccagcctccgccaatgagtagatacattgcgcttctccggaaacattagc

SEQ ID NO: 555 - DNA, 102 bp, Artificial Sequence
  Synthetic Polynucleotide
acaaccgcgtgttacaaggccaggcatccgagaggtctgggaatgctgccttcatagcgcatctggtggaacatcacattgcgcttctccggaaacattagc

SEQ ID NO: 556 - DNA, 102 bp, Artificial Sequence
  Synthetic Polynucleotide
acaaccgcgtgttacaaggccaggcatccgagaggtctgggaatgccgttgaccttcctgattacgaccataggcacattgcgcttctccggaaacattagc

SEQ ID NO: 557 - DNA, 102 bp, Artificial Sequence
  Synthetic Polynucleotide
acaaccgcgtgttacaaggccaggcatccgagaggtctgggaatgccctgcggcgtaccaatacgtttcttccacacattgcgcttctccggaaacattagc

SEQ ID NO: 558 - DNA, 102 bp, Artificial Sequence
  Synthetic Polynucleotide
acaaccgcgtgttacaaggccaggcatccgagaggtctgggaatgcccaggaccacgcgggatcagtttcgaaacacattgcgcttctccggaaacattagc

SEQ ID NO: 559 - DNA, 102 bp, Artificial Sequence
  Synthetic Polynucleotide
acaaccgcgtgttacaaggccaggcatccgagaggtctgggaatgccccgcccagcatcggcatacccatattgaacattgcgcttctccggaaacattagc

SEQ ID NO: 560 - DNA, 102 bp, Artificial Sequence
  Synthetic Polynucleotide
acaaccgcgtgttacaaggccaggcatccgagaggtctgggaatgcgacaaacggcaggatcagccagatgccgaacattgcgcttctccggaaacattagc

SEQ ID NO: 561 - DNA, 102 bp, Artificial Sequence
  Synthetic Polynucleotide
acaaccgcgtgttacaaggccaggcatccgagaggtctgggaatgcgatcacgccagacgtttcgcgggttgagaacattgcgcttctccggaaacattagc

SEQ ID NO: 562 - DNA, 102 bp, Artificial Sequence
  Synthetic Polynucleotide
acaaccgcgtgttacaaggccaggcatccgagaggtctgggaatgccacgccggaccagctctgacctgaatgtttcattgcgcttctccggaaacattagc

SEQ ID NO: 563 - DNA, 102 bp, Artificial Sequence
  Synthetic Polynucleotide
acaaccgcgtgttacaaggccaggcatccgagaggtctgggaatgcgcgctttcgcaacgaactgcacgaagtgttcattgcgcttctccggaaacattagc

SEQ ID NO: 564 - DNA, 102 bp, Artificial Sequence
  Synthetic Polynucleotide
acaaccgcgtgttacaaggccaggcatccgagaggtctgggaatgctgtgcctacggtgtccatatttgcggcgatcattgcgcttctccggaaacattagc

SEQ ID NO: 565 - DNA, 102 bp, Artificial Sequence
  Synthetic Polynucleotide
acaaccgcgtgttacaaggccaggcatccgagaggtctgggaatgccaccagtcactacgttaccagcacaaatggcattgcgcttctccggaaacattagc

SEQ ID NO: 566 - DNA, 102 bp, Artificial Sequence
  Synthetic Polynucleotide
acaaccgcgtgttacaaggccaggcatccgagaggtctgggaatgccaaacgaagtttaatgccgggttcaggtcgcattgcgcttctccggaaacattagc

SEQ ID NO: 567 - DNA, 102 bp, Artificial Sequence
  Synthetic Polynucleotide
acaaccgcgtgttacaaggccaggcatccgagaggtctgggaatgcaaatttctcgccgttctcctcaacgatgcgcattgcgcttctccggaaacattagc

SEQ ID NO: 568 - DNA, 102 bp, Artificial Sequence
  Synthetic Polynucleotide
acaaccgcgtgttacaaggccaggcatccgagaggtctgggaatgcagagtggagcgtttagggcggatgagaacgcattgcgcttctccggaaacattagc

SEQ ID NO: 569 - DNA, 102 bp, Artificial Sequence
  Synthetic Polynucleotide
acaaccgcgtgttacaaggccaggcatccgagaggtctgggaatgctggtgcagccaccatcgctgacgatcattccattgcgcttctccggaaacattagc

SEQ ID NO: 570 - DNA, 102 bp, Artificial Sequence
  Synthetic Polynucleotide
acaaccgcgtgttacaaggccaggcatccgagaggtctgggaatgcaacgatatcggcacctgagaggataagctccattgcgcttctccggaaacattagc

SEQ ID NO: 571 - DNA, 102 bp, Artificial Sequence
  Synthetic Polynucleotide
acaaccgcgtgttacaaggccaggcatccgagaggtctgggaatgccttgttcctgcacacgaataaacgtggtgccattgcgcttctccggaaacattagc

SEQ ID NO: 572 - DNA, 102 bp, Artificial Sequence
  Synthetic Polynucleotide
acaaccgcgtgttacaaggccaggcatccgagaggtctgggaatgcattgacgttccagttcaacatcggaacggccattgcgcttctccggaaacattagc

SEQ ID NO: 573 - DNA, 102 bp, Artificial Sequence
  Synthetic Polynucleotide
acaaccgcgtgttacaaggccaggcatccgagaggtctgggaatgcgacgcgagttgtacaaacagaacctgggcccattgcgcttctccggaaacattagc

SEQ ID NO: 574 - DNA, 102 bp, Artificial Sequence
  Synthetic Polynucleotide
acaaccgcgtgttacaaggccaggcatccgagaggtctgggaatgcgccaacgtgacgtttcatcgcagactcggacattgcgcttctccggaaacattagc

SEQ ID NO: 575 - DNA, 102 bp, Artificial Sequence
  Synthetic Polynucleotide
acaaccgcgtgttacaaggccaggcatccgagaggtctgggaatgccgcagcatcggcacattcgattaccgcagacattgcgcttctccggaaacattagc

SEQ ID NO: 576 - DNA, 102 bp, Artificial Sequence
  Synthetic Polynucleotide
acaaccgcgtgttacaaggccaggcatccgagaggtctgggaatgccgaaatccgcatcagacgtaccggtagaaacattgcgcttctccggaaacattagc

SEQ ID NO: 577 - DNA, 102 bp, Artificial Sequence
  Synthetic Polynucleotide
acaaccgcgtgttacaaggccaggcatccgagaggtctgggaatgcggcagtcagcgtgaccatggtaacacccttcattgcgcttctccggaaacattagc

SEQ ID NO: 578 - DNA, 102 bp, Artificial Sequence
  Synthetic Polynucleotide
acaaccgcgtgttacaaggccaggcatccgagaggtctgggaatgccaccatatccatggtcgggaccagttcggtcattgcgcttctccggaaacattagc

SEQ ID NO: 579 - DNA, 102 bp, Artificial Sequence
  Synthetic Polynucleotide
acaaccgcgtgttacaaggccaggcatccgagaggtctgggaatgcgcttcttctgccgcttccagcagaccttctcattgcgcttctccggaaacattagc

SEQ ID NO: 580 - DNA, 102 bp, Artificial Sequence
  Synthetic Polynucleotide
acaaccgcgtgttacaaggccaggcatccgagaggtctgggaatgccacttccatttcggttggtgcaccaaagctcattgcgcttctccggaaacattagc

SEQ ID NO: 581 - DNA, 102 bp, Artificial Sequence
  Synthetic Polynucleotide
acaaccgcgtgttacaaggccaggcatccgagaggtctgggaatgcgaactctggcagcggcggaacacagttcatcattgcgcttctccggaaacattagc

SEQ ID NO: 582 - DNA, 102 bp, Artificial Sequence
  Synthetic Polynucleotide
acaaccgcgtgttacaaggccaggcatccgagaggtctgggaatgcacgtgttgtcagctcatccagcgtttcgtgcattgcgcttctccggaaacattagc

SEQ ID NO: 583 - DNA, 102 bp, Artificial Sequence
  Synthetic Polynucleotide
acaaccgcgtgttacaaggccaggcatccgagaggtctgggaatgctattgatatcttccatgctgtgcgccacggcattgcgcttctccggaaacattagc

SEQ ID NO: 584 - DNA, 102 bp, Artificial Sequence
  Synthetic Polynucleotide
acaaccgcgtgttacaaggccaggcatccgagaggtctgggaatgcgctacgcggaaaccggtcatcacttcatcgcattgcgcttctccggaaacattagc

SEQ ID NO: 585 - DNA, 102 bp, Artificial Sequence
  Synthetic Polynucleotide
acaaccgcgtgttacaaggccaggcatccgagaggtctgggaatgcttgccatcaacatcgtacagataagcgccgcattgcgcttctccggaaacattagc

SEQ ID NO: 586 - DNA, 102 bp, Artificial Sequence
  Synthetic Polynucleotide
acaaccgcgtgttacaaggccaggcatccgagaggtctgggaatgcccgaggcaggttaaatctggcactacgccgcattgcgcttctccggaaacattagc

SEQ ID NO: 587 - DNA, 102 bp, Artificial Sequence
  Synthetic Polynucleotide
acaaccgcgtgttacaaggccaggcatccgagaggtctgggaatgcctcaaatgcggcgcgtacagaagccagatccattgcgcttctccggaaacattagc

SEQ ID NO: 588 - DNA, 102 bp, Artificial Sequence
  Synthetic Polynucleotide
acaaccgcgtgttacaaggccaggcatccgagaggtctgggaatgccaacttcgcaaacacccgacgtgcagcatccattgcgcttctccggaaacattagc

SEQ ID NO: 589 - DNA, 102 bp, Artificial Sequence
  Synthetic Polynucleotide
acaaccgcgtgttacaaggccaggcatccgagaggtctgggaatgccgcttaaagcgttccacgtcacaggccatccattgcgcttctccggaaacattagc

SEQ ID NO: 590 - DNA, 102 bp, Artificial Sequence
  Synthetic Polynucleotide
acaaccgcgtgttacaaggccaggcatccgagaggtctgggaatgcaggtatatttggcgaaatctgccggaacgccattgcgcttctccggaaacattagc

SEQ ID NO: 591 - DNA, 102 bp, Artificial Sequence
  Synthetic Polynucleotide
acaaccgcgtgttacaaggccaggcatccgagaggtctgggaatgcctcatggtcgcttcagtgccggagttcacccattgcgcttctccggaaacattagc

SEQ ID NO: 592 - DNA, 102 bp, Artificial Sequence
  Synthetic Polynucleotide
acaaccgcgtgttacaaggccaggcatccgagaggtctgggaatgcccagcgcatccattacatcacgacgaccaccattgcgcttctccggaaacattagc

SEQ ID NO: 593 - DNA, 102 bp, Artificial Sequence
  Synthetic Polynucleotide
acaaccgcgtgttacaaggccaggcatccgagaggtctgggaatgccgcttcaaacgctgacggtgccaggtaaaccattgcgcttctccggaaacattagc

SEQ ID NO: 594 - DNA, 102 bp, Artificial Sequence
  Synthetic Polynucleotide
acaaccgcgtgttacaaggccaggcatccgagaggtctgggaatgcgctgcgcgacttcattcagacaggcgaaaccattgcgcttctccggaaacattagc

SEQ ID NO: 595 - DNA, 102 bp, Artificial Sequence
  Synthetic Polynucleotide
acaaccgcgtgttacaaggccaggcatccgagaggtctgggaatgcgccatcgcaatcgggttaccggaaagcgtacattgcgcttctccggaaacattagc

SEQ ID NO: 596 - DNA, 102 bp, Artificial Sequence
  Synthetic Polynucleotide
acaaccgcgtgttacaaggccaggcatccgagaggtctgggaatgctaccgaacatgccgccaacgtggttaacgacattgcgcttctccggaaacattagc

SEQ ID NO: 597 - DNA, 102 bp, Artificial Sequence
  Synthetic Polynucleotide
acaaccgcgtgttacaaggccaggcatccgagaggtctgggaatgcctaacgtgagtgcgccagaaccggctttcacattgcgcttctccggaaacattagc

SEQ ID NO: 598 - DNA, 102 bp, Artificial Sequence
  Synthetic Polynucleotide
acaaccgcgtgttacaaggccaggcatccgagaggtctgggaatgcctgccaccggctcgacgataatacaggcaacattgcgcttctccggaaacattagc

SEQ ID NO: 599 - DNA, 102 bp, Artificial Sequence
  Synthetic Polynucleotide
acaaccgcgtgttacaaggccaggcatccgagaggtctgggaatgcccgatatacggcagatgacggtaacgctgtcattgcgcttctccggaaacattagc

SEQ ID NO: 600 - DNA, 102 bp, Artificial Sequence
  Synthetic Polynucleotide
acaaccgcgtgttacaaggccaggcatccgagaggtctgggaatgcccatatcgctgccgctgtctttgtaacgctcattgcgcttctccggaaacattagc

SEQ ID NO: 601 - DNA, 102 bp, Artificial Sequence
  Synthetic Polynucleotide
acaaccgcgtgttacaaggccaggcatccgagaggtctgggaatgcggttcgcgcaggcttaagatctcacgcactcattgcgcttctccggaaacattagc

SEQ ID NO: 602 - DNA, 102 bp, Artificial Sequence
  Synthetic Polynucleotide
acaaccgcgtgttacaaggccaggcatccgagaggtctgggaatgctcatgagatacctgaacttcacggcacaggcattgcgcttctccggaaacattagc

SEQ ID NO: 603 - DNA, 102 bp, Artificial Sequence
  Synthetic Polynucleotide
acaaccgcgtgttacaaggccaggcatccgagaggtctgggaatgcgtttatccagcagcgtacaaatcgccagcgcattgcgcttctccggaaacattagc

SEQ ID NO: 604 - DNA, 102 bp, Artificial Sequence
  Synthetic Polynucleotide
acaaccgcgtgttacaaggccaggcatccgagaggtctgggaatgcaaattctaccgggacgttcacttcacgacgcattgcgcttctccggaaacattagc

SEQ ID NO: 605 - DNA, 102 bp, Artificial Sequence
  Synthetic Polynucleotide
acaaccgcgtgttacaaggccaggcatccgagaggtctgggaatgcatcttcaacaatcagcacgtccttgccacgcattgcgcttctccggaaacattagc

SEQ ID NO: 606 - DNA, 102 bp, Artificial Sequence
  Synthetic Polynucleotide
acaaccgcgtgttacaaggccaggcatccgagaggtctgggaatgcccgctaccgtagctggaggcggtcataaagcattgcgcttctccggaaacattagc

SEQ ID NO: 607 - DNA, 102 bp, Artificial Sequence
  Synthetic Polynucleotide
acaaccgcgtgttacaaggccaggcatccgagaggtctgggaatgctcaatgccgtaacccaccacaaactcatcccattgcgcttctccggaaacattagc

SEQ ID NO: 608 - DNA, 102 bp, Artificial Sequence
  Synthetic Polynucleotide
acaaccgcgtgttacaaggccaggcatccgagaggtctgggaatgcaaacataaatgagccacgcagcagacccaccattgcgcttctccggaaacattagc

SEQ ID NO: 609 - DNA, 102 bp, Artificial Sequence
  Synthetic Polynucleotide
acaaccgcgtgttacaaggccaggcatccgagaggtctgggaatgcgacgacccagttcggcgatacgcgctttaacattgcgcttctccggaaacattagc

SEQ ID NO: 610 - DNA, 102 bp, Artificial Sequence
  Synthetic Polynucleotide
acaaccgcgtgttacaaggccaggcatccgagaggtctgggaatgcggtattcccggctgttagcgcttcagatttcattgcgcttctccggaaacattagc

SEQ ID NO: 611 - DNA, 102 bp, Artificial Sequence
  Synthetic Polynucleotide
acaaccgcgtgttacaaggccaggcatccgagaggtctgggaatgccgttcttgcaaacgcgagttaaagcgactgcattgcgcttctccggaaacattagc

SEQ ID NO: 612 - DNA, 102 bp, Artificial Sequence
  Synthetic Polynucleotide
acaaccgcgtgttacaaggccaggcatccgagaggtctgggaatgcgccaataatacgcagacgcacgttatgtcgcattgcgcttctccggaaacattagc

SEQ ID NO: 613 - DNA, 102 bp, Artificial Sequence
  Synthetic Polynucleotide
acaaccgcgtgttacaaggccaggcatccgagaggtctgggaatgcaaggcatacagcgttaacgcctcaataccgcattgcgcttctccggaaacattagc

SEQ ID NO: 614 - DNA, 102 bp, Artificial Sequence
  Synthetic Polynucleotide
acaaccgcgtgttacaaggccaggcatccgagaggtctgggaatgcccaccgtagttcgccgcaatattcagcgtccattgcgcttctccggaaacattagc

SEQ ID NO: 615 - DNA, 102 bp, Artificial Sequence
  Synthetic Polynucleotide
acaaccgcgtgttacaaggccaggcatccgagaggtctgggaatgcatctgatctggttgcaggtttccttgctgccattgcgcttctccggaaacattagc

SEQ ID NO: 616 - DNA, 102 bp, Artificial Sequence
  Synthetic Polynucleotide
acaaccgcgtgttacaaggccaggcatccgagaggtctgggaatgcggctttatgcccaaaggcacgaatcttccccattgcgcttctccggaaacattagc

SEQ ID NO: 617 - DNA, 102 bp, Artificial Sequence
  Synthetic Polynucleotide
acaaccgcgtgttacaaggccaggcatccgagaggtctgggaatgcccagttgcctgactccctggactatatccccattgcgcttctccggaaacattagc

SEQ ID NO: 618 - DNA, 102 bp, Artificial Sequence
  Synthetic Polynucleotide
acaaccgcgtgttacaaggccaggcatccgagaggtctgggaatgcgtcttgttcatcgaaatcgggccagagaaccattgcgcttctccggaaacattagc

SEQ ID NO: 619 - DNA, 102 bp, Artificial Sequence
  Synthetic Polynucleotide
acaaccgcgtgttacaaggccaggcatccgagaggtctgggaatgccgctatcgagcgcccacacaaacagttccacattgcgcttctccggaaacattagc

SEQ ID NO: 620 - DNA, 102 bp, Artificial Sequence
  Synthetic Polynucleotide
acaaccgcgtgttacaaggccaggcatccgagaggtctgggaatgcgccgccgaaacgacgctctcgattagcaaacattgcgcttctccggaaacattagc

SEQ ID NO: 621 - DNA, 102 bp, Artificial Sequence
  Synthetic Polynucleotide
acaaccgcgtgttacaaggccaggcatccgagaggtctgggaatgcccatgcgtagcgccaggtacaggctttcttcattgcgcttctccggaaacattagc

SEQ ID NO: 622 - DNA, 102 bp, Artificial Sequence
  Synthetic Polynucleotide
acaaccgcgtgttacaaggccaggcatccgagaggtctgggaatgcgaggcaggcagaaaccgcgtgttgttcattcattgcgcttctccggaaacattagc

SEQ ID NO: 623 - DNA, 102 bp, Artificial Sequence
  Synthetic Polynucleotide
acaaccgcgtgttacaaggccaggcatccgagaggtctgggaatgccgaggtatcgccgtggaaaccatctttgatcattgcgcttctccggaaacattagc

SEQ ID NO: 624 - DNA, 102 bp, Artificial Sequence
  Synthetic Polynucleotide
acaaccgcgtgttacaaggccaggcatccgagaggtctgggaatgcttattcgtcgtgcgagattatcgccgggatcattgcgcttctccggaaacattagc

SEQ ID NO: 625 - DNA, 102 bp, Artificial Sequence
  Synthetic Polynucleotide
acaaccgcgtgttacaaggccaggcatccgagaggtctgggaatgcgacgcccggtttaacatacggttcgatcatcattgcgcttctccggaaacattagc

SEQ ID NO: 626 - DNA, 102 bp, Artificial Sequence
  Synthetic Polynucleotide
acaaccgcgtgttacaaggccaggcatccgagaggtctgggaatgcagagatgcaaacggatttcggatagccgtgcattgcgcttctccggaaacattagc

SEQ ID NO: 627 - DNA, 102 bp, Artificial Sequence
  Synthetic Polynucleotide
acaaccgcgtgttacaaggccaggcatccgagaggtctgggaatgctaatcattacagatgcgatccagctcgccgcattgcgcttctccggaaacattagc

SEQ ID NO: 628 - DNA, 102 bp, Artificial Sequence
  Synthetic Polynucleotide
acaaccgcgtgttacaaggccaggcatccgagaggtctgggaatgcatcgccatctttcagcagcttagcatcgtccattgcgcttctccggaaacattagc

SEQ ID NO: 629 - DNA, 102 bp, Artificial Sequence
  Synthetic Polynucleotide
acaaccgcgtgttacaaggccaggcatccgagaggtctgggaatgcgcgttgaccattggctcgatggtgaacgtccattgcgcttctccggaaacattagc

SEQ ID NO: 630 - DNA, 102 bp, Artificial Sequence
  Synthetic Polynucleotide
acaaccgcgtgttacaaggccaggcatccgagaggtctgggaatgcaccgtccagccatctttcatggtgcggatccattgcgcttctccggaaacattagc

SEQ ID NO: 631 - DNA, 102 bp, Artificial Sequence
  Synthetic Polynucleotide
acaaccgcgtgttacaaggccaggcatccgagaggtctgggaatgccatccttgcgtagcgtcagaatttcgcagccattgcgcttctccggaaacattagc

SEQ ID NO: 632 - DNA, 102 bp, Artificial Sequence
  Synthetic Polynucleotide
acaaccgcgtgttacaaggccaggcatccgagaggtctgggaatgctccgcaatattcacgaacgacggagaagcccattgcgcttctccggaaacattagc

SEQ ID NO: 633 - DNA, 102 bp, Artificial Sequence
  Synthetic Polynucleotide
acaaccgcgtgttacaaggccaggcatccgagaggtctgggaatgctgcggttcttcatggaagccgcgaccaatacattgcgcttctccggaaacattagc

SEQ ID NO: 634 - DNA, 102 bp, Artificial Sequence
  Synthetic Polynucleotide
acaaccgcgtgttacaaggccaggcatccgagaggtctgggaatgcaggtttcagtacgacgttggtttcacgggacattgcgcttctccggaaacattagc

SEQ ID NO: 635 - DNA, 102 bp, Artificial Sequence
  Synthetic Polynucleotide
acaaccgcgtgttacaaggccaggcatccgagaggtctgggaatgccttcgacaaatttctgaatcgccgcaccgacattgcgcttctccggaaacattagc

SEQ ID NO: 636 - DNA, 102 bp, Artificial Sequence
  Synthetic Polynucleotide
acaaccgcgtgttacaaggccaggcatccgagaggtctgggaatgccgcccatgatggtcggcttaccgacgataacattgcgcttctccggaaacattagc

SEQ ID NO: 637 - DNA, 102 bp, Artificial Sequence
  Synthetic Polynucleotide
acaaccgcgtgttacaaggccaggcatccgagaggtctgggaatgccgcctgcgggaagctctgatacagcactttcattgcgcttctccggaaacattagc

SEQ ID NO: 638 - DNA, 102 bp, Artificial Sequence
  Synthetic Polynucleotide
acaaccgcgtgttacaaggccaggcatccgagaggtctgggaatgcgcttacgccctttgcctttgcccttaccttcattgcgcttctccggaaacattagc

SEQ ID NO: 639 - DNA, 102 bp, Artificial Sequence
  Synthetic Polynucleotide
acaaccgcgtgttacaaggccaggcatccgagaggtctgggaatgccgcaattggcgcatccgcaatccacgtattcattgcgcttctccggaaacattagc

SEQ ID NO: 640 - DNA, 102 bp, Artificial Sequence
  Synthetic Polynucleotide
acaaccgcgtgttacaaggccaggcatccgagaggtctgggaatgcagcggacgggcactcaacatgtcatagagtcattgcgcttctccggaaacattagc

SEQ ID NO: 641 - DNA, 102 bp, Artificial Sequence
  Synthetic Polynucleotide
acaaccgcgtgttacaaggccaggcatccgagaggtctgggaatgcggcttagctcttctaccgggcgaccaaagtcattgcgcttctccggaaacattagc

SEQ ID NO: 642 - DNA, 102 bp, Artificial Sequence
  Synthetic Polynucleotide
acaaccgcgtgttacaaggccaggcatccgagaggtctgggaatgcatgatcagcgccatgtaagcttcgttcgctcattgcgcttctccggaaacattagc

SEQ ID NO: 643 - DNA, 102 bp, Artificial Sequence
  Synthetic Polynucleotide
acaaccgcgtgttacaaggccaggcatccgagaggtctgggaatgcccaccagcatcactctgccgctttcgctatcattgcgcttctccggaaacattagc

SEQ ID NO: 644 - DNA, 102 bp, Artificial Sequence
  Synthetic Polynucleotide
acaaccgcgtgttacaaggccaggcatccgagaggtctgggaatgcggatttcgttgtcgccgctctgaccgagatcattgcgcttctccggaaacattagc

SEQ ID NO: 645 - DNA, 102 bp, Artificial Sequence
  Synthetic Polynucleotide
acaaccgcgtgttacaaggccaggcatccgagaggtctgggaatgcctggcaccatacagtttggtcggctggttgcattgcgcttctccggaaacattagc

SEQ ID NO: 646 - DNA, 102 bp, Artificial Sequence
  Synthetic Polynucleotide
acaaccgcgtgttacaaggccaggcatccgagaggtctgggaatgctttcaccataccgactaacagcgcctgctgcattgcgcttctccggaaacattagc

SEQ ID NO: 647 - DNA, 102 bp, Artificial Sequence
  Synthetic Polynucleotide
acaaccgcgtgttacaaggccaggcatccgagaggtctgggaatgcacggacggcgaatcatctcaatgctgttggcattgcgcttctccggaaacattagc

SEQ ID NO: 648 - DNA, 102 bp, Artificial Sequence
  Synthetic Polynucleotide
acaaccgcgtgttacaaggccaggcatccgagaggtctgggaatgccggtcatcattctgcggtgaccagacctggcattgcgcttctccggaaacattagc

SEQ ID NO: 649 - DNA, 102 bp, Artificial Sequence
  Synthetic Polynucleotide
acaaccgcgtgttacaaggccaggcatccgagaggtctgggaatgcagatttaccgtcggcacgttcatcgaacggcattgcgcttctccggaaacattagc

SEQ ID NO: 650 - DNA, 102 bp, Artificial Sequence
  Synthetic Polynucleotide
acaaccgcgtgttacaaggccaggcatccgagaggtctgggaatgcggtcatgtctggctcaagattgaccattcgcattgcgcttctccggaaacattagc

SEQ ID NO: 651 - DNA, 102 bp, Artificial Sequence
  Synthetic Polynucleotide
acaaccgcgtgttacaaggccaggcatccgagaggtctgggaatgccaaactgcggctcagaacctccgaccatcgcattgcgcttctccggaaacattagc

SEQ ID NO: 652 - DNA, 102 bp, Artificial Sequence
  Synthetic Polynucleotide
acaaccgcgtgttacaaggccaggcatccgagaggtctgggaatgcgctcaagaatacggtctttgctgtaacgcgcattgcgcttctccggaaacattagc

SEQ ID NO: 653 - DNA, 102 bp, Artificial Sequence
  Synthetic Polynucleotide
acaaccgcgtgttacaaggccaggcatccgagaggtctgggaatgcaacatatccttgatccaaccggctacaccgcattgcgcttctccggaaacattagc

SEQ ID NO: 654 - DNA, 102 bp, Artificial Sequence
  Synthetic Polynucleotide
acaaccgcgtgttacaaggccaggcatccgagaggtctgggaatgcccagtaagaacgctcgctggagaggaacagcattgcgcttctccggaaacattagc

SEQ ID NO: 655 - DNA, 102 bp, Artificial Sequence
  Synthetic Polynucleotide
acaaccgcgtgttacaaggccaggcatccgagaggtctgggaatgcatggtgatcagacgcggatcaagacggaagcattgcgcttctccggaaacattagc

SEQ ID NO: 656 - DNA, 102 bp, Artificial Sequence
  Synthetic Polynucleotide
acaaccgcgtgttacaaggccaggcatccgagaggtctgggaatgccaaacagacgctgctcaccgtttggcgaagcattgcgcttctccggaaacattagc

SEQ ID NO: 657 - DNA, 102 bp, Artificial Sequence
  Synthetic Polynucleotide
acaaccgcgtgttacaaggccaggcatccgagaggtctgggaatgcgtcgcctccagcagcttcaccatctcgttccattgcgcttctccggaaacattagc

SEQ ID NO: 658 - DNA, 102 bp, Artificial Sequence
  Synthetic Polynucleotide
acaaccgcgtgttacaaggccaggcatccgagaggtctgggaatgccgtcggtttccctttgcgtccaattggctccattgcgcttctccggaaacattagc

SEQ ID NO: 659 - DNA, 102 bp, Artificial Sequence
  Synthetic Polynucleotide
acaaccgcgtgttacaaggccaggcatccgagaggtctgggaatgccggctgttgctgcggctgagaagactgatccattgcgcttctccggaaacattagc

SEQ ID NO: 660 - DNA, 102 bp, Artificial Sequence
  Synthetic Polynucleotide
acaaccgcgtgttacaaggccaggcatccgagaggtctgggaatgcacggttgttctccatattgacgatcgtcgccattgcgcttctccggaaacattagc

SEQ ID NO: 661 - DNA, 102 bp, Artificial Sequence
  Synthetic Polynucleotide
acaaccgcgtgttacaaggccaggcatccgagaggtctgggaatgccggctggcttaaggccgtcagataagtcgccattgcgcttctccggaaacattagc

SEQ ID NO: 662 - DNA, 102 bp, Artificial Sequence
  Synthetic Polynucleotide
acaaccgcgtgttacaaggccaggcatccgagaggtctgggaatgctcgagataaacgccgtaaatggcgatcagccattgcgcttctccggaaacattagc

SEQ ID NO: 663 - DNA, 102 bp, Artificial Sequence
  Synthetic Polynucleotide
acaaccgcgtgttacaaggccaggcatccgagaggtctgggaatgcataatctgttgctgttgcagcagacgcagccattgcgcttctccggaaacattagc

SEQ ID NO: 664 - DNA, 102 bp, Artificial Sequence
  Synthetic Polynucleotide
acaaccgcgtgttacaaggccaggcatccgagaggtctgggaatgctgacggtcttctgtcgccagcaaagtatcccattgcgcttctccggaaacattagc

SEQ ID NO: 665 - DNA, 102 bp, Artificial Sequence
  Synthetic Polynucleotide
acaaccgcgtgttacaaggccaggcatccgagaggtctgggaatgctcgctcaacttacgctgtttcttcagtgcccattgcgcttctccggaaacattagc

SEQ ID NO: 666 - DNA, 102 bp, Artificial Sequence
  Synthetic Polynucleotide
acaaccgcgtgttacaaggccaggcatccgagaggtctgggaatgcctgttgcgtcagcgtactcgcaccctgtaccattgcgcttctccggaaacattagc

SEQ ID NO: 667 - DNA, 102 bp, Artificial Sequence
  Synthetic Polynucleotide
acaaccgcgtgttacaaggccaggcatccgagaggtctgggaatgcacaagattcagcggcgttggcgtctggttacattgcgcttctccggaaacattagc

SEQ ID NO: 668 - DNA, 102 bp, Artificial Sequence
  Synthetic Polynucleotide
acaaccgcgtgttacaaggccaggcatccgagaggtctgggaatgcgtttgccagcaccgcacgtccgattgagtacattgcgcttctccggaaacattagc

SEQ ID NO: 669 - DNA, 102 bp, Artificial Sequence
  Synthetic Polynucleotide
acaaccgcgtgttacaaggccaggcatccgagaggtctgggaatgctgccgtcaatgcccgcaaaccaggtatctacattgcgcttctccggaaacattagc

SEQ ID NO: 670 - DNA, 102 bp, Artificial Sequence
  Synthetic Polynucleotide
acaaccgcgtgttacaaggccaggcatccgagaggtctgggaatgccgcgttgtaccacctgctgcatggtccatacattgcgcttctccggaaacattagc

SEQ ID NO: 671 - DNA, 102 bp, Artificial Sequence
  Synthetic Polynucleotide
acaaccgcgtgttacaaggccaggcatccgagaggtctgggaatgcgcaggcagttgccagaccttgccatcaatacattgcgcttctccggaaacattagc

SEQ ID NO: 672 - DNA, 102 bp, Artificial Sequence
  Synthetic Polynucleotide
acaaccgcgtgttacaaggccaggcatccgagaggtctgggaatgcccgtcgtagtccacgcccatatctgcaatacattgcgcttctccggaaacattagc

SEQ ID NO: 673 - DNA, 102 bp, Artificial Sequence
  Synthetic Polynucleotide
acaaccgcgtgttacaaggccaggcatccgagaggtctgggaatgcacttcaccactaaagcggtcgacgaccacacattgcgcttctccggaaacattagc

SEQ ID NO: 674 - DNA, 102 bp, Artificial Sequence
  Synthetic Polynucleotide
acaaccgcgtgttacaaggccaggcatccgagaggtctgggaatgcgtacgcccagtttaatccaggtctccgtaacattgcgcttctccggaaacattagc

SEQ ID NO: 675 - DNA, 102 bp, Artificial Sequence
  Synthetic Polynucleotide
acaaccgcgtgttacaaggccaggcatccgagaggtctgggaatgccctgcagctcctgacgcaccagttgcataacattgcgcttctccggaaacattagc

SEQ ID NO: 676 - DNA, 102 bp, Artificial Sequence
  Synthetic Polynucleotide
acaaccgcgtgttacaaggccaggcatccgagaggtctgggaatgcgtcctgggccaccgagtcaaaggtagtgaacattgcgcttctccggaaacattagc

SEQ ID NO: 677 - DNA, 102 bp, Artificial Sequence
  Synthetic Polynucleotide
acaaccgcgtgttacaaggccaggcatccgagaggtctgggaatgcgcgcacctgtccttctttactgtccgggaacattgcgcttctccggaaacattagc

SEQ ID NO: 678 - DNA, 102 bp, Artificial Sequence
  Synthetic Polynucleotide
acaaccgcgtgttacaaggccaggcatccgagaggtctgggaatgcgcaagatacgcatgccaccgctgcaaacaacattgcgcttctccggaaacattagc

SEQ ID NO: 679 - DNA, 102 bp, Artificial Sequence
  Synthetic Polynucleotide
acaaccgcgtgttacaaggccaggcatccgagaggtctgggaatgcttcgtccgagacaacgatatcgcccactttcattgcgcttctccggaaacattagc

SEQ ID NO: 680 - DNA, 102 bp, Artificial Sequence
  Synthetic Polynucleotide
acaaccgcgtgttacaaggccaggcatccgagaggtctgggaatgcctgccggacagcctggtaactgaccgtattcattgcgcttctccggaaacattagc

SEQ ID NO: 681 - DNA, 102 bp, Artificial Sequence
  Synthetic Polynucleotide
acaaccgcgtgttacaaggccaggcatccgagaggtctgggaatgccaggcctcagcggcagcgatcagtttatcgcattgcgcttctccggaaacattagc

SEQ ID NO: 682 - DNA, 102 bp, Artificial Sequence
  Synthetic Polynucleotide
acaaccgcgtgttacaaggccaggcatccgagaggtctgggaatgcttcgcaaccgccgagactgatagtttgacgcattgcgcttctccggaaacattagc

SEQ ID NO: 683 - DNA, 102 bp, Artificial Sequence
  Synthetic Polynucleotide
acaaccgcgtgttacaaggccaggcatccgagaggtctgggaatgccatcaggctggactgtttagcggcaacagccattgcgcttctccggaaacattagc

SEQ ID NO: 684 - DNA, 102 bp, Artificial Sequence
  Synthetic Polynucleotide
acaaccgcgtgttacaaggccaggcatccgagaggtctgggaatgcatcacatctggcttgcagtgttccaacagccattgcgcttctccggaaacattagc

SEQ ID NO: 685 - DNA, 102 bp, Artificial Sequence
  Synthetic Polynucleotide
acaaccgcgtgttacaaggccaggcatccgagaggtctgggaatgccgccagaccaacagaaccgttgatgaaagccattgcgcttctccggaaacattagc

SEQ ID NO: 686 - DNA, 102 bp, Artificial Sequence
  Synthetic Polynucleotide
acaaccgcgtgttacaaggccaggcatccgagaggtctgggaatgctcgaagctaagatgagactgttgatcggcccattgcgcttctccggaaacattagc

SEQ ID NO: 687 - DNA, 102 bp, Artificial Sequence
  Synthetic Polynucleotide
acaaccgcgtgttacaaggccaggcatccgagaggtctgggaatgctagccatgtgcaagtttctgcaccagtgaccattgcgcttctccggaaacattagc

SEQ ID NO: 688 - DNA, 102 bp, Artificial Sequence
  Synthetic Polynucleotide
acaaccgcgtgttacaaggccaggcatccgagaggtctgggaatgcggagatggcgcgtacgacaacaaacgggaccattgcgcttctccggaaacattagc

SEQ ID NO: 689 - DNA, 102 bp, Artificial Sequence
  Synthetic Polynucleotide
acaaccgcgtgttacaaggccaggcatccgagaggtctgggaatgcgcaacctcggttccattcagttggccggtacattgcgcttctccggaaacattagc

SEQ ID NO: 690 - DNA, 102 bp, Artificial Sequence
  Synthetic Polynucleotide
acaaccgcgtgttacaaggccaggcatccgagaggtctgggaatgccatgggcgattgccgtcgcttccatctctacattgcgcttctccggaaacattagc

SEQ ID NO: 691 - DNA, 102 bp, Artificial Sequence
  Synthetic Polynucleotide
acaaccgcgtgttacaaggccaggcatccgagaggtctgggaatgcccgcagcgactttaccgatgcccgatttcacattgcgcttctccggaaacattagc

SEQ ID NO: 692 - DNA, 102 bp, Artificial Sequence
  Synthetic Polynucleotide
acaaccgcgtgttacaaggccaggcatccgagaggtctgggaatgccgctaacaatcaggccacgtacagcgttaacattgcgcttctccggaaacattagc

SEQ ID NO: 693 - DNA, 102 bp, Artificial Sequence
  Synthetic Polynucleotide
acaaccgcgtgttacaaggccaggcatccgagaggtctgggaatgcccaaatgccgtgacatccgcgtcgtgataacattgcgcttctccggaaacattagc

SEQ ID NO: 694 - DNA, 102 bp, Artificial Sequence
  Synthetic Polynucleotide
acaaccgcgtgttacaaggccaggcatccgagaggtctgggaatgccctccggagtttgcggcttcagtttgatttcattgcgcttctccggaaacattagc

SEQ ID NO: 695 - DNA, 102 bp, Artificial Sequence
  Synthetic Polynucleotide
acaaccgcgtgttacaaggccaggcatccgagaggtctgggaatgcggaatacgcgcttcatgagcggcgacaattcattgcgcttctccggaaacattagc

SEQ ID NO: 696 - DNA, 102 bp, Artificial Sequence
  Synthetic Polynucleotide
acaaccgcgtgttacaaggccaggcatccgagaggtctgggaatgcctttaatggtggcgtccacttccgtcgggtcattgcgcttctccggaaacattagc

SEQ ID NO: 697 - DNA, 102 bp, Artificial Sequence
  Synthetic Polynucleotide
acaaccgcgtgttacaaggccaggcatccgagaggtctgggaatgcctcgcggtaacaattcgcggatcaccggatcattgcgcttctccggaaacattagc

SEQ ID NO: 698 - DNA, 102 bp, Artificial Sequence
  Synthetic Polynucleotide
acaaccgcgtgttacaaggccaggcatccgagaggtctgggaatgctcggcatcttcgctgaagccgtaagtcgtgcattgcgcttctccggaaacattagc

SEQ ID NO: 699 - DNA, 102 bp, Artificial Sequence
  Synthetic Polynucleotide
acaaccgcgtgttacaaggccaggcatccgagaggtctgggaatgcggtgacaatcgccaccatcggttgcagatgcattgcgcttctccggaaacattagc

SEQ ID NO: 700 - DNA, 102 bp, Artificial Sequence
  Synthetic Polynucleotide
acaaccgcgtgttacaaggccaggcatccgagaggtctgggaatgcttctcaaagtcgccctggtaggtatccatgcattgcgcttctccggaaacattagc

SEQ ID NO: 701 - DNA, 102 bp, Artificial Sequence
  Synthetic Polynucleotide
acaaccgcgtgttacaaggccaggcatccgagaggtctgggaatgcgcttctgcgtagatgctggaaaccatcgcgcattgcgcttctccggaaacattagc

SEQ ID NO: 702 - DNA, 102 bp, Artificial Sequence
  Synthetic Polynucleotide
acaaccgcgtgttacaaggccaggcatccgagaggtctgggaatgctagcctcgtcgtcaatgccctcttccgtagcattgcgcttctccggaaacattagc

SEQ ID NO: 703 - DNA, 102 bp, Artificial Sequence
  Synthetic Polynucleotide
acaaccgcgtgttacaaggccaggcatccgagaggtctgggaatgcttcattaactgctgcgtgaccggatttggccattgcgcttctccggaaacattagc

SEQ ID NO: 704 - DNA, 102 bp, Artificial Sequence
  Synthetic Polynucleotide
acaaccgcgtgttacaaggccaggcatccgagaggtctgggaatgcctgataaccttcattggccagaacttcggccattgcgcttctccggaaacattagc

SEQ ID NO: 705 - DNA, 102 bp, Artificial Sequence
  Synthetic Polynucleotide
acaaccgcgtgttacaaggccaggcatccgagaggtctgggaatgcaccattcactggctccagcgggaattcacccattgcgcttctccggaaacattagc

SEQ ID NO: 706 - DNA, 102 bp, Artificial Sequence
  Synthetic Polynucleotide
acaaccgcgtgttacaaggccaggcatccgagaggtctgggaatgcccgggcgatggttgaaataaatcgtcgcaccattgcgcttctccggaaacattagc

SEQ ID NO: 707 - DNA, 102 bp, Artificial Sequence
  Synthetic Polynucleotide
acaaccgcgtgttacaaggccaggcatccgagaggtctgggaatgcgcgggccaatctgctgataatcttctacaccattgcgcttctccggaaacattagc

SEQ ID NO: 708 - DNA, 102 bp, Artificial Sequence
  Synthetic Polynucleotide
acaaccgcgtgttacaaggccaggcatccgagaggtctgggaatgccacgtccacgaattgtgcgacacagcgaaccattgcgcttctccggaaacattagc

SEQ ID NO: 709 - DNA, 102 bp, Artificial Sequence
  Synthetic Polynucleotide
acaaccgcgtgttacaaggccaggcatccgagaggtctgggaatgcgttatcggcagaaatcgcgctggaaacaaccattgcgcttctccggaaacattagc

SEQ ID NO: 710 - DNA, 102 bp, Artificial Sequence
  Synthetic Polynucleotide
acaaccgcgtgttacaaggccaggcatccgagaggtctgggaatgccggttaataccggtgccagcatctcggctacattgcgcttctccggaaacattagc

SEQ ID NO: 711 - DNA, 102 bp, Artificial Sequence
  Synthetic Polynucleotide
acaaccgcgtgttacaaggccaggcatccgagaggtctgggaatgccgcattaactcagccagcatttcggcacgacattgcgcttctccggaaacattagc

SEQ ID NO: 712 - DNA, 102 bp, Artificial Sequence
  Synthetic Polynucleotide
acaaccgcgtgttacaaggccaggcatccgagaggtctgggaatgccttcgccagccggatacacttccagcatcacattgcgcttctccggaaacattagc

SEQ ID NO: 713 - DNA, 102 bp, Artificial Sequence
  Synthetic Polynucleotide
acaaccgcgtgttacaaggccaggcatccgagaggtctgggaatgcacgatgcatcactctcatctgcttcggcaacattgcgcttctccggaaacattagc

SEQ ID NO: 714 - DNA, 102 bp, Artificial Sequence
  Synthetic Polynucleotide
acaaccgcgtgttacaaggccaggcatccgagaggtctgggaatgcgtatcaacctgcgtcagcacattggcgaaacattgcgcttctccggaaacattagc

SEQ ID NO: 715 - DNA, 102 bp, Artificial Sequence
  Synthetic Polynucleotide
acaaccgcgtgttacaaggccaggcatccgagaggtctgggaatgccatcacgaggatctgcccgtcagtgacgttcattgcgcttctccggaaacattagc

SEQ ID NO: 716 - DNA, 102 bp, Artificial Sequence
  Synthetic Polynucleotide
acaaccgcgtgttacaaggccaggcatccgagaggtctgggaatgccaatgccaataaccgggatcgccagtgcttcattgcgcttctccggaaacattagc

SEQ ID NO: 717 - DNA, 102 bp, Artificial Sequence
  Synthetic Polynucleotide
acaaccgcgtgttacaaggccaggcatccgagaggtctgggaatgcgaccatgttagcaccggcacgcataaccgtcattgcgcttctccggaaacattagc

SEQ ID NO: 718 - DNA, 102 bp, Artificial Sequence
  Synthetic Polynucleotide
acaaccgcgtgttacaaggccaggcatccgagaggtctgggaatgctggcgaagctatagtcataagcggtgatggcattgcgcttctccggaaacattagc

SEQ ID NO: 719 - DNA, 102 bp, Artificial Sequence
  Synthetic Polynucleotide
acaaccgcgtgttacaaggccaggcatccgagaggtctgggaatgctaggaatgtgaccgccggtaataccaaaggcattgcgcttctccggaaacattagc

SEQ ID NO: 720 - DNA, 102 bp, Artificial Sequence
  Synthetic Polynucleotide
acaaccgcgtgttacaaggccaggcatccgagaggtctgggaatgctgtacttctgcagtaaggagatggtggtcgcattgcgcttctccggaaacattagc

SEQ ID NO: 721 - DNA, 102 bp, Artificial Sequence
  Synthetic Polynucleotide
acaaccgcgtgttacaaggccaggcatccgagaggtctgggaatgctggaaactgtgttcttcgcccggataaacgcattgcgcttctccggaaacattagc

SEQ ID NO: 722 - DNA, 102 bp, Artificial Sequence
  Synthetic Polynucleotide
acaaccgcgtgttacaaggccaggcatccgagaggtctgggaatgcagcagcttctaaggctaatgcatcgctgagcattgcgcttctccggaaacattagc

SEQ ID NO: 723 - DNA, 102 bp, Artificial Sequence
  Synthetic Polynucleotide
acaaccgcgtgttacaaggccaggcatccgagaggtctgggaatgcctccacttcagccatatactgccgcacagccattgcgcttctccggaaacattagc

SEQ ID NO: 724 - DNA, 102 bp, Artificial Sequence
  Synthetic Polynucleotide
acaaccgcgtgttacaaggccaggcatccgagaggtctgggaatgcaacctaagtgaccacatacaggaacggcaccattgcgcttctccggaaacattagc

SEQ ID NO: 725 - DNA, 102 bp, Artificial Sequence
  Synthetic Polynucleotide
acaaccgcgtgttacaaggccaggcatccgagaggtctgggaatgcgtcagcatttgtacggtttctaccagccaccattgcgcttctccggaaacattagc

SEQ ID NO: 726 - DNA, 102 bp, Artificial Sequence
  Synthetic Polynucleotide
acaaccgcgtgttacaaggccaggcatccgagaggtctgggaatgcgcagtgtggtaggcgatatcggcaacggtacattgcgcttctccggaaacattagc

SEQ ID NO: 727 - DNA, 102 bp, Artificial Sequence
  Synthetic Polynucleotide
acaaccgcgtgttacaaggccaggcatccgagaggtctgggaatgccatacgccataaacggcaggtcagccagcacattgcgcttctccggaaacattagc

SEQ ID NO: 728 - DNA, 102 bp, Artificial Sequence
  Synthetic Polynucleotide
acaaccgcgtgttacaaggccaggcatccgagaggtctgggaatgcccagcgaatcgcccaccagcatgacgttaacattgcgcttctccggaaacattagc

SEQ ID NO: 729 - DNA, 102 bp, Artificial Sequence
  Synthetic Polynucleotide
acaaccgcgtgttacaaggccaggcatccgagaggtctgggaatgcccaggcggctaccagaattactgcccgtttcattgcgcttctccggaaacattagc

SEQ ID NO: 730 - DNA, 102 bp, Artificial Sequence
  Synthetic Polynucleotide
acaaccgcgtgttacaaggccaggcatccgagaggtctgggaatgcgatgtccggctggaccaggttgaacagcttcattgcgcttctccggaaacattagc

SEQ ID NO: 731 - DNA, 102 bp, Artificial Sequence
  Synthetic Polynucleotide
acaaccgcgtgttacaaggccaggcatccgagaggtctgggaatgccttgccttccatacgcaggcggcgaatttgcattgcgcttctccggaaacattagc

SEQ ID NO: 732 - DNA, 102 bp, Artificial Sequence
  Synthetic Polynucleotide
acaaccgcgtgttacaaggccaggcatccgagaggtctgggaatgcacgtttgtttagcttctcgcagtcctcctgcattgcgcttctccggaaacattagc

SEQ ID NO: 733 - DNA, 102 bp, Artificial Sequence
  Synthetic Polynucleotide
acaaccgcgtgttacaaggccaggcatccgagaggtctgggaatgcacgtaagtgtgggtttcagtaccgttcgggcattgcgcttctccggaaacattagc

SEQ ID NO: 734 - DNA, 102 bp, Artificial Sequence
  Synthetic Polynucleotide
acaaccgcgtgttacaaggccaggcatccgagaggtctgggaatgcgcgttgttccgccgtcagataaccgttacgcattgcgcttctccggaaacattagc

SEQ ID NO: 735 - DNA, 102 bp, Artificial Sequence
  Synthetic Polynucleotide
acaaccgcgtgttacaaggccaggcatccgagaggtctgggaatgcatcgtgcaggttacccatggtaggcaccagcattgcgcttctccggaaacattagc

SEQ ID NO: 736 - DNA, 102 bp, Artificial Sequence
  Synthetic Polynucleotide
acaaccgcgtgttacaaggccaggcatccgagaggtctgggaatgccagaccgtctttggcgcgcataattggcaccattgcgcttctccggaaacattagc

SEQ ID NO: 737 - DNA, 102 bp, Artificial Sequence
  Synthetic Polynucleotide
acaaccgcgtgttacaaggccaggcatccgagaggtctgggaatgccgggctttggcttcgtcgaccagcttcatacattgcgcttctccggaaacattagc

SEQ ID NO: 738 - DNA, 102 bp, Artificial Sequence
  Synthetic Polynucleotide
acaaccgcgtgttacaaggccaggcatccgagaggtctgggaatgcgcagcagcggcagggtttcgataattaacacattgcgcttctccggaaacattagc

SEQ ID NO: 739 - DNA, 102 bp, Artificial Sequence
  Synthetic Polynucleotide
acaaccgcgtgttacaaggccaggcatccgagaggtctgggaatgccaccttccagcatggtcgaaaggccaggaacattgcgcttctccggaaacattagc

SEQ ID NO: 740 - DNA, 102 bp, Artificial Sequence
  Synthetic Polynucleotide
acaaccgcgtgttacaaggccaggcatccgagaggtctgggaatgcccgcatgagtcactttcacgcggtggagttcattgcgcttctccggaaacattagc

SEQ ID NO: 741 - DNA, 102 bp, Artificial Sequence
  Synthetic Polynucleotide
acaaccgcgtgttacaaggccaggcatccgagaggtctgggaatgcccaggtgcgagcttcttcatctggcatggtcattgcgcttctccggaaacattagc

SEQ ID NO: 742 - DNA, 102 bp, Artificial Sequence
  Synthetic Polynucleotide
acaaccgcgtgttacaaggccaggcatccgagaggtctgggaatgcgccgcgatggcataagtggagaaacgcttgcattgcgcttctccggaaacattagc

SEQ ID NO: 743 - DNA, 102 bp, Artificial Sequence
  Synthetic Polynucleotide
acaaccgcgtgttacaaggccaggcatccgagaggtctgggaatgctcctggtcaatggcgcaagaaccttcatagcattgcgcttctccggaaacattagc

SEQ ID NO: 744 - DNA, 102 bp, Artificial Sequence
  Synthetic Polynucleotide
acaaccgcgtgttacaaggccaggcatccgagaggtctgggaatgctcaagcaacctgtaccggaatcgctttcgccattgcgcttctccggaaacattagc

SEQ ID NO: 745 - DNA, 102 bp, Artificial Sequence
  Synthetic Polynucleotide
acaaccgcgtgttacaaggccaggcatccgagaggtctgggaatgcagctggcgatgatgacaatatcgccgacaccattgcgcttctccggaaacattagc

SEQ ID NO: 746 - DNA, 102 bp, Artificial Sequence
  Synthetic Polynucleotide
acaaccgcgtgttacaaggccaggcatccgagaggtctgggaatgccagtgggccgccgcaccgttaacagaaatacattgcgcttctccggaaacattagc

SEQ ID NO: 747 - DNA, 102 bp, Artificial Sequence
  Synthetic Polynucleotide
acaaccgcgtgttacaaggccaggcatccgagaggtctgggaatgccgaaagcgtcgtgataggtcaggccgctttcattgcgcttctccggaaacattagc

SEQ ID NO: 748 - DNA, 102 bp, Artificial Sequence
  Synthetic Polynucleotide
acaaccgcgtgttacaaggccaggcatccgagaggtctgggaatgcggtttccgggctgatgcgcatacccaatttcattgcgcttctccggaaacattagc

SEQ ID NO: 749 - DNA, 102 bp, Artificial Sequence
  Synthetic Polynucleotide
acaaccgcgtgttacaaggccaggcatccgagaggtctgggaatgcctgcaactgccagatatcgcgggttaatgtcattgcgcttctccggaaacattagc

SEQ ID NO: 750 - DNA, 102 bp, Artificial Sequence
  Synthetic Polynucleotide
acaaccgcgtgttacaaggccaggcatccgagaggtctgggaatgcggaacgccgggttcacgcgcatatcgttatcattgcgcttctccggaaacattagc

SEQ ID NO: 751 - DNA, 102 bp, Artificial Sequence
  Synthetic Polynucleotide
acaaccgcgtgttacaaggccaggcatccgagaggtctgggaatgccgcggtgacggttcttcatccagctcgttgcattgcgcttctccggaaacattagc

SEQ ID NO: 752 - DNA, 102 bp, Artificial Sequence
  Synthetic Polynucleotide
acaaccgcgtgttacaaggccaggcatccgagaggtctgggaatgcgccgtctccagcagtgggtaccagaacatgcattgcgcttctccggaaacattagc

SEQ ID NO: 753 - DNA, 102 bp, Artificial Sequence
  Synthetic Polynucleotide
acaaccgcgtgttacaaggccaggcatccgagaggtctgggaatgcatacaggctgttgatagtgaaatcgcggcgcattgcgcttctccggaaacattagc

SEQ ID NO: 754 - DNA, 102 bp, Artificial Sequence
  Synthetic Polynucleotide
acaaccgcgtgttacaaggccaggcatccgagaggtctgggaatgcgtttaagcgattcttcaaacaggcgtgccgcattgcgcttctccggaaacattagc

SEQ ID NO: 755 - DNA, 102 bp, Artificial Sequence
  Synthetic Polynucleotide
acaaccgcgtgttacaaggccaggcatccgagaggtctgggaatgcacagcttataggtttcgtaaccgtagcccgcattgcgcttctccggaaacattagc

SEQ ID NO: 756 - DNA, 102 bp, Artificial Sequence
  Synthetic Polynucleotide
acaaccgcgtgttacaaggccaggcatccgagaggtctgggaatgcgcagttacggaacagtttgcgcacctgctccattgcgcttctccggaaacattagc

SEQ ID NO: 757 - DNA, 102 bp, Artificial Sequence
  Synthetic Polynucleotide
acaaccgcgtgttacaaggccaggcatccgagaggtctgggaatgctttccgggttaccaatcagacggataacgccattgcgcttctccggaaacattagc

SEQ ID NO: 758 - DNA, 102 bp, Artificial Sequence
  Synthetic Polynucleotide
acaaccgcgtgttacaaggccaggcatccgagaggtctgggaatgctcataagccgcacggaacttaggatgctcccattgcgcttctccggaaacattagc

SEQ ID NO: 759 - DNA, 102 bp, Artificial Sequence
  Synthetic Polynucleotide
acaaccgcgtgttacaaggccaggcatccgagaggtctgggaatgctcagatccttcatgccgccaacgtaatcaccattgcgcttctccggaaacattagc

SEQ ID NO: 760 - DNA, 102 bp, Artificial Sequence
  Synthetic Polynucleotide
acaaccgcgtgttacaaggccaggcatccgagaggtctgggaatgcggtcgctgacgttaccttcgtggtgtccaccattgcgcttctccggaaacattagc

SEQ ID NO: 761 - DNA, 102 bp, Artificial Sequence
  Synthetic Polynucleotide
acaaccgcgtgttacaaggccaggcatccgagaggtctgggaatgcgtcgcaacttcgataatctccgggccaaaccattgcgcttctccggaaacattagc

SEQ ID NO: 762 - DNA, 102 bp, Artificial Sequence
  Synthetic Polynucleotide
acaaccgcgtgttacaaggccaggcatccgagaggtctgggaatgcccaaccagccaggcttcgtatcccgctttacattgcgcttctccggaaacattagc

SEQ ID NO: 763 - DNA, 102 bp, Artificial Sequence
  Synthetic Polynucleotide
acaaccgcgtgttacaaggccaggcatccgagaggtctgggaatgcgcgcagcatacgtaccggatcttcacggtacattgcgcttctccggaaacattagc

SEQ ID NO: 764 - DNA, 102 bp, Artificial Sequence
  Synthetic Polynucleotide
acaaccgcgtgttacaaggccaggcatccgagaggtctgggaatgccatgcgcgtttaccctgacgacgggacatacattgcgcttctccggaaacattagc

SEQ ID NO: 765 - DNA, 102 bp, Artificial Sequence
  Synthetic Polynucleotide
acaaccgcgtgttacaaggccaggcatccgagaggtctgggaatgccgcgtatcggtattcttcagcacctgttcacattgcgcttctccggaaacattagc

SEQ ID NO: 766 - DNA, 102 bp, Artificial Sequence
  Synthetic Polynucleotide
acaaccgcgtgttacaaggccaggcatccgagaggtctgggaatgccgttacgctcaacttcagctcgcaaggccacattgcgcttctccggaaacattagc

SEQ ID NO: 767 - DNA, 102 bp, Artificial Sequence
  Synthetic Polynucleotide
acaaccgcgtgttacaaggccaggcatccgagaggtctgggaatgcccgtgaagtagcgggtaatggtcgggaacacattgcgcttctccggaaacattagc

SEQ ID NO: 768 - DNA, 102 bp, Artificial Sequence
  Synthetic Polynucleotide
acaaccgcgtgttacaaggccaggcatccgagaggtctgggaatgcccggatcagcggtaaacacgccgtcaacttcattgcgcttctccggaaacattagc

SEQ ID NO: 769 - DNA, 102 bp, Artificial Sequence
  Synthetic Polynucleotide
acaaccgcgtgttacaaggccaggcatccgagaggtctgggaatgcgcaacaggctgatagcttctgcccagctgtcattgcgcttctccggaaacattagc

SEQ ID NO: 770 - DNA, 102 bp, Artificial Sequence
  Synthetic Polynucleotide
acaaccgcgtgttacaaggccaggcatccgagaggtctgggaatgcccagcacttcgctgtaagtcagttgctcgtcattgcgcttctccggaaacattagc

SEQ ID NO: 771 - DNA, 102 bp, Artificial Sequence
  Synthetic Polynucleotide
acaaccgcgtgttacaaggccaggcatccgagaggtctgggaatgcgctttcagcaccacatcggcttcaatttcgcattgcgcttctccggaaacattagc

SEQ ID NO: 772 - DNA, 102 bp, Artificial Sequence
  Synthetic Polynucleotide
acaaccgcgtgttacaaggccaggcatccgagaggtctgggaatgcaccaatcaccacaccaacctgaatacccagcattgcgcttctccggaaacattagc

SEQ ID NO: 773 - DNA, 102 bp, Artificial Sequence
  Synthetic Polynucleotide
acaaccgcgtgttacaaggccaggcatccgagaggtctgggaatgcttcctgagccatacgatccagtatgcttgccattgcgcttctccggaaacattagc

SEQ ID NO: 774 - DNA, 102 bp, Artificial Sequence
  Synthetic Polynucleotide
acaaccgcgtgttacaaggccaggcatccgagaggtctgggaatgccgaatcggtaatttatggtcacgagccagccattgcgcttctccggaaacattagc

SEQ ID NO: 775 - DNA, 102 bp, Artificial Sequence
  Synthetic Polynucleotide
acaaccgcgtgttacaaggccaggcatccgagaggtctgggaatgctcgcacacgccattcaatggaatagcggaccattgcgcttctccggaaacattagc

SEQ ID NO: 776 - DNA, 102 bp, Artificial Sequence
  Synthetic Polynucleotide
acaaccgcgtgttacaaggccaggcatccgagaggtctgggaatgcgtgccctgcagagcttcgccactcaacttacattgcgcttctccggaaacattagc

SEQ ID NO: 777 - DNA, 102 bp, Artificial Sequence
  Synthetic Polynucleotide
acaaccgcgtgttacaaggccaggcatccgagaggtctgggaatgcgcaggcaagctgctgagtcggtggtaaagacattgcgcttctccggaaacattagc

SEQ ID NO: 778 - DNA, 102 bp, Artificial Sequence
  Synthetic Polynucleotide
acaaccgcgtgttacaaggccaggcatccgagaggtctgggaatgcttacctgtaccggcggagaggatcaccacacattgcgcttctccggaaacattagc

SEQ ID NO: 779 - DNA, 102 bp, Artificial Sequence
  Synthetic Polynucleotide
acaaccgcgtgttacaaggccaggcatccgagaggtctgggaatgcccatcgactttaacgatcctgtcgcctgctcattgcgcttctccggaaacattagc

SEQ ID NO: 780 - DNA, 102 bp, Artificial Sequence
  Synthetic Polynucleotide
acaaccgcgtgttacaaggccaggcatccgagaggtctgggaatgccttcgacgatggcgttgaacggcccatactcattgcgcttctccggaaacattagc

SEQ ID NO: 781 - DNA, 102 bp, Artificial Sequence
  Synthetic Polynucleotide
acaaccgcgtgttacaaggccaggcatccgagaggtctgggaatgcttggcgatagagatcggcccactgaggttgcattgcgcttctccggaaacattagc

SEQ ID NO: 782 - DNA, 102 bp, Artificial Sequence
  Synthetic Polynucleotide
acaaccgcgtgttacaaggccaggcatccgagaggtctgggaatgcacgtaaatcgagctttacatcccgccgttgcattgcgcttctccggaaacattagc

SEQ ID NO: 783 - DNA, 102 bp, Artificial Sequence
  Synthetic Polynucleotide
acaaccgcgtgttacaaggccaggcatccgagaggtctgggaatgcccgggcaacccagaaatgaccaaattcatgcattgcgcttctccggaaacattagc

SEQ ID NO: 784 - DNA, 102 bp, Artificial Sequence
  Synthetic Polynucleotide
acaaccgcgtgttacaaggccaggcatccgagaggtctgggaatgcgcatcacaaaggtcacccactgcgttaaggcattgcgcttctccggaaacattagc

SEQ ID NO: 785 - DNA, 102 bp, Artificial Sequence
  Synthetic Polynucleotide
acaaccgcgtgttacaaggccaggcatccgagaggtctgggaatgctattattgaaggcatggtggcggagttccgcattgcgcttctccggaaacattagc

SEQ ID NO: 786 - DNA, 102 bp, Artificial Sequence
  Synthetic Polynucleotide
acaaccgcgtgttacaaggccaggcatccgagaggtctgggaatgctcgctttaccattacccggtttactctccgcattgcgcttctccggaaacattagc

SEQ ID NO: 787 - DNA, 102 bp, Artificial Sequence
  Synthetic Polynucleotide
acaaccgcgtgttacaaggccaggcatccgagaggtctgggaatgctaacgctaaggatttacccgggttatcccgcattgcgcttctccggaaacattagc

SEQ ID NO: 788 - DNA, 102 bp, Artificial Sequence
  Synthetic Polynucleotide
acaaccgcgtgttacaaggccaggcatccgagaggtctgggaatgcccagtacaggttcaatttgcggcccacgagcattgcgcttctccggaaacattagc

SEQ ID NO: 789 - DNA, 102 bp, Artificial Sequence
  Synthetic Polynucleotide
acaaccgcgtgttacaaggccaggcatccgagaggtctgggaatgcgttcacgctaataagcgcaagaaacggcagcattgcgcttctccggaaacattagc

SEQ ID NO: 790 - DNA, 102 bp, Artificial Sequence
  Synthetic Polynucleotide
acaaccgcgtgttacaaggccaggcatccgagaggtctgggaatgcgcccaacgggatcagggcgataacatattccattgcgcttctccggaaacattagc

SEQ ID NO: 791 - DNA, 102 bp, Artificial Sequence
  Synthetic Polynucleotide
acaaccgcgtgttacaaggccaggcatccgagaggtctgggaatgcctcatctggcaaaggaatgactttcggctccattgcgcttctccggaaacattagc

SEQ ID NO: 792 - DNA, 102 bp, Artificial Sequence
  Synthetic Polynucleotide
acaaccgcgtgttacaaggccaggcatccgagaggtctgggaatgcgaccaactgcaaacgcacggcatcccaatccattgcgcttctccggaaacattagc

SEQ ID NO: 793 - DNA, 102 bp, Artificial Sequence
  Synthetic Polynucleotide
acaaccgcgtgttacaaggccaggcatccgagaggtctgggaatgctgccaaatggcgctactgtaatggtggtgccattgcgcttctccggaaacattagc

SEQ ID NO: 794 - DNA, 102 bp, Artificial Sequence
  Synthetic Polynucleotide
acaaccgcgtgttacaaggccaggcatccgagaggtctgggaatgcttaacagcaccagcagaatcgagccaatgccattgcgcttctccggaaacattagc

SEQ ID NO: 795 - DNA, 102 bp, Artificial Sequence
  Synthetic Polynucleotide
acaaccgcgtgttacaaggccaggcatccgagaggtctgggaatgccccagcatactgaccgtcagcttcatcagccattgcgcttctccggaaacattagc

SEQ ID NO: 796 - DNA, 102 bp, Artificial Sequence
  Synthetic Polynucleotide
acaaccgcgtgttacaaggccaggcatccgagaggtctgggaatgcaagtacacccagtgcaacgatgaacgaagccattgcgcttctccggaaacattagc

SEQ ID NO: 797 - DNA, 102 bp, Artificial Sequence
  Synthetic Polynucleotide
acaaccgcgtgttacaaggccaggcatccgagaggtctgggaatgcagttccgtacctggtgcaatttgtgcttcccattgcgcttctccggaaacattagc

SEQ ID NO: 798 - DNA, 102 bp, Artificial Sequence
  Synthetic Polynucleotide
acaaccgcgtgttacaaggccaggcatccgagaggtctgggaatgcaccggatcttctttatcaggctcaaacgcccattgcgcttctccggaaacattagc

SEQ ID NO: 799 - DNA, 102 bp, Artificial Sequence
  Synthetic Polynucleotide
acaaccgcgtgttacaaggccaggcatccgagaggtctgggaatgcatcgaattggctgctatttcgccaaccacccattgcgcttctccggaaacattagc

SEQ ID NO: 800 - DNA, 102 bp, Artificial Sequence
  Synthetic Polynucleotide
acaaccgcgtgttacaaggccaggcatccgagaggtctgggaatgcgcttatcagttcgccgccagagcgccttaccattgcgcttctccggaaacattagc

SEQ ID NO: 801 - DNA, 102 bp, Artificial Sequence
  Synthetic Polynucleotide
acaaccgcgtgttacaaggccaggcatccgagaggtctgggaatgccctattgagaaacgctcaacgcgaacaccacattgcgcttctccggaaacattagc

SEQ ID NO: 802 - DNA, 102 bp, Artificial Sequence
  Synthetic Polynucleotide
acaaccgcgtgttacaaggccaggcatccgagaggtctgggaatgctgaagtttgcaaccggacctgcggcaataacattgcgcttctccggaaacattagc

SEQ ID NO: 803 - DNA, 102 bp, Artificial Sequence
  Synthetic Polynucleotide
acaaccgcgtgttacaaggccaggcatccgagaggtctgggaatgccgccgttacgtggtgcatcagcatgatgttcattgcgcttctccggaaacattagc

SEQ ID NO: 804 - DNA, 102 bp, Artificial Sequence
  Synthetic Polynucleotide
acaaccgcgtgttacaaggccaggcatccgagaggtctgggaatgccgttctggatctgcacaccttctttcgcttcattgcgcttctccggaaacattagc

SEQ ID NO: 805 - DNA, 102 bp, Artificial Sequence
  Synthetic Polynucleotide
acaaccgcgtgttacaaggccaggcatccgagaggtctgggaatgcccatctccggttccatggcattgatgatgtcattgcgcttctccggaaacattagc

SEQ ID NO: 806 - DNA, 102 bp, Artificial Sequence
  Synthetic Polynucleotide
acaaccgcgtgttacaaggccaggcatccgagaggtctgggaatgccgttggcaatcgctttagtcacccacgggtcattgcgcttctccggaaacattagc

SEQ ID NO: 807 - DNA, 102 bp, Artificial Sequence
  Synthetic Polynucleotide
acaaccgcgtgttacaaggccaggcatccgagaggtctgggaatgctacgcatcagcgcatcttccatcgacaggtcattgcgcttctccggaaacattagc

SEQ ID NO: 808 - DNA, 102 bp, Artificial Sequence
  Synthetic Polynucleotide
acaaccgcgtgttacaaggccaggcatccgagaggtctgggaatgccaggtgctctttccacagggagtcaagcgtcattgcgcttctccggaaacattagc

SEQ ID NO: 809 - DNA, 102 bp, Artificial Sequence
  Synthetic Polynucleotide
acaaccgcgtgttacaaggccaggcatccgagaggtctgggaatgccgctcacgcagcgtctcttcatgcagttctcattgcgcttctccggaaacattagc

SEQ ID NO: 810 - DNA, 102 bp, Artificial Sequence
  Synthetic Polynucleotide
acaaccgcgtgttacaaggccaggcatccgagaggtctgggaatgcgacgaccagaacgaccgcgcaactggttatcattgcgcttctccggaaacattagc

SEQ ID NO: 811 - DNA, 102 bp, Artificial Sequence
  Synthetic Polynucleotide
acaaccgcgtgttacaaggccaggcatccgagaggtctgggaatgcctgcctgccagctaccaccgagcacaatatcattgcgcttctccggaaacattagc

SEQ ID NO: 812 - DNA, 102 bp, Artificial Sequence
  Synthetic Polynucleotide
acaaccgcgtgttacaaggccaggcatccgagaggtctgggaatgcacgggattcgtgacgctcggtaccgatgatcattgcgcttctccggaaacattagc

SEQ ID NO: 813 - DNA, 102 bp, Artificial Sequence
  Synthetic Polynucleotide
acaaccgcgtgttacaaggccaggcatccgagaggtctgggaatgccacgggcaaggatcgttacgtcctactttgcattgcgcttctccggaaacattagc

SEQ ID NO: 814 - DNA, 102 bp, Artificial Sequence
  Synthetic Polynucleotide
acaaccgcgtgttacaaggccaggcatccgagaggtctgggaatgctatcccacatttcttccagcgactgtggtgcattgcgcttctccggaaacattagc

SEQ ID NO: 815 - DNA, 102 bp, Artificial Sequence
  Synthetic Polynucleotide
acaaccgcgtgttacaaggccaggcatccgagaggtctgggaatgcggagtccacttcgtccaccagcgcatagtgcattgcgcttctccggaaacattagc

SEQ ID NO: 816 - DNA, 102 bp, Artificial Sequence
  Synthetic Polynucleotide
acaaccgcgtgttacaaggccaggcatccgagaggtctgggaatgccataccgccgagtaactgaacgtcgaagtgcattgcgcttctccggaaacattagc

SEQ ID NO: 817 - DNA, 102 bp, Artificial Sequence
  Synthetic Polynucleotide
acaaccgcgtgttacaaggccaggcatccgagaggtctgggaatgcgatggagatagtacccaccagcaccggctgcattgcgcttctccggaaacattagc

SEQ ID NO: 818 - DNA, 102 bp, Artificial Sequence
  Synthetic Polynucleotide
acaaccgcgtgttacaaggccaggcatccgagaggtctgggaatgcttcaacgactccagcatcgctgcaaacatgcattgcgcttctccggaaacattagc

SEQ ID NO: 819 - DNA, 102 bp, Artificial Sequence
  Synthetic Polynucleotide
acaaccgcgtgttacaaggccaggcatccgagaggtctgggaatgcttatacatttccgagctgtcttctgccgggcattgcgcttctccggaaacattagc

SEQ ID NO: 820 - DNA, 102 bp, Artificial Sequence
  Synthetic Polynucleotide
acaaccgcgtgttacaaggccaggcatccgagaggtctgggaatgctgcacgcctttaccggttagtgcgttcaggcattgcgcttctccggaaacattagc

SEQ ID NO: 821 - DNA, 102 bp, Artificial Sequence
  Synthetic Polynucleotide
acaaccgcgtgttacaaggccaggcatccgagaggtctgggaatgcctgttgttccagctcctcaacctcttcaggcattgcgcttctccggaaacattagc

SEQ ID NO: 822 - DNA, 102 bp, Artificial Sequence
  Synthetic Polynucleotide
acaaccgcgtgttacaaggccaggcatccgagaggtctgggaatgcttgtcgcgcaggtagtcaaagccgtattcgcattgcgcttctccggaaacattagc

SEQ ID NO: 823 - DNA, 102 bp, Artificial Sequence
  Synthetic Polynucleotide
acaaccgcgtgttacaaggccaggcatccgagaggtctgggaatgcacagacggaagtagttctggaaggtgatcgcattgcgcttctccggaaacattagc

SEQ ID NO: 824 - DNA, 102 bp, Artificial Sequence
  Synthetic Polynucleotide
acaaccgcgtgttacaaggccaggcatccgagaggtctgggaatgcttatccagccactcggcaattggcaaatcgcattgcgcttctccggaaacattagc

SEQ ID NO: 825 - DNA, 102 bp, Artificial Sequence
  Synthetic Polynucleotide
acaaccgcgtgttacaaggccaggcatccgagaggtctgggaatgctacgctgtacacgttcttcagggctgaacgcattgcgcttctccggaaacattagc

SEQ ID NO: 826 - DNA, 102 bp, Artificial Sequence
  Synthetic Polynucleotide
acaaccgcgtgttacaaggccaggcatccgagaggtctgggaatgccgcttcgttggcgtggaatttggcgttcagcattgcgcttctccggaaacattagc

SEQ ID NO: 827 - DNA, 102 bp, Artificial Sequence
  Synthetic Polynucleotide
acaaccgcgtgttacaaggccaggcatccgagaggtctgggaatgccatgcccggcaggttgataccgacagtcagcattgcgcttctccggaaacattagc

SEQ ID NO: 828 - DNA, 102 bp, Artificial Sequence
  Synthetic Polynucleotide
acaaccgcgtgttacaaggccaggcatccgagaggtctgggaatgccgcttcagtcatgtagaccaggtccggcagcattgcgcttctccggaaacattagc

SEQ ID NO: 829 - DNA, 102 bp, Artificial Sequence
  Synthetic Polynucleotide
acaaccgcgtgttacaaggccaggcatccgagaggtctgggaatgcttcatccatgatgccctctttcaccagcagcattgcgcttctccggaaacattagc

SEQ ID NO: 830 - DNA, 102 bp, Artificial Sequence
  Synthetic Polynucleotide
acaaccgcgtgttacaaggccaggcatccgagaggtctgggaatgcaacgatgtagtcgacgtcacgggtaaacagcattgcgcttctccggaaacattagc

SEQ ID NO: 831 - DNA, 102 bp, Artificial Sequence
  Synthetic Polynucleotide
acaaccgcgtgttacaaggccaggcatccgagaggtctgggaatgccgagaagtggccttcgccctggaaggtttccattgcgcttctccggaaacattagc

SEQ ID NO: 832 - DNA, 102 bp, Artificial Sequence
  Synthetic Polynucleotide
acaaccgcgtgttacaaggccaggcatccgagaggtctgggaatgcccacgacccgccatattggtcgcgatagtccattgcgcttctccggaaacattagc

SEQ ID NO: 833 - DNA, 102 bp, Artificial Sequence
  Synthetic Polynucleotide
acaaccgcgtgttacaaggccaggcatccgagaggtctgggaatgcaggtggataccctgacgcagatagtccatccattgcgcttctccggaaacattagc

SEQ ID NO: 834 - DNA, 102 bp, Artificial Sequence
  Synthetic Polynucleotide
acaaccgcgtgttacaaggccaggcatccgagaggtctgggaatgcgcagttgcttacgaatgtcgaagttacggccattgcgcttctccggaaacattagc

SEQ ID NO: 835 - DNA, 102 bp, Artificial Sequence
  Synthetic Polynucleotide
acaaccgcgtgttacaaggccaggcatccgagaggtctgggaatgctttacgctgatacacttcgatggactgcgccattgcgcttctccggaaacattagc

SEQ ID NO: 836 - DNA, 102 bp, Artificial Sequence
  Synthetic Polynucleotide
acaaccgcgtgttacaaggccaggcatccgagaggtctgggaatgcacagttcgttacgctgggagtaaatggcgccattgcgcttctccggaaacattagc

SEQ ID NO: 837 - DNA, 102 bp, Artificial Sequence
  Synthetic Polynucleotide
acaaccgcgtgttacaaggccaggcatccgagaggtctgggaatgcgcttcgcctggcttcatacccagtttacgccattgcgcttctccggaaacattagc

SEQ ID NO: 838 - DNA, 102 bp, Artificial Sequence
  Synthetic Polynucleotide
acaaccgcgtgttacaaggccaggcatccgagaggtctgggaatgccgtaccgtaagtgatgtcagctgcgtaagccattgcgcttctccggaaacattagc

SEQ ID NO: 839 - DNA, 102 bp, Artificial Sequence
  Synthetic Polynucleotide
acaaccgcgtgttacaaggccaggcatccgagaggtctgggaatgccctgcttccagtaccgcatcgtgacgtacccattgcgcttctccggaaacattagc

SEQ ID NO: 840 - DNA, 102 bp, Artificial Sequence
  Synthetic Polynucleotide
acaaccgcgtgttacaaggccaggcatccgagaggtctgggaatgcataccggctttggtcagttcgtttgacacccattgcgcttctccggaaacattagc

SEQ ID NO: 841 - DNA, 102 bp, Artificial Sequence
  Synthetic Polynucleotide
acaaccgcgtgttacaaggccaggcatccgagaggtctgggaatgcgctgttaatggtttcgctcacatcgctgaccattgcgcttctccggaaacattagc

SEQ ID NO: 842 - DNA, 102 bp, Artificial Sequence
  Synthetic Polynucleotide
acaaccgcgtgttacaaggccaggcatccgagaggtctgggaatgcacgaatcattggacggttggtcggaacaaccattgcgcttctccggaaacattagc

SEQ ID NO: 843 - DNA, 102 bp, Artificial Sequence
  Synthetic Polynucleotide
acaaccgcgtgttacaaggccaggcatccgagaggtctgggaatgcgtacgcatttcggcgatgcagcgttcgttacattgcgcttctccggaaacattagc

SEQ ID NO: 844 - DNA, 102 bp, Artificial Sequence
  Synthetic Polynucleotide
acaaccgcgtgttacaaggccaggcatccgagaggtctgggaatgctaccaaagacgcgcttacttgcctcacgtacattgcgcttctccggaaacattagc

SEQ ID NO: 845 - DNA, 102 bp, Artificial Sequence
  Synthetic Polynucleotide
acaaccgcgtgttacaaggccaggcatccgagaggtctgggaatgctgcatttgcgctaaacgctcggcttccatacattgcgcttctccggaaacattagc

SEQ ID NO: 846 - DNA, 102 bp, Artificial Sequence
  Synthetic Polynucleotide
acaaccgcgtgttacaaggccaggcatccgagaggtctgggaatgcgcatgacgcctttctcgaagtgacgcatcacattgcgcttctccggaaacattagc

SEQ ID NO: 847 - DNA, 102 bp, Artificial Sequence
  Synthetic Polynucleotide
acaaccgcgtgttacaaggccaggcatccgagaggtctgggaatgccacgttgcgccaggtagtcgttgacggtaacattgcgcttctccggaaacattagc

SEQ ID NO: 848 - DNA, 102 bp, Artificial Sequence
  Synthetic Polynucleotide
acaaccgcgtgttacaaggccaggcatccgagaggtctgggaatgccggctgcagagtcgtcatcctgatggctaacattgcgcttctccggaaacattagc

SEQ ID NO: 849 - DNA, 102 bp, Artificial Sequence
  Synthetic Polynucleotide
acaaccgcgtgttacaaggccaggcatccgagaggtctgggaatgccctgcatggtacgaccggtgtgttcgtcaacattgcgcttctccggaaacattagc

SEQ ID NO: 850 - DNA, 102 bp, Artificial Sequence
  Synthetic Polynucleotide
acaaccgcgtgttacaaggccaggcatccgagaggtctgggaatgcaccatccctaataagagatgcggccagaagcattgcgcttctccggaaacattagc

SEQ ID NO: 851 - DNA, 102 bp, Artificial Sequence
  Synthetic Polynucleotide
acaaccgcgtgttacaaggccaggcatccgagaggtctgggaatgccagcgcgctgagcgtatccagtaatgcaagcattgcgcttctccggaaacattagc

SEQ ID NO: 852 - DNA, 102 bp, Artificial Sequence
  Synthetic Polynucleotide
acaaccgcgtgttacaaggccaggcatccgagaggtctgggaatgcttcgcttccagcaaggccaattgaccaaagcattgcgcttctccggaaacattagc

SEQ ID NO: 853 - DNA, 102 bp, Artificial Sequence
  Synthetic Polynucleotide
acaaccgcgtgttacaaggccaggcatccgagaggtctgggaatgcgcgttgctgagcgcaggcaaacctaaactccattgcgcttctccggaaacattagc

SEQ ID NO: 854 - DNA, 102 bp, Artificial Sequence
  Synthetic Polynucleotide
acaaccgcgtgttacaaggccaggcatccgagaggtctgggaatgcaatcaacggaatagttcgaattcgggcggccattgcgcttctccggaaacattagc

SEQ ID NO: 855 - DNA, 102 bp, Artificial Sequence
  Synthetic Polynucleotide
acaaccgcgtgttacaaggccaggcatccgagaggtctgggaatgcgcgcctgaagaggcaaagattcttcagcaacattgcgcttctccggaaacattagc

SEQ ID NO: 856 - DNA, 102 bp, Artificial Sequence
  Synthetic Polynucleotide
acaaccgcgtgttacaaggccaggcatccgagaggtctgggaatgcccagaatagtgacgctggcaccctgtggttcattgcgcttctccggaaacattagc

SEQ ID NO: 857 - DNA, 102 bp, Artificial Sequence
  Synthetic Polynucleotide
acaaccgcgtgttacaaggccaggcatccgagaggtctgggaatgcgcggagaaatcacgccgcaggtagagacttcattgcgcttctccggaaacattagc

SEQ ID NO: 858 - DNA, 102 bp, Artificial Sequence
  Synthetic Polynucleotide
acaaccgcgtgttacaaggccaggcatccgagaggtctgggaatgccgctgtcggttaagtcttccggtttggtgtcattgcgcttctccggaaacattagc

SEQ ID NO: 859 - DNA, 102 bp, Artificial Sequence
  Synthetic Polynucleotide
acaaccgcgtgttacaaggccaggcatccgagaggtctgggaatgcttctttccacagcgcagcggtaatttcctgcattgcgcttctccggaaacattagc

SEQ ID NO: 860 - DNA, 102 bp, Artificial Sequence
  Synthetic Polynucleotide
acaaccgcgtgttacaaggccaggcatccgagaggtctgggaatgcgctggcatattgcgcccgtaataaatctcgcattgcgcttctccggaaacattagc

SEQ ID NO: 861 - DNA, 102 bp, Artificial Sequence
  Synthetic Polynucleotide
acaaccgcgtgttacaaggccaggcatccgagaggtctgggaatgcagacgttcacatccaccatgtcatacagcgcattgcgcttctccggaaacattagc

SEQ ID NO: 862 - DNA, 102 bp, Artificial Sequence
  Synthetic Polynucleotide
acaaccgcgtgttacaaggccaggcatccgagaggtctgggaatgcacaggtttctgacaggatttcggtcagacgcattgcgcttctccggaaacattagc

SEQ ID NO: 863 - DNA, 102 bp, Artificial Sequence
  Synthetic Polynucleotide
acaaccgcgtgttacaaggccaggcatccgagaggtctgggaatgccggcgcggaaggtacataaaccgccttcagcattgcgcttctccggaaacattagc

SEQ ID NO: 864 - DNA, 102 bp, Artificial Sequence
  Synthetic Polynucleotide
acaaccgcgtgttacaaggccaggcatccgagaggtctgggaatgcatcaagatgggcaacgaccgtttctggcagcattgcgcttctccggaaacattagc

SEQ ID NO: 865 - DNA, 102 bp, Artificial Sequence
  Synthetic Polynucleotide
acaaccgcgtgttacaaggccaggcatccgagaggtctgggaatgcgtcgatgagtttcgggtcaaccggttcttccattgcgcttctccggaaacattagc

SEQ ID NO: 866 - DNA, 102 bp, Artificial Sequence
  Synthetic Polynucleotide
acaaccgcgtgttacaaggccaggcatccgagaggtctgggaatgcataagcaatataaccgtcgcgctcttcggccattgcgcttctccggaaacattagc

SEQ ID NO: 867 - DNA, 102 bp, Artificial Sequence
  Synthetic Polynucleotide
acaaccgcgtgttacaaggccaggcatccgagaggtctgggaatgcctcaagctggtggatcaggtaattcagcgccattgcgcttctccggaaacattagc

SEQ ID NO: 868 - DNA, 102 bp, Artificial Sequence
  Synthetic Polynucleotide
acaaccgcgtgttacaaggccaggcatccgagaggtctgggaatgcccgcgcacgcgataatcaatggttacgatacattgcgcttctccggaaacattagc

SEQ ID NO: 869 - DNA, 102 bp, Artificial Sequence
  Synthetic Polynucleotide
acaaccgcgtgttacaaggccaggcatccgagaggtctgggaatgcgccaacgtcgctgaagtaatggctgagtttcattgcgcttctccggaaacattagc

SEQ ID NO: 870 - DNA, 102 bp, Artificial Sequence
  Synthetic Polynucleotide
acaaccgcgtgttacaaggccaggcatccgagaggtctgggaatgccggatcgtcgtagctaccggcgttatggttcattgcgcttctccggaaacattagc

SEQ ID NO: 871 - DNA, 102 bp, Artificial Sequence
  Synthetic Polynucleotide
acaaccgcgtgttacaaggccaggcatccgagaggtctgggaatgctagataaactcgtcgcgctcggtggtttgtcattgcgcttctccggaaacattagc

SEQ ID NO: 872 - DNA, 102 bp, Artificial Sequence
  Synthetic Polynucleotide
acaaccgcgtgttacaaggccaggcatccgagaggtctgggaatgcgggccagtagcggaacatgggtcatcatctcattgcgcttctccggaaacattagc

SEQ ID NO: 873 - DNA, 102 bp, Artificial Sequence
  Synthetic Polynucleotide
acaaccgcgtgttacaaggccaggcatccgagaggtctgggaatgcgccgccgataatcagcacatgtttcgcgtgcattgcgcttctccggaaacattagc

SEQ ID NO: 874 - DNA, 102 bp, Artificial Sequence
  Synthetic Polynucleotide
acaaccgcgtgttacaaggccaggcatccgagaggtctgggaatgcccgataggatcggtgcagtcggagataatgcattgcgcttctccggaaacattagc

SEQ ID NO: 875 - DNA, 102 bp, Artificial Sequence
  Synthetic Polynucleotide
acaaccgcgtgttacaaggccaggcatccgagaggtctgggaatgccgcgcctgaataatttcggttgagagatggcattgcgcttctccggaaacattagc

SEQ ID NO: 876 - DNA, 102 bp, Artificial Sequence
  Synthetic Polynucleotide
acaaccgcgtgttacaaggccaggcatccgagaggtctgggaatgcgccgtatggattgccggattgtaataacggcattgcgcttctccggaaacattagc

SEQ ID NO: 877 - DNA, 102 bp, Artificial Sequence
  Synthetic Polynucleotide
acaaccgcgtgttacaaggccaggcatccgagaggtctgggaatgcgatactgacggcagaacgatacgacacccgcattgcgcttctccggaaacattagc

SEQ ID NO: 878 - DNA, 102 bp, Artificial Sequence
  Synthetic Polynucleotide
acaaccgcgtgttacaaggccaggcatccgagaggtctgggaatgccatccagcgccattacgcgaccaaatgcagcattgcgcttctccggaaacattagc

SEQ ID NO: 879 - DNA, 102 bp, Artificial Sequence
  Synthetic Polynucleotide
acaaccgcgtgttacaaggccaggcatccgagaggtctgggaatgcaacgaaattgacgccatcgtcgatcaccagcattgcgcttctccggaaacattagc

SEQ ID NO: 880 - DNA, 102 bp, Artificial Sequence
  Synthetic Polynucleotide
acaaccgcgtgttacaaggccaggcatccgagaggtctgggaatgcatctaccgcaaagtactgcccaaactggtccattgcgcttctccggaaacattagc

SEQ ID NO: 881 - DNA, 102 bp, Artificial Sequence
  Synthetic Polynucleotide
acaaccgcgtgttacaaggccaggcatccgagaggtctgggaatgcgtcatgataccgccgtaataggtcgggatccattgcgcttctccggaaacattagc

SEQ ID NO: 882 - DNA, 102 bp, Artificial Sequence
  Synthetic Polynucleotide
acaaccgcgtgttacaaggccaggcatccgagaggtctgggaatgcgtgcgacgaagataccgccaggattcaggccattgcgcttctccggaaacattagc

SEQ ID NO: 883 - DNA, 102 bp, Artificial Sequence
  Synthetic Polynucleotide
acaaccgcgtgttacaaggccaggcatccgagaggtctgggaatgcaagccagtgcgtcttgcagatactgaggtacattgcgcttctccggaaacattagc

SEQ ID NO: 884 - DNA, 102 bp, Artificial Sequence
  Synthetic Polynucleotide
acaaccgcgtgttacaaggccaggcatccgagaggtctgggaatgccaatgccgctgagatcgcggtagctgtcttcattgcgcttctccggaaacattagc

SEQ ID NO: 885 - DNA, 102 bp, Artificial Sequence
  Synthetic Polynucleotide
acaaccgcgtgttacaaggccaggcatccgagaggtctgggaatgcctgccgttaaatcggccatatcttcggcttcattgcgcttctccggaaacattagc

SEQ ID NO: 886 - DNA, 102 bp, Artificial Sequence
  Synthetic Polynucleotide
acaaccgcgtgttacaaggccaggcatccgagaggtctgggaatgccagacggccatcaggctgccgaataacactcattgcgcttctccggaaacattagc

SEQ ID NO: 887 - DNA, 102 bp, Artificial Sequence
  Synthetic Polynucleotide
acaaccgcgtgttacaaggccaggcatccgagaggtctgggaatgcttgacgtaggcaagcaggcttaaggaatcgcattgcgcttctccggaaacattagc

SEQ ID NO: 888 - DNA, 102 bp, Artificial Sequence
  Synthetic Polynucleotide
acaaccgcgtgttacaaggccaggcatccgagaggtctgggaatgctgtcgaaggtgtcgtaattactgaggtccccattgcgcttctccggaaacattagc

SEQ ID NO: 889 - DNA, 102 bp, Artificial Sequence
  Synthetic Polynucleotide
acaaccgcgtgttacaaggccaggcatccgagaggtctgggaatgcccagtgcgcgacgaatttgcccgttaggtacattgcgcttctccggaaacattagc

SEQ ID NO: 890 - DNA, 102 bp, Artificial Sequence
  Synthetic Polynucleotide
acaaccgcgtgttacaaggccaggcatccgagaggtctgggaatgcccgactggcgaattaaatccagcaccatggcattgcgcttctccggaaacattagc

SEQ ID NO: 891 - DNA, 102 bp, Artificial Sequence
  Synthetic Polynucleotide
acaaccgcgtgttacaaggccaggcatccgagaggtctgggaatgctcactgacattacggaagaaatgcagcgcgcattgcgcttctccggaaacattagc

SEQ ID NO: 892 - DNA, 102 bp, Artificial Sequence
  Synthetic Polynucleotide
acaaccgcgtgttacaaggccaggcatccgagaggtctgggaatgcttagcaacaggccagttcgaaatccagacgcattgcgcttctccggaaacattagc

SEQ ID NO: 893 - DNA, 102 bp, Artificial Sequence
  Synthetic Polynucleotide
acaaccgcgtgttacaaggccaggcatccgagaggtctgggaatgcttgcggataaagctgtgaatcgagcgacagcattgcgcttctccggaaacattagc

SEQ ID NO: 894 - DNA, 102 bp, Artificial Sequence
  Synthetic Polynucleotide
acaaccgcgtgttacaaggccaggcatccgagaggtctgggaatgcacgccaatccaggtctggagtttacgttgccattgcgcttctccggaaacattagc

SEQ ID NO: 895 - DNA, 102 bp, Artificial Sequence
  Synthetic Polynucleotide
acaaccgcgtgttacaaggccaggcatccgagaggtctgggaatgcttaatgcttcaatacggctctggtccacgccattgcgcttctccggaaacattagc

SEQ ID NO: 896 - DNA, 102 bp, Artificial Sequence
  Synthetic Polynucleotide
acaaccgcgtgttacaaggccaggcatccgagaggtctgggaatgctgtaggtaaatcaaagctgcaacagccgcccattgcgcttctccggaaacattagc

SEQ ID NO: 897 - DNA, 102 bp, Artificial Sequence
  Synthetic Polynucleotide
acaaccgcgtgttacaaggccaggcatccgagaggtctgggaatgcgtcaagttctttcaacagctcagtgcggaccattgcgcttctccggaaacattagc

SEQ ID NO: 898 - DNA, 102 bp, Artificial Sequence
  Synthetic Polynucleotide
acaaccgcgtgttacaaggccaggcatccgagaggtctgggaatgcgaaattgcccgatacgcggcgcggaaattacattgcgcttctccggaaacattagc

SEQ ID NO: 899 - DNA, 102 bp, Artificial Sequence
  Synthetic Polynucleotide
acaaccgcgtgttacaaggccaggcatccgagaggtctgggaatgcgcgggttcaggctggcaatccaggtttctacattgcgcttctccggaaacattagc

SEQ ID NO: 900 - DNA, 102 bp, Artificial Sequence
  Synthetic Polynucleotide
acaaccgcgtgttacaaggccaggcatccgagaggtctgggaatgcgctcagtcgctgacgcaccagagcaatcaacattgcgcttctccggaaacattagc

SEQ ID NO: 901 - DNA, 102 bp, Artificial Sequence
  Synthetic Polynucleotide
acaaccgcgtgttacaaggccaggcatccgagaggtctgggaatgccccgcaggttgggcaattcaccgtaatagtcattgcgcttctccggaaacattagc

SEQ ID NO: 902 - DNA, 102 bp, Artificial Sequence
  Synthetic Polynucleotide
acaaccgcgtgttacaaggccaggcatccgagaggtctgggaatgctcactgctttggttcttcgctccagtcatccattgcgcttctccggaaacattagc

SEQ ID NO: 903 - DNA, 102 bp, Artificial Sequence
  Synthetic Polynucleotide
acaaccgcgtgttacaaggccaggcatccgagaggtctgggaatgccttcagcagcccattctccgaggtcgatcacattgcgcttctccggaaacattagc

SEQ ID NO: 904 - DNA, 102 bp, Artificial Sequence
  Synthetic Polynucleotide
acaaccgcgtgttacaaggccaggcatccgagaggtctgggaatgccctcaacgccgcatagcgacaggctttcttcattgcgcttctccggaaacattagc

SEQ ID NO: 905 - DNA, 102 bp, Artificial Sequence
  Synthetic Polynucleotide
acaaccgcgtgttacaaggccaggcatccgagaggtctgggaatgcccatcacctcttcaccgtccatccacagggcattgcgcttctccggaaacattagc

SEQ ID NO: 906 - DNA, 102 bp, Artificial Sequence
  Synthetic Polynucleotide
acaaccgcgtgttacaaggccaggcatccgagaggtctgggaatgcgcgctgcttgttccacttcatcaagcaaggcattgcgcttctccggaaacattagc

SEQ ID NO: 907 - DNA, 102 bp, Artificial Sequence
  Synthetic Polynucleotide
acaaccgcgtgttacaaggccaggcatccgagaggtctgggaatgcccgttgccaggaccgttcgctacctttcagcattgcgcttctccggaaacattagc

SEQ ID NO: 908 - DNA, 102 bp, Artificial Sequence
  Synthetic Polynucleotide
acaaccgcgtgttacaaggccaggcatccgagaggtctgggaatgcttcatcgccagcgaattccagttgattggccattgcgcttctccggaaacattagc

SEQ ID NO: 909 - DNA, 102 bp, Artificial Sequence
  Synthetic Polynucleotide
acaaccgcgtgttacaaggccaggcatccgagaggtctgggaatgctacttctgctgcacgaaattgcggtaagcccattgcgcttctccggaaacattagc

SEQ ID NO: 910 - DNA, 102 bp, Artificial Sequence
  Synthetic Polynucleotide
acaaccgcgtgttacaaggccaggcatccgagaggtctgggaatgcttcacctcttcattaaaccagtgcccgacccattgcgcttctccggaaacattagc

SEQ ID NO: 911 - DNA, 102 bp, Artificial Sequence
  Synthetic Polynucleotide
acaaccgcgtgttacaaggccaggcatccgagaggtctgggaatgcatggacatacgcacctttaccactccggtacattgcgcttctccggaaacattagc

SEQ ID NO: 912 - DNA, 102 bp, Artificial Sequence
  Synthetic Polynucleotide
acaaccgcgtgttacaaggccaggcatccgagaggtctgggaatgcagtcgatactgatagccatcgagcttcggtcattgcgcttctccggaaacattagc

SEQ ID NO: 913 - DNA, 102 bp, Artificial Sequence
  Synthetic Polynucleotide
acaaccgcgtgttacaaggccaggcatccgagaggtctgggaatgcgcagcacttcaacttccagcgtcgcggtatcattgcgcttctccggaaacattagc

SEQ ID NO: 914 - DNA, 102 bp, Artificial Sequence
  Synthetic Polynucleotide
acaaccgcgtgttacaaggccaggcatccgagaggtctgggaatgcgcatttctgcttcttccaggtagtgtgtggcattgcgcttctccggaaacattagc

SEQ ID NO: 915 - DNA, 102 bp, Artificial Sequence
  Synthetic Polynucleotide
acaaccgcgtgttacaaggccaggcatccgagaggtctgggaatgcaccagtgaaacaaacagctcttccagacggcattgcgcttctccggaaacattagc

SEQ ID NO: 916 - DNA, 102 bp, Artificial Sequence
  Synthetic Polynucleotide
acaaccgcgtgttacaaggccaggcatccgagaggtctgggaatgcctgcctgattcaccacaatttgctgcacggcattgcgcttctccggaaacattagc

SEQ ID NO: 917 - DNA, 102 bp, Artificial Sequence
  Synthetic Polynucleotide
acaaccgcgtgttacaaggccaggcatccgagaggtctgggaatgcatcccgccagataacatacgcgcacgttcgcattgcgcttctccggaaacattagc

SEQ ID NO: 918 - DNA, 102 bp, Artificial Sequence
  Synthetic Polynucleotide
acaaccgcgtgttacaaggccaggcatccgagaggtctgggaatgccctgcggcaccagtcccaactgacgtttagcattgcgcttctccggaaacattagc

SEQ ID NO: 919 - DNA, 102 bp, Artificial Sequence
  Synthetic Polynucleotide
acaaccgcgtgttacaaggccaggcatccgagaggtctgggaatgcgcattaacgcacgggcaatcattaaacggccattgcgcttctccggaaacattagc

SEQ ID NO: 920 - DNA, 102 bp, Artificial Sequence
  Synthetic Polynucleotide
acaaccgcgtgttacaaggccaggcatccgagaggtctgggaatgcacattgagcggcgaagttcaatatccacgccattgcgcttctccggaaacattagc

SEQ ID NO: 921 - DNA, 102 bp, Artificial Sequence
  Synthetic Polynucleotide
acaaccgcgtgttacaaggccaggcatccgagaggtctgggaatgctctcgagatcgtaaccaaatacgctgaccccattgcgcttctccggaaacattagc

SEQ ID NO: 922 - DNA, 102 bp, Artificial Sequence
  Synthetic Polynucleotide
acaaccgcgtgttacaaggccaggcatccgagaggtctgggaatgcgatgtacgcttctttgcgctccacgccgtacattgcgcttctccggaaacattagc

SEQ ID NO: 923 - DNA, 102 bp, Artificial Sequence
  Synthetic Polynucleotide
acaaccgcgtgttacaaggccaggcatccgagaggtctgggaatgccggtgcgagatcgagaataaaggtttccgacattgcgcttctccggaaacattagc

SEQ ID NO: 924 - DNA, 102 bp, Artificial Sequence
  Synthetic Polynucleotide
acaaccgcgtgttacaaggccaggcatccgagaggtctgggaatgcccaccagctcaccgtgttgaataatgccgacattgcgcttctccggaaacattagc

SEQ ID NO: 925 - DNA, 102 bp, Artificial Sequence
  Synthetic Polynucleotide
acaaccgcgtgttacaaggccaggcatccgagaggtctgggaatgctcacccgcttcgacctgcaaatctatcccacattgcgcttctccggaaacattagc

SEQ ID NO: 926 - DNA, 102 bp, Artificial Sequence
  Synthetic Polynucleotide
acaaccgcgtgttacaaggccaggcatccgagaggtctgggaatgctgatgacgcaacgttggcgtaggcattggtcattgcgcttctccggaaacattagc

SEQ ID NO: 927 - DNA, 102 bp, Artificial Sequence
  Synthetic Polynucleotide
acaaccgcgtgttacaaggccaggcatccgagaggtctgggaatgcttagctacgcaaaccacgtccacgttggatcattgcgcttctccggaaacattagc

SEQ ID NO: 928 - DNA, 102 bp, Artificial Sequence
  Synthetic Polynucleotide
acaaccgcgtgttacaaggccaggcatccgagaggtctgggaatgcgcgtctgcacccagatacgcataaagcgatcattgcgcttctccggaaacattagc

SEQ ID NO: 929 - DNA, 102 bp, Artificial Sequence
  Synthetic Polynucleotide
acaaccgcgtgttacaaggccaggcatccgagaggtctgggaatgcaaagtaaagggtcatggtgatgactggcggcattgcgcttctccggaaacattagc

SEQ ID NO: 930 - DNA, 102 bp, Artificial Sequence
  Synthetic Polynucleotide
acaaccgcgtgttacaaggccaggcatccgagaggtctgggaatgcggcaaacacaccgttcagcaaacccgcaagcattgcgcttctccggaaacattagc

SEQ ID NO: 931 - DNA, 102 bp, Artificial Sequence
  Synthetic Polynucleotide
acaaccgcgtgttacaaggccaggcatccgagaggtctgggaatgctacgtgagtggcgttaacacaaaggttggccattgcgcttctccggaaacattagc

SEQ ID NO: 932 - DNA, 102 bp, Artificial Sequence
  Synthetic Polynucleotide
acaaccgcgtgttacaaggccaggcatccgagaggtctgggaatgcctgcatatagctgaagccatgcatatcgcccattgcgcttctccggaaacattagc

SEQ ID NO: 933 - DNA, 102 bp, Artificial Sequence
  Synthetic Polynucleotide
acaaccgcgtgttacaaggccaggcatccgagaggtctgggaatgctataaacgattgggttcaggtgcgacagcccattgcgcttctccggaaacattagc

SEQ ID NO: 934 - DNA, 102 bp, Artificial Sequence
  Synthetic Polynucleotide
acaaccgcgtgttacaaggccaggcatccgagaggtctgggaatgctatccggcaataatgacgtgagtcggaacccattgcgcttctccggaaacattagc

SEQ ID NO: 935 - DNA, 102 bp, Artificial Sequence
  Synthetic Polynucleotide
acaaccgcgtgttacaaggccaggcatccgagaggtctgggaatgcccgtgagcaccagcgttaaggcaacgaatacattgcgcttctccggaaacattagc

SEQ ID NO: 936 - DNA, 102 bp, Artificial Sequence
  Synthetic Polynucleotide
acaaccgcgtgttacaaggccaggcatccgagaggtctgggaatgctgaccagcggaacatcattgataccgaggacattgcgcttctccggaaacattagc

SEQ ID NO: 937 - DNA, 102 bp, Artificial Sequence
  Synthetic Polynucleotide
acaaccgcgtgttacaaggccaggcatccgagaggtctgggaatgccgccacaataaagaccaccagtacgccaaacattgcgcttctccggaaacattagc